European Patent Specification EP 3 830 276 B1, published July 24, 2024. Title: Method. Applicant: British American Tobacco (Investments) Limited. The sequence listing filed with the application follows.

SEQUENCE LISTING (60 sequences)

SEQ ID NO: 1 - DNA, 3406 bp, Artificial Sequence
  genomic sequence encoding protein of the invention
attattttttcctatataaacattaatcatacgactacaaccagaggaattaatcgttcaaatataactaactactcctctaaacatggagataagtcgcagcaatgttagtggtggtggcggcagcggcggcgctctggacgacagttttagcagttttaggacggaactgctgtctccggctgctcaggcggtggtggatcagtcgtcttcgtcggcgtcatggagacttaacattagcgaattccgtcttcccgaacgaagccgctcctcctccgatcatcactcctttagtgtccgtcgtctacttcccactcccagtatgtgtatatatatatatatatatatatatattcctcacttcacttgtctttacaatgtattaaacctttctacttcctttgaacttcttcggatttgttaattaatgttaagagatttgagggaagccttggcttactggtaaagtgatggcatgtgacttcccagtcacatgtttaagccgtgttaaagttgttggcatgtgacctcctggtcacaggtttaagccgtggaaatagactttcgtagaaatacaggtaaagaaatgcaggtaaggttgcgtacttgtgatctggccctttctcgaatctcgcacataaatgaagcttagtgcctttttttaaggttaatagttttttagtcagaatagtaccaaaattagactagaagattcatagttctaatattggtaaaccaaaatttacgacttatatatatttacataaatgggcgaggaatctttattcttatcatgccatagtccatggaacgtactgagcctttaatttctatttgctattgctgggaaatgaatcagatggccaattttcttatgtatacatattctcactggtatgggatcgaatcggcgacagaactccaagttagaggattctttttcattaagtcattacttattttaagttcaagtaacagcactggaagttcaactaagagttgataaacatgatcagtgaaactcacaattgtttgtcctaaattttggatctttacttggaaagtgtagatgttagtatatgcttatgctatactggccagcagtgctcgtaacagtatctatgagtactaataggcttatgctatattactgtatttataatgctaatcagctaatgagatatgataactcatatatgacaactacagtaggaaattcagataaccatattcattttttcagtagtctcagttttgagttttgcttttcccttgcctgagtttacctaatggaatcatttgaaattcatccgtagggaaacaaggtaaaattgctgaatactacaaaaaacaagaaaggctgcttgaagggttcaatgagatggacaccattaatgaatctggttgtttacctggaagtctaactgaggtgtgtttctggaatctggatactgttttcaattgatgataagtatgtgaatttttgtatcgaccgatcatgtttgttcaggatgaaatgaagcagcttgcaagaagtgaaaggatggctattcatttatcaaacatggctaatgtggttcttttcattgcaaaaatctacgcttctattgagagcagatctttggctgtaatcgcgtcaacgttggactccctcttagacctcttatcagggtttatactgtggttcacttctcatgccatgaaaaatccaaaccagtatcactatcctattggaaaaaagaggatgcagccattggtgagtcttcaaatatatgtgacatcccttaaaagaattatctctggcatttgttctgtttcgtgtctgcgataaaatgaccttaatgttcaattcatggatcatattttaccttgtttctgtagaaccctttttactcattagatgcaatttgttcagggtattattgtttttgcatctgtaatggcgacactaggattacaaatattgttcgagtcagctaaagaactcataactaaggtatgtgaattgcttcacttcaactatcctgagaattttcagagcagcaggttcttatggttagtagagttttgagtttctaaaatcttttacatcaagacaaaaaaaaacatgcaatttataggaaacaagaagacgaaaaacgggttgagttactactgaaatgaagttgtagccaaaccagttaggccaaagatgtttacataagataaattaggctactgtatactacctaataaaaagggactggttttgatatttctactgatgttgcatagctaagtgaagattaactcgcatagtgctacttcaattgtaggatatagacttgtaacttactgcaatttcactaacaattgcattacccttgacatcttaatctacgtttgttgtttcggtggttctatgcttacgatcagtctcgccctgagatggaccatgagaaggaaaaatggacgattggtattatggtctctgtcactatggtcaagtttctgcttatggtctactgtcgaaggttcaaaaacgaaatcgtaagagcctatgctcaagatcatttctttgatgtcatcaccaactcagttggattagtgactgctgtcttagcagtccgattctactggtggattgatcctacgggagctataattgtgagttcacaatcacaactcaaatatttcaattagtaagcttgtaaatatatactccaaccttgtttcacactgctggtgatgttaagagtctaatacatcttgcatattcagatagctatgtacacaattagcacgtgggcgaagacagtggcagaaaatgtctggtcactcattggaagaacagctccaccagattttcttacgaaattaacctatcttatatggaatcatcacgaagagatcaagcacattgatactgttcgagcatatacttttggtgctcattattttgtagaggttgatatagtgttgccagaggacatgctgttgaacaaggcacataatattggtgagacactgcaagaaaaattggagcaactccctgaagttgagcgagcttttgttcatatagacttcgagttcactcacaggccagaacacaaaactatggtataatgacaccagaatttaaactctatgtgttcaaccttaaagatttttagcgttgaatcaatcatatttttaaagttatgggttcatttctactatttgttgcaattttaataatttttacgcataaatttgtatttcgcgtcgaaagtactaggttcacatgaatccggtatcaaagggctagatccgccccctgactacacatcatttacggtgtttctttttgtaactcaaaataattttaatggtgcttcttagagttgaatctgtgaattagtcgcacctttaaggcttatgagatggg

SEQ ID NO: 2 - DNA, 1251 bp, Artificial Sequence
  cDNA sequence encoding protein of the invention
atggagataagtcgcagcaatgttagtggtggtggcggcagcggcggcgctctggacgacagttttagcagttttaggacggaactgctgtctccggctgctcaggcggtggtggatcagtcgtcttcgtcggcgtcatggagacttaacattagcgaattccgtcttcccgaacgaagccgctcctcctccgatcatcactcctttagtgtccgtcgtctacttcccactcccaggaaacaaggtaaaattgctgaatactacaaaaaacaagaaaggctgcttgaagggttcaatgagatggacaccattaatgaatctggttgtttacctggaagtctaactgaggatgaaatgaagcagcttgcaagaagtgaaaggatggctattcatttatcaaacatggctaatgtggttcttttcattgcaaaaatctacgcttctattgagagcagatctttggctgtaatcgcgtcaacgttggactccctcttagacctcttatcagggtttatactgtggttcacttctcatgccatgaaaaatccaaaccagtatcactatcctattggaaaaaagaggatgcagccattgggtattattgtttttgcatctgtaatggcgacactaggattacaaatattgttcgagtcagctaaagaactcataactaagtctcgccctgagatggaccatgagaaggaaaaatggacgattggtattatggtctctgtcactatggtcaagtttctgcttatggtctactgtcgaaggttcaaaaacgaaatcgtaagagcctatgctcaagatcatttctttgatgtcatcaccaactcagttggattagtgactgctgtcttagcagtccgattctactggtggattgatcctacgggagctataattatagctatgtacacaattagcacgtgggcgaagacagtggcagaaaatgtctggtcactcattggaagaacagctccaccagattttcttacgaaattaacctatcttatatggaatcatcacgaagagatcaagcacattgatactgttcgagcatatacttttggtgctcattattttgtagaggttgatatagtgttgccagaggacatgctgttgaacaaggcacataatattggtgagacactgcaagaaaaattggagcaactccctgaagttgagcgagcttttgttcatatagacttcgagttcactcacaggccagaacacaaaactatggtataa

SEQ ID NO: 3 - protein, 416 aa, Artificial Sequence
  polypeptide sequence of protein of the invention
MEISRSNVSGGGGSGGALDDSFSSFRTELLSPAAQAVVDQSSSSASWRLNISEFRLPERSRSSSDHHSFSVRRLLPTPRKQGKIAEYYKKQERLLEGFNEMDTINESGCLPGSLTEDEMKQLARSERMAIHLSNMANVVLFIAKIYASIESRSLAVIASTLDSLLDLLSGFILWFTSHAMKNPNQYHYPIGKKRMQPLGIIVFASVMATLGLQILFESAKELITKSRPEMDHEKEKWTIGIMVSVTMVKFLLMVYCRRFKNEIVRAYAQDHFFDVITNSVGLVTAVLAVRFYWWIDPTGAIIIAMYTISTWAKTVAENVWSLIGRTAPPDFLTKLTYLIWNHHEEIKHIDTVRAYTFGAHYFVEVDIVLPEDMLLNKAHNIGETLQEKLEQLPEVERAFVHIDFEFTHRPEHKTMV

SEQ ID NO: 4 - DNA, 3691 bp, Nicotiana tabacum
ataaacattaatcatacgactataaccagaggaattaattgttcaaatattagaaactactcctctaaacatggagatgagtcggagtgacgttagtggtggcggcggcagcggcggcgctttggacgacagttttagcagttttaggacggaactactgtctccggctgctcaggcggtggtggatcagtcgtcttcttcggcgtcatggagacttaacattagcgaattccgtcttcccgaacgaagccgctcctcctccgatcatcacacctttagtgtccgtcgcctacttcccactcccagtatgtatgtgtatatatatatatattatattcctctcttcacttgtctttacaatgtattaaacctttctactctttgaacttcttcggctttgttaattagtgttgagagttttgaaaggtagcctgacgtaactggtaaagttgtcgccatgtgacctcctggtcacaggttagaaatagtctcttgcgtaaatgcagggtatgactgcgtacaatatttatatgaaataaatatgaagtacaagaacccagactctctcaaaacaccacgcatagctggaacttagtgcactagccacgctttttaatgttaagagttttctactcagaatagtaccaaaattagactagaagattcatagttctaatattggcaaaccaaaatttacgacttatatatatttacataaatgggcgatgaatctttattcttatcatgccatagtccatggaacatactaagcctttaatttctactccctccgtttcaattcatgtgaactcatttgatcgggcacggaatttaagaaaagagagaaaacttttgaacttctggtgtaaatgaggcacatatattttatgtggctataaattattgcataaagataaattgtttccaaatagggaaatgactcattctttttggtatgtactaaaaaggaaatagggaaacggagggagtatttgctattgctgggaaatgaatcagatggccaattttcttatgtatatatacatattctcactggcatgggatcaaatcggcgacagaactccaagttagaggactctttttcatgaagtcattacttaatttaagttcaagtaacagcagtggaagttcaactaagagttgataaacatgatcagtgaaactcacaattgttcgtccaaatttcggatattcacttggaaggtgtagatgttagtatatgcttatgctatattggccagcagtactcgtagcagtatctatgagtactaaaatgcttatgctatattactgtatttgtaatgttaatgagatatgattactcatatatatgacaactacagggggagattcagataaccaagttcatttcagtctgtaattcagtctcagttttgagttttgcttttctcttgggtgagtttacctgatgaaattattttaaattcatccgtaggaaaacaaggtaaaattgctgaatactacaaaaaacaagaaaggctgcttgaagggttcaatgagatggacaccattaatgaatctggctgtttacctggaagtctaactgaggttggtttctgaaatctggatactatttgcaattgacgaataagtatgtgaatttttgtatcgaccgaccatgttttttcaggatgaaatgaagcagctagcaaggagtgaaaggatggctattcatttatcaaacatggctaatgtggttcttttcattgcaaaaatctacgcttctattgagagcagatctttggctgtaatcgcgtcaacgttggactccctcttagacctcttatcagggtttatactgtggttcacttctcatgccatgaaaaatccaaaccagtatcactatcctattggaaaaaagaggatgcagccagtggtgagtcttcaaatatatgtaacatcctgaaattattatctctggcttttgttctgtcttcgtttatttgcaaaaatgaccttaatgttcaatacatagatcacattttacatttgaccttcacattttttcctttgctgttgctgatacattgtctctttccttcttgtgccgagggtctaccgaaaacagcctctctactcctccggagtaggggtaaggtctgcgtacacactaccctccccagactcaacttgtgggatctcattgggttgttgttgtctgtagaactgttttatagatcacattttaccttgtttccgttgaaccgtttttactcattagttgcattttcttcagggtattattgtttttgcatctgtgatggcgacactaggattacaaatgttgttcgagtctgctaaggaactcataactaaggtatgtgaattggttcacctcaactatcctgagaattttcagagcagcaggttcttatggctgtattagtagagttttgagtttctataatctttaacatcaagatgaaaaaccatgcaatttataggaaacaagaagacgaaaaaggggttgagttactactgaaatgaagttgcagtcaaaacagttaagccaaagatgtttacataagataaattaggctactgtatactactaataaaagtgactggttttgatatttctattgatgttgcatagcttaataaagattatctcgcatagtgctacttctattgtaggatatagacttgtaagttattgcattttcactaacaattgcattacgcttgacatcttaacctatgtttgttgtttcgatggttctatgcttacgatcagtctcgccctgagatggatcatgagaaggaaaaatggacaattgggattatggtctctgtcactatggtcaagtttctgcttatgatctactgtcgaaggttcaaaaacgaaatcgtaagagcctatgctcaagatcatttctttgatgtcatcactaactcagttggattagtgacggctgtcttagcagtacgattctactggtggattgatcctacaggagctataattgtgagttcacaatcacaactcaaaaacttacacaattagcaatcacacttctggtaatgtcaatagtctaatatattttgcatatccagatagctgtgtacacaattagcacgtgggcgaagacagtggctgaaaatgtctggtcgctcattggaagaacagctccaccagattttcttacgaaattaacctatcttatatggaatcatcacgaagagatcaagcacattgatactgttagagcatatacttttggtgcgcattactttgtggaggttgatatagtgttgccagaggacatgctgttgaatcaggcacataatattggtgagacactgcaagaaaaattggagcaactccctgaagttgagcgagcttttgttcatatagactttgagttcactcacaggccagaacacaaaaccatggtataatgacatagtggttgcaacaagtacgcacataggcggatccaagctttaaactctatacgtacaacctttaagatttttagcgttgaactgatcatatttttaaagttatggcttcatatctactactatttgttgcaattttaataaatttttttacataaatttgtattctacatcgaaagtactgggttcagataaacttggtgaccaaagggctggatccgcccctgactacacattatttaca

SEQ ID NO: 5 - DNA, 1251 bp, Nicotiana tabacum
atggagatgagtcggagtgacgttagtggtggcggcggcagcggcggcgctttggacgacagttttagcagttttaggacggaactactgtctccggctgctcaggcggtggtggatcagtcgtcttcttcggcgtcatggagacttaacattagcgaattccgtcttcccgaacgaagccgctcctcctccgatcatcacacctttagtgtccgtcgcctacttcccactcccagaaaacaaggtaaaattgctgaatactacaaaaaacaagaaaggctgcttgaagggttcaatgagatggacaccattaatgaatctggctgtttacctggaagtctaactgaggatgaaatgaagcagctagcaaggagtgaaaggatggctattcatttatcaaacatggctaatgtggttcttttcattgcaaaaatctacgcttctattgagagcagatctttggctgtaatcgcgtcaacgttggactccctcttagacctcttatcagggtttatactgtggttcacttctcatgccatgaaaaatccaaaccagtatcactatcctattggaaaaaagaggatgcagccagtgggtattattgtttttgcatctgtgatggcgacactaggattacaaatgttgttcgagtctgctaaggaactcataactaagtctcgccctgagatggatcatgagaaggaaaaatggacaattgggattatggtctctgtcactatggtcaagtttctgcttatgatctactgtcgaaggttcaaaaacgaaatcgtaagagcctatgctcaagatcatttctttgatgtcatcactaactcagttggattagtgacggctgtcttagcagtacgattctactggtggattgatcctacaggagctataattatagctgtgtacacaattagcacgtgggcgaagacagtggctgaaaatgtctggtcgctcattggaagaacagctccaccagattttcttacgaaattaacctatcttatatggaatcatcacgaagagatcaagcacattgatactgttagagcatatacttttggtgcgcattactttgtggaggttgatatagtgttgccagaggacatgctgttgaatcaggcacataatattggtgagacactgcaagaaaaattggagcaactccctgaagttgagcgagcttttgttcatatagactttgagttcactcacaggccagaacacaaaaccatggtataa

SEQ ID NO: 6 - protein, 416 aa, Nicotiana tabacum
MEMSRSDVSGGGGSGGALDDSFSSFRTELLSPAAQAVVDQSSSSASWRLNISEFRLPERSRSSSDHHTFSVRRLLPTPRKQGKIAEYYKKQERLLEGFNEMDTINESGCLPGSLTEDEMKQLARSERMAIHLSNMANVVLFIAKIYASIESRSLAVIASTLDSLLDLLSGFILWFTSHAMKNPNQYHYPIGKKRMQPVGIIVFASVMATLGLQMLFESAKELITKSRPEMDHEKEKWTIGIMVSVTMVKFLLMIYCRRFKNEIVRAYAQDHFFDVITNSVGLVTAVLAVRFYWWIDPTGAIIIAVYTISTWAKTVAENVWSLIGRTAPPDFLTKLTYLIWNHHEEIKHIDTVRAYTFGAHYFVEVDIVLPEDMLLNQAHNIGETLQEKLEQLPEVERAFVHIDFEFTHRPEHKTMV

SEQ ID NO: 7 - DNA, 4523 bp, Nicotiana tabacum
acagtttgagcctatttttcctctcattatatctatgtgttatctttcctcaaaagtatctttaactaaacctatctttagaagagtccttttgcgtctccctacttcgacttactagtatacaactatagataaatatcaaaacacaagtacattgtcattcgtacaaatatttagtaacaattttcatggaaatcgttggcggtaacggtggtgatcatggcggcgccactcatcagccgttgccgttgtcgttatcttcctcttcgccgtcggcgtcgtggaggctgaatataggggagtttcgtgtccctgaaaatggcactgctgatcatcgtcaatctttcagtttacgtcgactcttacgtcgcccttctagtaattttccttccttttatcttttatatttcttctatgatattgtttgctagctttattgcacttgtcgaaaaaaaaaaaactacttggaaatcattgcattttaatggtatttgaatccattcaaccatctcctagcaaattactcccaccgttttattttatgtgaatttgtttgactgaaaacaaaatttaagaaaggaattactactttggaacttgtagtattaaacatttcaccaccttaatttgtatgtaaaataaaaataattaatgttaaattatttctaaatatagaaagatcgtctttttttgaaagcaagattaaaaaataattgtgtgttttaagtacaactcacttcaaccaattgttttaagttctaactttggtttggatatccttttttttcttttgtcttcaagaactacttaactaagaaaatagtttttataaattttctattacctatcttagttttcagcctgtcaacatccattatttgtaaggattttatcttttatcttacaaatcattttcatatatatctctatatatagaaaaacaaggcaaagtagctgaatattacgagaagcaagaaaggttggttgaagggttcaatgagatggacactgttcatgaatctggctttttacctggaactctaaccgaggttcgtctcttttcctcaataataaactgataatgaaagaatttatacgtcacttaaaaattcacacaagatatgatatataggccggtgcataaagtattctgtatccacgcagggtcttggaagtatcaccgcaccacctcaagaagtgtgatgtagacagccgacctaatgcaaatattagtggttgcttttacggctcgaacccgtgacctgtaggtcacacgacaactttattatttttttagtcatgagtctcatgacctatatgtcacttaaaaatatattactgttaaatatttataataagaaaaattaataacctggaaaataagtcaaacagcctcgtaggatatatatattaatagtgtaattttttttttatagtcaatatttggcctcagtatcacagcttggggatatgatgtcggggcatgtgtcccctaacttttctaagtttaatttcctactcttaggaaatgtcaaatttttggaaattttgctttagtgaaaattcttcttctccttctttccttgtaaaagtgtcctactcttcagaagttttgtgtttttggcataagtttacttgtgggaggtcaactttactatttttcaagttcgttacttcacttattatagatggttagtttaagttatctttcaagtgacatatagtagtagaaaatttttagattgttaatgcataaaaggttaaaagttaaactcaaaaaaagagcataacttataaacaacaattacttttttttaaaccttttgttaggtcacttaacagataattacaagtcacggtctataatatataagtgagactagtaatcttaacaaattctgataacttgctacaacaggtcaaaatagtctaactaataaagtaggattaatctcacttttattctctacaactcaatatttgtcaggatgaaatgaagcagcttgctaagagtgagaggatggcaattcatgtatcaaacatagcaaatgtggttcttttcattgcaaaaatctatgcttctattgcaagtagatctttggctgtgattgcatcaactttggactcactcttagacttattgtctggatttattctgtggttcactgtatatgcaatgaaaaatccaaaccaataccactatccaattggtaaaaagagaatgcagcctgtggtgagtcttcaaaaataacgttgtgacattttgatatttgttacattcattctatactttgtgtcagtctgatatgagttttatagccaaataaaatatttatatgtaatatttatagggtattattgtttttgcatcggtgatggcaacccttggattacaaatactatttgagtctggtaaagaactcatacataaggtacgtgactcggttctctaaagtctttttttagaaaaaaaaaggaatttctaaatttaacttttcaaaataatacaaaatgatgaaaactgttctcctatatcatgatctttctcttggacttcaagacgcagttgtttatgctacattatttggctattagatgaagtattgaccaatatctttatgcacgttagttgacttttatgtactcatagtataaaaaagatatttatacaatttggtcttatataacgtgatatatgtaactttgatgataagcattactccatttgtttaattaatatgacggtatttcactaaatatggagttcaagaaacaaaaaaaaaggagacttctgcaacttgtgttcatacatgccatgaaattttgtggctataaaatcatgtcattaaggataaaatgcaagatgaggagtaattggtaaatatttagtactatcacagattaaactacactaatgtcagtttattgtttcttcttgttcaatgcttatcatatcagtctcgtcctaatacggatcctgagaaggaaaaatggatgattgggatcatggtctctgtcactgttgttaagtttctgcttatggtttattgtcgaagattcaagaatgaaattgtaagagcctatgctcaagaccatttatttgatgtcattaccaactctgttggattagtgactgcagttttagcaattcgattctgctggtggattgatcctacgggagctatattggtgagttcacaatcatcacttatacttcttttgcttttatctacttatttaataggcatctcgatgcataacgtatttcccgttcatacatgattcgggaaaagccgcacctaaaaggtatgatatagatatcctaccctaatgcaagcattaatgattgctttcacggttcgaaccatatagtggtgttcgcatcaacttgcgcagcacctcaactatttcacttagtacatgtaatctctcactaaaaaatttaccggacaccttgttactccccaaggctttggcgtgtgggaataacttgtattttttgtctctactagaaaaggaatcctaatttcaacctttatatcaattttattgatcactaagtcatactcttgggtgcacgtgcacacacatacgacactacatctgtctcaatttactaagtactatttcctttttgttttcttttgtcctgaaagattgatatctttatagctttagaaactccaaacatttatttatatttttatatcaagattgacacctttatgtatatatggtatttctgacttattaagcatattaaacttctatgtcagagatctcttttattttttaaacttcatgtctagtcaaaggatgctaaaccaattgtggtggacgactatcactaaatgattgagcaaataaaatgagtagaaattttcaaagacatccctccaaattttccattattattaaggataacattatgtatttgcagatagcactatacacaattggtacgtgggcaaagacagtaatcgaaaatatgcgatcactcatcggaagaacagctccaccagaatttctggcgaaattaacatatcttatatggaatcatcacaaagaaatcaagcacattgatactgtgagagcatacacatttggtacaaattactttgtggaagttgatatagttttgccagaggacatgcttctaagccaagcacataatattggtgaaacattgcaagaaaaattagagcagcttcctgatgttgagagagcttttgtgcatgttgatttcgagttcactcatagaccagagcacaagactatggtctaatgacataaataaactaggtaattaataattaaaaattagtttgagcttgaactttgttgttgggcactgtttccttgcacctggagtagtaacttaccaaaaaaaaaagttctttaatgtggagaacccaaccatgttgaaacttgttgaatttgcattctcaaaatttatgtaacctaatgtttatttttaactcaagatgcctcatgagtcatgaacgacaagtatatacctacgt

SEQ ID NO: 8 - DNA, 1206 bp, Nicotiana tabacum
atggaaatcgttggcggtaacggtggtgatcatggcggcgccactcatcagccgttgccgttgtcgttatcttcctcttcgccgtcggcgtcgtggaggctgaatataggggagtttcgtgtccctgaaaatggcactgctgatcatcgtcaatctttcagtttacgtcgactcttacgtcgcccttctaaaaaacaaggcaaagtagctgaatattacgagaagcaagaaaggttggttgaagggttcaatgagatggacactgttcatgaatctggctttttacctggaactctaaccgaggatgaaatgaagcagcttgctaagagtgagaggatggcaattcatgtatcaaacatagcaaatgtggttcttttcattgcaaaaatctatgcttctattgcaagtagatctttggctgtgattgcatcaactttggactcactcttagacttattgtctggatttattctgtggttcactgtatatgcaatgaaaaatccaaaccaataccactatccaattggtaaaaagagaatgcagcctgtgggtattattgtttttgcatcggtgatggcaacccttggattacaaatactatttgagtctggtaaagaactcatacataagtctcgtcctaatacggatcctgagaaggaaaaatggatgattgggatcatggtctctgtcactgttgttaagtttctgcttatggtttattgtcgaagattcaagaatgaaattgtaagagcctatgctcaagaccatttatttgatgtcattaccaactctgttggattagtgactgcagttttagcaattcgattctgctggtggattgatcctacgggagctatattgatagcactatacacaattggtacgtgggcaaagacagtaatcgaaaatatgcgatcactcatcggaagaacagctccaccagaatttctggcgaaattaacatatcttatatggaatcatcacaaagaaatcaagcacattgatactgtgagagcatacacatttggtacaaattactttgtggaagttgatatagttttgccagaggacatgcttctaagccaagcacataatattggtgaaacattgcaagaaaaattagagcagcttcctgatgttgagagagcttttgtgcatgttgatttcgagttcactcatagaccagagcacaagactatggtctaa

SEQ ID NO: 9 - protein, 401 aa, Nicotiana tabacum
MEIVGGNGGDHGGATHQPLPLSLSSSSPSASWRLNIGEFRVPENGTADHRQSFSLRRLLRRPSKKQGKVAEYYEKQERLVEGFNEMDTVHESGFLPGTLTEDEMKQLAKSERMAIHVSNIANVVLFIAKIYASIASRSLAVIASTLDSLLDLLSGFILWFTVYAMKNPNQYHYPIGKKRMQPVGIIVFASVMATLGLQILFESGKELIHKSRPNTDPEKEKWMIGIMVSVTVVKFLLMVYCRRFKNEIVRAYAQDHLFDVITNSVGLVTAVLAIRFCWWIDPTGAILIALYTIGTWAKTVIENMRSLIGRTAPPEFLAKLTYLIWNHHKEIKHIDTVRAYTFGTNYFVEVDIVLPEDMLLSQAHNIGETLQEKLEQLPDVERAFVHVDFEFTHRPEHKTMV

SEQ ID NO: 10 - DNA, 6216 bp, Nicotiana tabacum
  misc_feature (1259)..(1840): n is a, c, g, or t
tatagaagagtccttttgcttctccctacttgcaaatgataaatatcaaaacacaagtacattttcactcgtacaaatactagtaacaattttcatggagatcgttggcagcaacggcggtgatcatggcggcgccacccatcagccggtgccgttatcttcctcttcaccgtcggcgtcgtggaggctgaatataggggagtttcgtgtccctgaatatggcactggtgatcatcgtcaatctttcagtttacgtcgactcttgcgtcgcccttctagtaattttccttcaatttatctttttttttgtccttttatgatattgttttccattttttgcacttgtcgaagtaaaaactacttgaataaatggttgaattaagacaaatattgattaatctgaaggtattaaatcattgcattttaattgtcattgaattcatttaactatctcctagaaaactactctctcgattttattttatgtgaatctatttgataaaagatgaaaacttaagaaagaacggctttgaaacttatgagttacatttcaacatatttgtgcagtaaaattaaaaaaaaattaaagtaatattattttttaaatataaaaaagatcatgtcattctttttaaaacaagattaaaaagtaaattgctcttttaagtacaactcaattctaccaatggttttaagttctaactttggtttggatatccttttaatttcttcttcttttgtcttcaagaactactcaactaaagaaattggttttagtctttttaaacaaagaggtatgacatttttttcgatagcttaaaacggaaagtatgacatataaattggaatatatatatgaattaagtactattataaattaaatcatatttttaaggattttgtcttttatgttacacgacttgatgagatcattttaatatctctatatatagaaaaacaaggcaaagtagctgaatattacgagaagcaagaaaggttgcttgaagggttcaatgagatggacactgttcatgaatctggctttttacccggaagtctaaccgaggtttgtctcttttcctcacactattaagttacttaaaaaattattaccattatttatttataataaataaaattagtaacctgaaatataagacaaacaatatcttatacgatatgtatactaatagtgtaagttttcttgttacgtcaatatttcacagataggtgacatgatgtcggggccggtgttcccnnnnnnnnnnnnnnnnnnnnnnnnnnnnnnnnnnnnnnnnnnnnnnnnnnnnnnnnnnnnnnnnnnnnnnnnnnnnnnnnnnnnnnnnnnnnnnnnnnnnnnnnnnnnnnnnnnnnnnnnnnnnnnnnnnnnnnnnnnnnnnnnnnnnnnnnnnnnnnnnnnnnnnnnnnnnnnnnnnnnnnnnnnnnnnnnnnnnnnnnnnnnnnnnnnnnnnnnnnnnnnnnnnnnnnnnnnnnnnnnnnnnnnnnnnnnnnnnnnnnnnnnnnnnnnnnnnnnnnnnnnnnnnnnnnnnnnnnnnnnnnnnnnnnnnnnnnnnnnnnnnnnnnnnnnnnnnnnnnnnnnnnnnnnnnnnnnnnnnnnnnnnnnnnnnnnnnnnnnnnnnnnnnnnnnnnnnnnnnnnnnnnnnnnnnnnnnnnnnnnnnnnnnnnnnnnnnnnnnnnnnnnnnnnnnnnnnnnnnnnnnnnnnnnnnnnnnnnnnnnnnnnnnnnnnnnnnnnnnnnnnnnnnnnnnnnnnnnnnnnnnnnnnnnnnnnnnnnnnnnnnnnnnnnnnnnnnnnnnnnnnnnnnnnnnnnnnnnnnnnnnattttccggtgaagggatgccaattgagtccccttgccaatgagtggctccgccactgctttcggcataagtttacttgtgggaggtctactttcctacttttcaagttccttacttcacttaggaaatttttcaaggaatttagggtgttcaaacttgaaagaaatgaaaaaatctccaataaattaaagagtgttcaatatatatatatatatatatatataaagattaatattttacctatataatcagtgtaattttttgatgaagggtgatcaattaaccatcattgattgttacttaaattttattgtatcgtatcgttaaatccgtcgttacgtaacgacgaaaagtactactttgtgtaacgaccaatttggtgtggtctcatcgttaccttgtcttttctctcatttcgcccttcattataattaaattattttattttatcttttaccctgcttctttatatagtaataattttattccgtgtcataatttttctttatgatattgcaaatgtattcttcatattgctggtacttgatatcatgaaacgacgacaaacgatacaatctattcaaacattgtatttatcaaacaatacagtacaatataatacaatacaatatatatacactgatatcgcaaaaaaaattatttgctataattagtaacttgaaaagtggaacagacaacctaataaaacatgtttgctgtctacacttgatatttgacaggatgaaatgaagcagcttgctaagagtgaaaggatggcaattcatgtatcaaacatagcaaatttgattcttttcattgcaaaaatctatgcttctattgcaagcagatctttggctgtgattgcatcaactttggactctctcttagacttattgtctggatttattctgtggttcactgtttatgctatgaaaaaaccaaaccaataccactatccaattggtaaaaagagaatgcagcctgtggtgagtttcaaatataatgccacattttgatatttattacatgcattttatactttgtgtcagtgtgcagtgtgattttaagatttatacttgtaagtaggggtggcagacggtcgggccgggtcgggtatgagcgagccaaaacggataatttaaaaaaatggacaaattatccgccccgacccgtatttgaaatggataaaaacgggtttatccggcgtatatggatatccatattatccctggcttcttaaatatgatcagtacatatgagagaattctttgtcttccaaactttgaggaactccaatttgaagctttacaatgtataagctaaacatattagttatccatttggttaaccattttctgagtggataatatggttctttatccatattcgacccatttttaaatggttcattatccaacccatgttttaatggataatatggatggataactgtttttttaaaccattttgccaccttttctggtaagtaaactggcctttatacacaattaaaagaagcaaaacatctaccctcctcttcatacttaaagattgacaaaagattggagttaacttatatacattaatttttatattatttttgctgtaataggttgtgtaccatcccttataggttatcatatcatgttaccggtatcaaaagttactttttttgtcaattaacttcataattaatgtactaattatttacattgtccgttagagcagttaagtatactatttgtgtattttgtcctattattttatatttgaagttatcaaattagggttactatagatagttacctgtaattatatgccattattataatttgacagtgtaaaaaatttctaaccgctcggtgtacacaagctaagctctaaatgaaaaggtagccaaaactaacattttaattatcatatcaaaatcctttatttccttgtttcttcttaattaaagactaccaacaacaacaacagcaacaacccagtgtaattccacaagtggggtctggggagggtaatatgtacgcagaccttacctctaccccgagggacagagaggctgtttccaggagaccctcgcattctttaacattttatcatatcatatttacagggtattattgtcttcgcatctgtgatggcaactcttggattacaaatactatttgagtctggtaaggaactcatatataaggtatgtgactcagttttctgaaggattctatactaggaatagatttaaacttatagttttaaacctatcaaggcatttctgtaatctataaaaaacttctttaaggttaaaatgaaaatttaaggctaaattattttcaactttggatatgtgtcattattttttggacagacgaataaataatgagtgtcacataaaatcaaataaattgagtaattggtaacctggtaaacatgataattgacttactatcacaagttaaactacagttatatcataaaaaaatattttgtcagtgtatttatcttaaatttatgcatagttaaacctctctataacaatctcgtttatttcgaatatttttggatgttatagcgaaatgttgttatagagaatatatattataacataatttaaaaattggttccgaaaaagtttggcttttatagtgaggtgttgttatatagggatactgttatagagaggtccgaccgtaaaagtaattgaatttcactagtaaaatgcttaatgctccactctttaacaccagatttattgtttcttctggtttaatgcttatgatcatcagtctcgtcctaatacggattctgagaaggaaaaatggatgattgggatcatggtctctgtcactgtggtaaaatttctgctgatgttgtattgtcgaagattcaagaatgaaattgtaagagcctatgctcaagaccatttctttgatgtcattaccaactctgttggattagtgactgcagttttagcaattcgattctgctggtggattgatcccatgggagctatattggtgagttcacaatcatcacttatacttcttttgtttttatctctacttttctagatggcagtccggtgcataaagtattgtaagtccacgcaagatccgaatgagagtcgcacccaaagagtatgacgtagacatcttaccctaatgcaaggattagtggttgcttccacggctcgaacctgtaacctttaggtcacatggagagaacttgcacatatatagtgatgtttgcatcaactggcgcacaactcaactatttcacttagtacatgttatctctcactaaaaaatttaccggacaccttgttactcaccaaggcttaggcgtgtggaataactcgtattttttgtctctactagtaatggaatcctaatttcaacctttataccaattttattgaccactaggtcatactcgtggatgcatcgtgcacacacatacgacactacatctgtctcaatttactaggcactatttccttttttttcttttgtcctacaagattgacatctttatagctttagaaactccaaacatttatttatatttttatatcaagattgacacctttatgtacgtatatatggtattactgacttatatattaagcatatttaacttctgtgtcagttatctcttttatttcttaaacttcatgtctagtcgtgctaaaccaattgtggtggacgactatcactaaatgaatgagcaaataaaatgagtagaaaatttcaaagatatccctccaaattttccattattattaacgataacattatgtatttgcagatagcactatacacaattggcacatgggcaaagacagtaatcgaaaacatgcgatcactcatcggaagaacagctccaccagaatttctggcgaaattgacatatcttatatggaatcatcacaaagagataaagcacattgacacagtgagagcatacacatttggtgcaaattactttgtggaagttgatatagttttgccagaggacatgcttctaagccaagcacataatattggtgaaacattgcaagaaaaattagagcagcttcctgatgttgagagagcttttgtgcatgttgatttcgagttcactcatagaccagagcacaagactatggtctaatgacataaataaactaggtaattaataattaataattagtttgagctttaactttattctttggacactgtttccttgcacctaaagtagtaacttaccaaaaaaaaagttctttaatgtggagaacccaacaatgttgaaacttgttgaatttgcattctcaaaatttatgtaacctaatgtttatttttaactcaagatgcctaatgattcatgaacac

SEQ ID NO: 11 - DNA, 1200 bp, Nicotiana tabacum
atggagatcgttggcagcaacggcggtgatcatggcggcgccacccatcagccggtgccgttatcttcctcttcaccgtcggcgtcgtggaggctgaatataggggagtttcgtgtccctgaatatggcactggtgatcatcgtcaatctttcagtttacgtcgactcttgcgtcgcccttctaaaaaacaaggcaaagtagctgaatattacgagaagcaagaaaggttgcttgaagggttcaatgagatggacactgttcatgaatctggctttttacccggaagtctaaccgaggatgaaatgaagcagcttgctaagagtgaaaggatggcaattcatgtatcaaacatagcaaatttgattcttttcattgcaaaaatctatgcttctattgcaagcagatctttggctgtgattgcatcaactttggactctctcttagacttattgtctggatttattctgtggttcactgtttatgctatgaaaaaaccaaaccaataccactatccaattggtaaaaagagaatgcagcctgtgggtattattgtcttcgcatctgtgatggcaactcttggattacaaatactatttgagtctggtaaggaactcatatataagtctcgtcctaatacggattctgagaaggaaaaatggatgattgggatcatggtctctgtcactgtggtaaaatttctgctgatgttgtattgtcgaagattcaagaatgaaattgtaagagcctatgctcaagaccatttctttgatgtcattaccaactctgttggattagtgactgcagttttagcaattcgattctgctggtggattgatcccatgggagctatattgatagcactatacacaattggcacatgggcaaagacagtaatcgaaaacatgcgatcactcatcggaagaacagctccaccagaatttctggcgaaattgacatatcttatatggaatcatcacaaagagataaagcacattgacacagtgagagcatacacatttggtgcaaattactttgtggaagttgatatagttttgccagaggacatgcttctaagccaagcacataatattggtgaaacattgcaagaaaaattagagcagcttcctgatgttgagagagcttttgtgcatgttgatttcgagttcactcatagaccagagcacaagactatggtctaa

SEQ ID NO: 12 - protein, 399 aa, Nicotiana tabacum
MEIVGSNGGDHGGATHQPVPLSSSSPSASWRLNIGEFRVPEYGTGDHRQSFSLRRLLRRPSKKQGKVAEYYEKQERLLEGFNEMDTVHESGFLPGSLTEDEMKQLAKSERMAIHVSNIANLILFIAKIYASIASRSLAVIASTLDSLLDLLSGFILWFTVYAMKKPNQYHYPIGKKRMQPVGIIVFASVMATLGLQILFESGKELIYKSRPNTDSEKEKWMIGIMVSVTVVKFLLMLYCRRFKNEIVRAYAQDHFFDVITNSVGLVTAVLAIRFCWWIDPMGAILIALYTIGTWAKTVIENMRSLIGRTAPPEFLAKLTYLIWNHHKEIKHIDTVRAYTFGANYFVEVDIVLPEDMLLSQAHNIGETLQEKLEQLPDVERAFVHVDFEFTHRPEHKTMV

SEQ ID NO: 13 - DNA, 6329 bp, Nicotiana tabacum
aagtactaacgtaagcgagtgtgcgtggtttcttgattggacggacggtgggtgagtggtacggatcctttgcattcccattgtccatattcatgccgtattcctaattcctaataataactattccagtataaacagtattcaaagttccaacgaagttcataattaaccagcagctactcatctaaacatggaaatcagtcgcagtaatgatagtgtcacactggacgacagttttaggacggagttgctgtctcccgctgctcaggcggtggttgatcattccatgactttggggccgacgtggaagctcaacacaactgacttccatcttccccaacgccgctcctctgatcatcaatctttcagtttcctccgtctcctacgagttttcagtaattcctcagctcatgccattagcatttacttttcaagtactcctgtttattttacatgacatgttggagtttttttttttttttaaaaaaggaaaactttttgcatatattattctagtgcctatattccatgttaatctattattttttggggagtcaaataatattttttttaaccacattttttacaaatactttttaaatattttggaaaattaactatggtaatttatagtagtagttttgatgtaatttctaaatatgtaaatttaatttcaaaaagatttaaaattttatgtgcaaattcatactaaatattaattattttgatcctaactattttctccggtccactttaagtgatttttttggccttttttgtggtctacaatatctgattgtttcatatattaagaatgaattaacttcttctttccaaagttgtctttggagtaaagaatctaggagtagtttgttatatttctaatgaacaaattaaggttaaaatgattaattttattgttaattaattctaaaaggtgaattttttaatatgtgtgaaaagagtaaaaaaaaatacttaaagtgaaccggaggaagtactattaagaacttgccattaattgaaaatttaaagctaaagagttaccgtatacaaagatgtatccttttagaccatctccgactctaacatcaaatttcacaccaaatttactccaaccattacaccattttttacactaaaaagaatatttcttctctctcttctatattatattattatcttctatttaaattttattttttatttccttcaaacaaattctatcttttttttttccatattcatcatatataattcacattcaccacttatataattttttttccatattcaccatatataattctatctttagcaacattagatatcttacatttgcattttttatttttaaataatggttatgtttctttttatacaattataataataataaaattaacttataattttatataaatataatatatacaaaaattaaaatatcaaaaaaatagggtataaaattaaaattataaatatcttaatataaaaattaattatatacacaatatatgataaattaaaagttcaaaaaaataaaaaaaataaaaaagatgaataaaataataataaatcaaatttggtgttgatgaatagtgtcgcaccacactatttacgcactataatggtgcaagatttggtgttccattggagcaaaaaaaaaaataccaaatttaaattttgtgcaaaaaatagtgcacctttgaagatacccttacacttaaatgtttgttatttttctttaggatatctgaagcctttgaaactcgatcagtttccctttgaccctttaatttgtaaccttagagtattctagtgttattattataatatctaacaactctttctgatcatgactattacctaacttattgattgttaatactatcgtctttcaagtggttcattagcattaccaaaacaaaaaaaatggttctttagtttctgaatatagaatattggagtttgatattttctgggagttgaaggctgaagggtgaaattacaatcttgtttctaatagtactttacttaaagtttcaattcttgtctgtagcagaatattattttgttaattttccttcttccactctagcaattttaattggtttaagaggggaaatggtcaaatattagcgccttattatttatttacatcttccaactaatggaagaggaaaacgggtagatggttttattcaaatcctttactatctttaattatgtgggacaagcacagagttacgattttgaatcactgaaaagagaattgcttggcaaagaagaattttgaaaagttgtatctaaaaatttagtaaatacaaaatcataaaaatttaaatactccgagtctccaagaacagttgtgcgggatgcacaggatcatgtaacatattctgaagcttgtattgctgatttttcatactaaggtgtcgtttggtagagatattaaaataaaaataaaaataatgcaagcattagcttaatttgtgcattactaatccctggtttggtacattttttcaacatatgtgtattagttatacctccgatttggtattatccaatgtataactaaaacataacaaactatggtattaacaatgcaagagtttttaatacttgtataaacatggttaaagacataactgcccctcaaatccctcaaaacctattccaaatatttttcgccatatttttgtggagggtatatttgtaaacaatcaattttttaagaaattatgcaatgccttaatataccaaactaaacagtggataagaaataatctcaatataattaatgatagtataactagtctcaacattattaataccatcgttactgatacaccttattcaacattatttttaaacctcctaccaagcgacccctaagaatgttttatttgaagtaacttcaaatcatatacttgacctcattcttgtaaaaaaaatttgtttgttgagaaggtaaacttgttaaagaaattagtcacatttcttcccttttgcatataaaactacggatatcaaagagtttttggtgttttattttgttcaaggttattagtcctgtttgattttgctctacaactctacagttttctttcatatttactctcttaaaatttaagaaggcgccggtaatttaactaccaggttgaggactacctagcagcccgcggatggatagggtgggggaagcgcgaaggggatggatgtctgagcggttgaaagagtcagtcttgaaaatcaaagtatttatagaataccgggggttcaaatccctctccatccgcgagatcataagttggtctcttgagttatatatagataagaagatattgggtcgactggactgatatgatagatggaatggtagactgaagttgttacttattttcagttaaggaacaaaaattcacttgatactctgtaagggtgatatgcaaagcaggcaacaaaatccatctttgttggaccaaaatatgctcttaattacttgtaaatgttccctgaccaaatgctttgattgctgaagctaatagtttaaaaacttatctttcttggactgaaataggctctcttatttggaatggacatattcaagaatataagttatcatacccttaggaatgatatactaagtaggtgatttcagataatcagattcattgtttcagataattaaactttccatttccgtcttcactttcttgatcacttgatggaatcgtgttaatcatgtatagggaatcagagaaaagttgctgaatactacaaaaaacaagaaaggctgcttgaaggattcaatgagatggacacaattaatgaatgtggttacttacctggaaatctaactgaggttggtctatgagattggcagattcttatcagtttaatcatcacaattttttagtcgtcaaaataactttcttttctttgttgcactgtcaaccaatatatacaatcacctttagtgaaattcgtgtgtttgtggatcaacttgtgtttatcttctattgttgttcataaagctataatttgcaatttcaaatctcagatgttgtttttcaggatgaattgaagcaacatgctaagagcgaaaggatggctattcttgtgtcaaacatagcaaatatggctcttttcattgctaaaatctatgcttctattgacagcagatcactggctgtaattgcgtctaccttagactccctattagacctcttagctggatttattctgtggttcacttctcatgcaatgaaaacgccaaaccaatactgttatccaattggaaagaagagaatgcagccagtggtgagtcttctactgttttaatttcttccaacgaacacccttgtttcagggtatttctccgaaattaaagtaaaaagaagaaaaaaaacatatcccttcagctcccaagaaagaaaaagaaaagatgtcttcgccaatttctgtttattgtttgaactgatctgctgcaatattttcagggtatagttgtttttgcatccgtaatggcgaccctgggattacaaatattgttcgagtctggtaaagaactcataactaaggtatgtaacttggttctcttcaagtgtgttgtgagatggatgtgtcatgtgtgagctggtacaaggttgaatttccaaatacatgtattttgtaaaattaatgtcgaattgataaagaacttccccagaaagtgcattttggcagcaaaatataaaatatcttagaaggttctgataccatgttaagcaaaataaattttggacctaattcaacacaacagttcactcatgagatgaggatttttcgaggtcatataaagcgattagagctcaacctgtgtgggatgctaaaaatattcataattcttcttcccctaaaagtcagtagcctggagttctctctaggtttttgtacttctacaattgattttaaattatttacagagttgaaatggtagtactttgtcccaagtaattcattcttcacattgatggacatttatattgttgaaaactagcactagcttttatgttaaatgagatagattttatgtacgatgtgagtgctttaggaaaagtagttgatcttaaggatcaaaaggaaagaccaaaattagaagctgaattgctgctaaaaggaatttgcagtagcatgtacaagttaggccctctaatctatgtataatggtaaactagctgtttgtgctctaattgaaatcgactagtcttgatacgaggatgcaacatagattaataaggactattcctacacaatacattttgtattgaaggactgaactctaatttgccggaatttcattttgtaatatgcctgacacttaacctcaatttgtttttctggttccatgcttaatgatttgtttttctggttctatgcttaatgattagtctcgtcctgatatggaccctgagaaggaaaaatggatgatcggaattatggtttctgtcactgtggtcaagtttatgcttctgatctactgccgaagattcaaaaatgaaattgtaagggcctatgctcaagaccatttctttgatgtcattaccaactcaatcgggttagcggcagcagtcttagccatccatttctattggtggattgatcctactggagctataattgtgagtttagaattacaacacacgaactctttaatctatataccttgtctgttatcgcaattgagatatttttgcattcctatggacaactgatcatcctttgttatgtgtttcagatagcactttacacaatgagcacatgggcaaagacagtgatggaaaatgtgtggtcacttattggaagaacagctccacccgaatttctagcaaagttaacatatcttatatggaatcaccatgaaaggatcaaacacattgatactgttagagcatataattttggcatacaatattttgtggaggttgatatagtgctgccggaggacatgttcctgaaccaggcacataatattggtgaaacgctgcaggaaaaattggagcaacttgttgaagttgagcgtgctttcgtccatgtagattttgacataactcataggctggaacataagtctatgatcaaatgacgtcaaattgacatataatttttagaatgacggccgcttaattcctgtttaattataccattgtatttcctatttgttactctctatattggatcagatgagctttatcatccgtcccagctgagagctttatcgtcctttggtgtgtccctcacctctctcttttgaggcctgtttcctctactgtcacttcttt

SEQ ID NO: 14 - DNA, 1224 bp, Nicotiana tabacum
atggaaatcagtcgcagtaatgatagtgtcacactggacgacagttttaggacggagttgctgtctcccgctgctcaggcggtggttgatcattccatgactttggggccgacgtggaagctcaacacaactgacttccatcttccccaacgccgctcctctgatcatcaatctttcagtttcctccgtctcctacgagttttcaggaatcagagaaaagttgctgaatactacaaaaaacaagaaaggctgcttgaaggattcaatgagatggacacaattaatgaatgtggttacttacctggaaatctaactgaggatgaattgaagcaacatgctaagagcgaaaggatggctattcttgtgtcaaacatagcaaatatggctcttttcattgctaaaatctatgcttctattgacagcagatcactggctgtaattgcgtctaccttagactccctattagacctcttagctggatttattctgtggttcacttctcatgcaatgaaaacgccaaaccaatactgttatccaattggaaagaagagaatgcagccagtgggtatagttgtttttgcatccgtaatggcgaccctgggattacaaatattgttcgagtctggtaaagaactcataactaagtctcgtcctgatatggaccctgagaaggaaaaatggatgatcggaattatggtttctgtcactgtggtcaagtttatgcttctgatctactgccgaagattcaaaaatgaaattgtaagggcctatgctcaagaccatttctttgatgtcattaccaactcaatcgggttagcggcagcagtcttagccatccatttctattggtggattgatcctactggagctataattatagcactttacacaatgagcacatgggcaaagacagtgatggaaaatgtgtggtcacttattggaagaacagctccacccgaatttctagcaaagttaacatatcttatatggaatcaccatgaaaggatcaaacacattgatactgttagagcatataattttggcatacaatattttgtggaggttgatatagtgctgccggaggacatgttcctgaaccaggcacataatattggtgaaacgctgcaggaaaaattggagcaacttgttgaagttgagcgtgctttcgtccatgtagattttgacataactcataggctggaacataagtctatgatcaaatga

SEQ ID NO: 15 - protein, 407 aa, Nicotiana tabacum
MEISRSNDSVTLDDSFRTELLSPAAQAVVDHSMTLGPTWKLNTTDFHLPQRRSSDHQSFSFLRLLRVFRNQRKVAEYYKKQERLLEGFNEMDTINECGYLPGNLTEDELKQHAKSERMAILVSNIANMALFIAKIYASIDSRSLAVIASTLDSLLDLLAGFILWFTSHAMKTPNQYCYPIGKKRMQPVGIVVFASVMATLGLQILFESGKELITKSRPDMDPEKEKWMIGIMVSVTVVKFMLLIYCRRFKNEIVRAYAQDHFFDVITNSIGLAAAVLAIHFYWWIDPTGAIIIALYTMSTWAKTVMENVWSLIGRTAPPEFLAKLTYLIWNHHERIKHIDTVRAYNFGIQYFVEVDIVLPEDMFLNQAHNIGETLQEKLEQLVEVERAFVHVDFDITHRLEHKSMIK

SEQ ID NO: 16 - DNA, 6780 bp, Nicotiana tabacum
tgcattcccattgtccatattcacgccgtattcctaataactattctagtataaacagtattcaaagttccaacgaagttcataattaaccagcagctactcatctaaacatggaaatcagtcgcagtaatgagagtgtcacactggacgacagttttaggacggagttgctgtctcccgctgctcaggcggtggttgatcactccatgtctctggggccgacatggaagctcaacacaactgacttccatcttccccaactccgctcctctgatcatcaatctttcagtttcctccgtctcctacgagctttcagtaattcctcagctcatgccattagcctaattttcttttcaactactcctgtaatcacatgttggatttaaaaataaaaaaaaaataaaaaatcttttttgcatatattatactagtgcctatgttccatgttaatctattattatttggggtgtcacataatattttctttaaccacattttttacaaatgttttctaaatacttattttggaatattaattatggtaatttatacagtagtagtttttatgtaatttctaaatatgtaaatttaaaattactagttaatttgatcctaactacaattaagtacttgccattatttgaaaatttaaagctaaagagttaccgtatacaaagatgtatccttttacatttattttagtgtttgttatttttgtttactatgtctgaagcctttgaaactcgttcggtttccctttgaccttttagtttgtaaccttagagtattctagtgttattattataatatctaactactatttctgatcataagtcatgactattacctaacttattgatagttaatactatcgcctttcaagtggttcattagcattaccaaaaaaagtagttctttagtttctgaatatagaatatcggagttggatattttcggcgagttgaagcctgaaaagtgaaattacaatcttgtttctaatagtactttacttcaagtttcaattcttgtctgtagcattgtagtggagcagaatatcctaatgtgctcaggagatcttattaacaaagttttgaatcgattagatatgatgggcacttcaaagggatcaaacttgctaaataaactggcaactttataattcaaacaccgatatgtaaaagctcatgggccatgtcgcgacttcattttgtcctaaaagttcaaagttcctggtcagatttttcttttattattttgttaattttccttcttccgctctagcaattttaattggtttaagaggggaaatggtcaaatattagcgccttattgtttatttacatcttccaattaatggaagagaaaaacgggtagatggttgtatatccaaatcctttactttctttaattatgtgggacaagcacagagttacgattttgaatcattgaaaagagaattgcttggcaaagaagaattttgaaaagttgaatctaaaacatttagtaaatagaaaatctcaaaaatttaaatactccgagtctccaagaacaattgtgtgggatgcaattgtgaagcttgtattactgatttttcatactaagggtcgtttggtaggggatattaaaaaaaataatgcaggcattaactttgtgcattactaattggaaaaatgacaatgtataggcgatgtaaaaataatagacgaaaaaatgtataaaatttgtatatttttttgtatatatatacattttgtattttgtatatatatacattttgtatgttatatacaaaaattatgcaaattttatacacttccggctaccagatgtaaatagtttctagcgcgggctaaaagtgataataccccttactaatcccttgtttggtacattttttgtattagttatacatcccatttagcattatattatgtataactaaaacatagcaaactatggtattagcaatgcaaaagtttttaatacttgtataaacatggttaaagacataactacccctcaaatccctcaaaacctattccaaatatttttcaccatatttttctagagggtatatttgtaaacaatcaattttttaagaaattatgcaatgctttaatataccaaactaaacagtggataagaaataatctcagtataatgccggcataactaatccagcactactgatgcaccttattcaacactatttttatacctcctaccaagcgacccctaagattgttttatttgaagtaacttcaatgttttatttgaagtaacttcaaatcatatacttgatctcattcttgtaaaagtgtttttttttttggttgagaaggtaaacttataaaagaaattagtcacatttgcttccctttggcatataaaactacggtgttccagatattaaagagttttgggtgttctatttagtccgcggttattagtcctgtttgatttttctctacagctctagatttttctttcatatttactctcttaaaagttaagaaggcgccgataatttaactaccaggttgaggaccacctgtcagcgcgcggatggatagggtggatgtctgagtggttgaaagagtcggtcttgataaccgaagtatttatagaataccgggggttcgaatccctctccatccgcgagaacataagttctctcttgagttatctatagataagaagttattgggccgactcgactgatatgatagatggaatggtagactgaagttgttacttattttcagctaaggaacaaaagttcacttgataatctgtaagggtgatctgcaaagcaggcaacaaaatccatctttgttggaccaaaatttgctcttatttacttgtaaatgttcccttaccaaatgctttgattgctgaagctaatagttcaaaaacttatctttcttggactgaaattggctctcttatttggaatggacataattcaagagtaatgtgttataagctaatataagctatcatacccttaagaataatgcttaaagtaggtggtttcagataaccaaattcattgttttaggcaattaaagttttcactttgttttttaatctaacctgactgcttcatggaatctctgtaatcatatatagggaatcagaaaaaagttgctgaatactacaaaaagcaagaaaggctgcttgaaggattcaatgagatggacacaattaatgaatgtggttatttacctggaaatctaactgaggttggtcttttcctcacttgccacaactaatgaatgtggttatttctgttctttgttgcactatttccaccttcaaccgaaacaatcacctttagtgttcagaaattcatgtgtctctggatcagataagactacttgtgtttatgttctttttcttcttggagaaggtgatttcttgatcaatctctgcctcttcaataactacaatgtttttccatgttaacccgagtgtatattaggactttcagtcagattcttaggtttcttgaatcttgatctctgttaatattcgtaataagaatcaacaaataatgttgtttttcctgtctaccaatgattattaatgccaggatgaaatgaagcaacatgctaagagcgaacgaatggctattcatgcgtcaaacatagcaaatatggttcttttcattgctaaagtctacgcttctattgacagcagatcgctggctgtaatttcatcgaccttagactcgctattagacctcttatctggatttattctgtggttcacttctcatgcaatgaaaacgccaaaccagtaccgctatccaattggaaagaagagaatgcagccagtggtgagtcttctactgttttttcttccaaggaacacccttgtttcagggtatttctccgaaattagagtaaaaagaagaaaaaacatattcctttagctccctagaaagaataagaaaagatgtctgatcaccaatttatgtttatatatctggataatacctttgtgccttctgacagtttcctcaagaattaacagcttaaagggtagcacgtaaaccagaatatcttgcttgtgtgcaatattttttacattaatatggtttattgtttgaaatgatctgctgcaatattttcagggtatagttgtttttgcatccgtaatggcgaccctaggattacaaatattgttcgagtctggtaaagaactcataactaaggtatgtaacttggttctcttcagctgtgtcatgagatggatgtgtcatgtgtgagctggtacaaggttgagtattgtgacttctaaaaataatgtcaaattgatgaagaacgtttcctcaaatatactttgagagcacaatatccttactggtcttttaataatccatgttaggcaaaatgaattttggacctaactcaacagttttgctcaagtgatttcgcaatatgtgcatgtattacaaaagtttactcgggtgagatgaggatcttctagggccatataaagagactacagcttatgccctcaatcagtgtgggactcttaacaatattcgtatttccttcttcccctaaatatcagcagcctagagttctctccggattttgtacttctatagttgattttaagttgttttgtagtagagtttacggtagtcctttgccctaagtaatccctttcttaaaattgatggacaatttatattgttgaatattaccactagcttgtctgataaatgaaatatgtcgtacaatgcgacaaaagacctaaaatagaagctgaattgctactaaaagaaagttgcagtaacacaagatatgccctctaatccatgtataaagatgaactagtcgtttgtgctctaactgaaaacaactagttttgatactacatatgaagcacagattaataaagattagtcccacatgatacatttcttattgaaggactgaactctaatttaccgcaatttcactagtgaaatattgtaatatgcttgacacttaacctcaatttgtttttctggttctatgctttaattattagtctcgtcctgatatggaccctgagaaggaacaatggatgataggaataatggtttctgtcactgtggtcaagtttatgcttctgatctactgccgaagattcaaaaatgaaattgtaagggcctatgctcaagatcatttctttgatgtcattaccaactcaatcggattaatggcagcagtcttagccatccatttctactggtggattgatcctactggagctataattgtgagttcagaataacaccacatagttcttttatttgtataccttgtctgttgttgcaattgagatgtttttgcatttcctatggagaactgatcatcctttgttactgcaacagctttttaaagtagtagtatttgtttagtttaagcaattaattagcattttgaagaataaagtagcatatctttattaattaatcttattagtctctgttgtgtgtttcagatagcactttacacaatgagcacatgggcaaagacagtgatggaaaatgtgtggtcacttattggaagaacagctccacccgaatttctagcaaagttaacatatcttatatggaatcaccatgaaaggatcaaacacattgatactgttagagcatataactttagaatactattctaccactggaccattggtatattttattttaagactgtcttttatttgatttatacactttaattgtattttcgtatgaaaataaccgatcaaagttggtcagttttttaaaattatcaaccgaattaaccgaccaactttggtcggtttttttaatattaatttttatttattttaattgaaaaaccgaccaaagttggttggtttcttgaaaaataaattttgcgggactcaaaaatcgtttcccgcatttttgcgccaaagaaaaacgaccaaagttggtcggttttgtaaaacaaaatttaaaaataaaatattttgaaaaaccgaccaactttggtcggttttttggccggttttttgatcgaccaaagttggtcggtcgaccttggtcagtttttgccgaaacacaatctatgggagcgagttgaatgtttgtcactagatgatatttaatgaagaatattgcctagtattaaataggcagccgttgcagagaatttgggcattcatgacctgtcgtttcatgttcatcaatgactccttttattgtaatttaagaggggcttgatcctaggatcttgtttcctaggtatagctataaatagtagcttcaacaaccattgtagacagagaaaatatctcgcaaaaacttatgctacactttattctcaagctaaacaatacaaatttactttccatatgatattgctcttatttctgtcctcggaagcattgctcccggagctaggcctgccatttcctttggttttaacgctaagtcttatttttaatctaatttacttattattttgggttaaatcagtttgcttgtctataaaccacataacgaatacaactgtaccgttttacaggtaaacagtttggcgccccaccgcgggtcttagacaactgcataattaagttgatccttgcatatattactaactcgtttgattctttatttcttagaaaaaatagcacacaacattgaggcacaccaaaatctacctcaacatgaggattcaatcagtgatacccgcaatgagagagatgtggaaactccggtccatggcagacaatatcgccgacacgtgcggg

SEQ ID NO: 17 - DNA, 1102 bp, Nicotiana tabacum
atggaaatcagtcgcagtaatgagagtgtcacactggacgacagttttaggacggagttgctgtctcccgctgctcaggcggtggttgatcactccatgtctctggggccgacatggaagctcaacacaactgacttccatcttccccaactccgctcctctgatcatcaatctttcagtttcctccgtctcctacgagctttcaggaatcagaaaaaagttgctgaatactacaaaaagcaagaaaggctgcttgaaggattcaatgagatggacacaattaatgaatgtggttatttacctggaaatctaactgaggatgaaatgaagcaacatgctaagagcgaacgaatggctattcatgcgtcaaacatagcaaatatggttcttttcattgctaaagtctacgcttctattgacagcagatcgctggctgtaatttcatcgaccttagactcgctattagacctcttatctggatttattctgtggttcacttctcatgcaatgaaaacgccaaaccagtaccgctatccaattggaaagaagagaatgcagccagtgggtatagttgtttttgcatccgtaatggcgaccctaggattacaaatattgttcgagtctggtaaagaactcataactaagtctcgtcctgatatggaccctgagaaggaacaatggatgataggaataatggtttctgtcactgtggtcaagtttatgcttctgatctactgccgaagattcaaaaatgaaattgtaagggcctatgctcaagatcatttctttgatgtcattaccaactcaatcggattaatggcagcagtcttagccatccatttctactggtggattgatcctactggagctataattatagcactttacacaatgagcacatgggcaaagacagtgatggaaaatgtgtggtcacttattggaagaacagctccacccgaatttctagcaaagttaacatatcttatatggaatcaccatgaaaggatcaaacacattgatactgttagagcatataactttagaatactattctaccactggaccattggtatattttattttaagactgtcttttatttga

SEQ ID NO: 18 - protein, 366 aa, Nicotiana tabacum
MEISRSNESVTLDDSFRTELLSPAAQAVVDHSMSLGPTWKLNTTDFHLPQLRSSDHQSFSFLRLLRAFRNQKKVAEYYKKQERLLEGFNEMDTINECGYLPGNLTEDEMKQHAKSERMAIHASNIANMVLFIAKVYASIDSRSLAVISSTLDSLLDLLSGFILWFTSHAMKTPNQYRYPIGKKRMQPVGIVVFASVMATLGLQILFESGKELITKSRPDMDPEKEQWMIGIMVSVTVVKFMLLIYCRRFKNEIVRAYAQDHFFDVITNSIGLMAAVLAIHFYWWIDPTGAIIIALYTMSTWAKTVMENVWSLIGRTAPPEFLAKLTYLIWNHHERIKHIDTVRAYNFEYYSTTGPLVYFILRLSFI

SEQ ID NO: 19 - DNA, 5390 bp, Nicotiana tabacum
catttttagttccactttccttgttcaaaaaagttccgccatataaagcctctacaactacccacccaaagaactccaaattacataaaggtccctggagttcatcaaatttacgcactttaccactcccctgcggctccttcaagtaggtgcctccagtttttttacctagtgttttcaactgtttttttccctattttccggtgaccggaaaatgttggaagtagtacctcttcacggcggcgatcacggcgccggcaccgaagaggagcttttattgctggagacaaacaatgccgaccggtcatggagattaaacttcgacgagttgcggttgtcgtctgaatccaaagagaagcctccacgtggcctccatgattgccttggagttttaagtacattctccacctctctatgcgacgtcgttttttgttattctctgctaatttcttaactagttgcattaggttgacgtaagagagacaccacttgaatagagcggaatttatataaaggaattatacagctgattcctattaaatacttgactgatattctgttgtgcgtaggattttactaattgcggaaattttcaaacactaagcttactcctttagttggttaattagtggggactctttttatacttttcagtttcagaaagtattttcttgccacgtgggttcaattttctgaagaacaaaatgattcttgtatggatggtgtaaatttgctaaagatgttaagctatattcactttttattgttctctggacaattgaacatgcttatgggcagttcactggtttggagcaaattggcatatatttgtatgtagatggatgattctttttggataagttttagatggataatttttgttataagaacatgagctttagagctcaaatttaatgcgtttcagcacttcagtttactgaaaataagaagggaactttagctgagtgcgctcgccaggtaagtttatgtggttaggtcagtgtaataaaaccagaggcagacctatgttaatatgtgagggtgcactggcaccctgtagtttccgatgaaactatatggagtatataaaattcttataacactactatgtattttaggtggcaattgcaatgacaaagtagcggtaggaggatttgttaaaatatgtgtttttacctgagttgttgtcttctcatattgaatacttacataattgaaccaaattaatgcaataccatcaaacgaacttaatgcactttagatgatatgacttgttcgaatctttagtgcaccggcaaccttcacttggtgtgtgtgtgtttgcatgtgacatgagccagtcaaaagattgttccaagaggctacttttgcattctgttgaattgttaagttgtcatatgagaatgtatgtttggaattgataatggtactttgacaatttataatcggctttggtatgagtggtggactctaaatgcaggtcagccttggttctcatcaactctttggtttagtacttataggaggctatagtgctatatagagatgcatgtagaatggatttactgaatgctttcactgtaagacatggggtgttcttgaagggacggattatgacgctgtgtttttctttggtgcttacaggtcaagaagacaacattgctgagtactaccagcaacaggtagaaatgctcgagggcttcaatgaaatggacgccttgaccgatcgcggttttgtacctgggatgtcaaaggttttgatagcttcttctttatgtataagaccaaccatttgtttcttctctagatgtatcattcttatcttattatataacttgatgacctgatcatctaattaaaaaagaatgttactcaaagcttggactgacaagctcaattaatttgattgcaggaagagagggaaaaaacggctagaaatgaaacatttgccattaggatatcaaatgttgcaaacatggttctctttgccgctaaagtatatgcgtcagtcaagagtggttcattggccatcatagcatccacattggattcgctgcttgatcttctctctggtttcatattatggtttacagctttctccatgcagacaccaaacccatatcaatatcctattggaaaaaaacgtatgcagccgttggttagtgctgctgcttttattcttaagttttttgcatcttctatgccttcaatcgggccaatttgcattctgcacttgtcacttgctattgggctaatactcatgactgcatataataacaatttccttgctttttcatgcgtttaaaaattgtctaacaaggtaattgtactatgcattcttgtcacatttgattctaaagggaccttaagttctgccactgctatttttatgttgtggtcatggtaagccttaacattcgttttgtttgttgatgcagaggcaatttagccttcttcttgagttcaatctctaatcatcacatgttgtagtccaaaaataaaggaataattttcacctaaaagtatggaaccacgagaaattcaaacttaatgcatctaagacaaattaaatgaattaaaacaacatcatatctgatagtaaccatctataaaaggttgaaataaaagaaaagatgtgcagaattttaataatgtcctctagcagacagcttacatgactgcattaaaacctacagagattcaaatcttcagcatctctttctccaatagttgtcttttaggtgtagcctcagtggagaaccacacatgtttctgagatagaaaggtgagagaagatagctgatggcaggggaaggggaaagagagagatgagaccagaagggaaggccacatagattgaagctgatttggcagagagaattgagtgagatgatgaaacactggctgctgtgagtggcagtatagaattagagagggtggggttacggggagattatgaagtgtctattagtaattttacaagatttagttgttttgtttttactgtggagggatgaatatggtccttgtttatgatctgtgatggataccggagcttataacctcccatatgcaccattttctcccacatcaggttaggttgatagccattgcgttcgctctaagtagcgatcctcaaattcaattaattaatcgtattatggtgatgttgatatagacatctagactgtcactcctgatgttacctatcaaaaaaaaaaactatcatctcctagatgtttctattaatccaatgtctgtacataactaaggagggatcctagacttgagttacacagagattcttacatagtctttgttgctgttcatctcttcctgttatctcattttcattatcaaaattgacagtaagcacttgctccgtgaatgtaactagtctgggcatgaatttggtgtagtactcataacagttgcatttagtttggaagcttagagagtagtgctttctagtgtggtggtttgatgattattttgcgtaatatctgtaaataaatacctctgtgaagttttactttggtgctaagtacttaaattgcaatcgtggagatactattatctattcagataactttgacgttctggtttaaatcagttgataattccttaggatactaggatgatcccactgtaagtattatgagcttattttgatatttgagatctttattgaccattatacatccataaaagttcccgtactttggcagaaggagacttttcttctgtttctagagaaccatttgcagaagactgtcatttttcaattacatgatttaaaagatatggttttcttcttccatcatttgttgctaacagaaaaaaagaagtggaaattttgatttagatctgagactctatgtaacttccactatgttgctgaatgttgtgtagaaaaagatctagtctgcaaacaagttttgccctgtatgctggctgatcctatgaagttgacatgattttacttatcttttgatttttcatggaggtagagcaaactgcaggtctatggctatcttcatagtgcatgttgtgtaattcccagtgggttcaaaatgaactgtgttttaactttcagttttacttgtatttctaaatatctggtgataacatcgtacaggcatgaatagaaatattgtatgattgttttctattcttccttgggagctggtccaatttaacttgaaaaatgatacacagggaatccttgtttttgcttctgtcatggcgactttgggactgcagataattctggagtctatgcgtacactaatatctgatgtaagttgtggctcctaagataagtttattgctttattatgttgtattgtctggttgaaaattacatgcatggattcttataattattccttgaccctgtacaacggcaaatgttataaacattgaccttctcacaggagtctgatttcaacctcaccaaggagcaggagagatgggttgttgggattatggtctttgtgactttggtgaaactagttttaatgttgtattgccggtcttttaccaatgagattgtgaaagcatatgcccaggatcatttctttgatgttatcacaaacatcattggtctcattgcagcattgcttgctaactacattaccgactggatagatcccgttggagctatgattgtaagttctatctccctgattctgttccaccaatcaggattggaaagaaaagggaaaagttttaatgtggctgtcaatcctctcgctttaaccaaggttagtggctttaagcaattttccctctgctgcagcttgcattgtataccattcgaacttggtcaatgactgtattggagaatgtgaactctctcgtcggcaagtctgctgcaccagaatacttacagaagctgacttacctctgctggaaccatcacaaggccataaggcatatagataccgtgagggcttatacatttggttcgcactactttgttgaagttgatatcgtcctgcctgcggacatgcctttgcaagaggcacatgatattggtgagtcgttgcaggagaagcttgaactattgcctgagattgagcgtgccttcgttcatcttgactatgaatacagccataaacctgaacatgctcaggcataccaatagtcaaaaggattttgtgacatcttctctagccaatgtacctaatacctctgcatagtgaactctgatatgctgttcgagatcggctaatctggtgattgctctttaaaagaaaatctgggaaagaaaaggctgctatgatctggatgttccctagaacaagtaatatgaattattattttgttaaattttaccttgcctattcatatatataacatgatttctcagtttgcttgctcctggt

SEQ ID NO: 20 - DNA, 1200 bp, Nicotiana tabacum
atgttggaagtagtacctcttcacggcggcgatcacggcgccggcaccgaagaggagcttttattgctggagacaaacaatgccgaccggtcatggagattaaacttcgacgagttgcggttgtcgtctgaatccaaagagaagcctccacgtggcctccatgattgccttggagttttaagtcaagaagacaacattgctgagtactaccagcaacaggtagaaatgctcgagggcttcaatgaaatggacgccttgaccgatcgcggttttgtacctgggatgtcaaaggaagagagggaaaaaacggctagaaatgaaacatttgccattaggatatcaaatgttgcaaacatggttctctttgccgctaaagtatatgcgtcagtcaagagtggttcattggccatcatagcatccacattggattcgctgcttgatcttctctctggtttcatattatggtttacagctttctccatgcagacaccaaacccatatcaatatcctattggaaaaaaacgtatgcagccgttgggaatccttgtttttgcttctgtcatggcgactttgggactgcagataattctggagtctatgcgtacactaatatctgatgagtctgatttcaacctcaccaaggagcaggagagatgggttgttgggattatggtctttgtgactttggtgaaactagttttaatgttgtattgccggtcttttaccaatgagattgtgaaagcatatgcccaggatcatttctttgatgttatcacaaacatcattggtctcattgcagcattgcttgctaactacattaccgactggatagatcccgttggagctatgattcttgcattgtataccattcgaacttggtcaatgactgtattggagaatgtgaactctctcgtcggcaagtctgctgcaccagaatacttacagaagctgacttacctctgctggaaccatcacaaggccataaggcatatagataccgtgagggcttatacatttggttcgcactactttgttgaagttgatatcgtcctgcctgcggacatgcctttgcaagaggcacatgatattggtgagtcgttgcaggagaagcttgaactattgcctgagattgagcgtgccttcgttcatcttgactatgaatacagccataaacctgaacatgctcaggcataccaatag

SEQ ID NO: 21 - protein, 399 aa, Nicotiana tabacum
MLEVVPLHGGDHGAGTEEELLLLETNNADRSWRLNFDELRLSSESKEKPPRGLHDCLGVLSQEDNIAEYYQQQVEMLEGFNEMDALTDRGFVPGMSKEEREKTARNETFAIRISNVANMVLFAAKVYASVKSGSLAIIASTLDSLLDLLSGFILWFTAFSMQTPNPYQYPIGKKRMQPLGILVFASVMATLGLQIILESMRTLISDESDFNLTKEQERWVVGIMVFVTLVKLVLMLYCRSFTNEIVKAYAQDHFFDVITNIIGLIAALLANYITDWIDPVGAMILALYTIRTWSMTVLENVNSLVGKSAAPEYLQKLTYLCWNHHKAIRHIDTVRAYTFGSHYFVEVDIVLPADMPLQEAHDIGESLQEKLELLPEIERAFVHLDYEYSHKPEHAQAYQ

SEQ ID NO: 22 - DNA, 5468 bp, Nicotiana tabacum
catttttagttccactttccttgttcaaaaaagttccgccatatatagcctccacaactacccaccactaagaactccaaattacataaaggtccctcgagtttcatcaaatttactcactttaccactttctgcggctccttcaagtaggtgccgccagttttttacctagtgtattcaactggttttttcctgttttccggtgaccggaaaatgttagaagtagtacctcttcacggcggcgatcaaggcgtcggcgccgaagaggagcttttattgctggagacaaacaatgccgaccgatcatggagattaaacttcgacgagttgcggttatcgtctgaaaccaaagagaagcctccacgtggcctccatgattgccttggggttttaagtacattctccacctctctatgcgacgccgctttgagtgttattctctgctaatttcttaactagttgcattaggatagtaaattagtggagacaccacttgaatggagtggaatttatataaaggatttatacagctgattcctattaatcagtgatggagaaatacttgactgatattctgttgtgcgtaggaagtttactaattgtggaaattttctaacactaagcttacttctttagttgagttattagggggctctttttaatacttttcagtgtcagaaagtattcatgccacgtggattcaattttcggaagaacaaaatgattcttgtatggatggtgtaaatttgctaaagatattaagctatattcactttttattgttctctggacaattgaacatgcttatgggcagttcactggtttggagcaaattggcatatattttgtatgtagatggatgattctttttggataagttttagatggataattattgttataagagcatgagcgttaaagcttaaatttaatgcgtttcagcacttcagtttactgaaaataagaagaaaactttagctgagtgcactcaccaggtaagtctatgtggttaggtcagtgtaatagaaccagaggcagatctatgttaatatgtgagggtgcactggcacccgagtatataaaattcttataaaactactactcatgtattttaggtggcaacctcaattacaaagtagcggtaggaggatttgttaaaatatgtgtttttacctgagttgttgtcttctcatattgaatacttacaaagttgaatcaaattaatgcaataccatcaaaccaactgaatgcactttagacgacatgacttgttcgaagctttagtgcaccggcaaccttcaattccttgatatgcctctgaatagaacaggttaattggtgcgcgtgtgtgtttgcatgtgacatgagccagtcaacagattgtttcaagaggctacttttgcattctgttgaattgttaaattgtcatatgagaatgtatgtttcgaattgataatggtactttaacaatttataattggttttggtacgagtggtggcctttaaatgcaggtcacccttggttcccatcaactctttggtttagtacttatagggggctatagtgagggatttactgaatgctttcaccgtaagacatggggtgttcttgaaggcacggattatgacactgtgtttttctttggtgcttataggtcaagaagacaacattgctgagtactaccagcaacaggtagaaatgctcgagggcttcaatgaaatggacaccttgactgatcgtggttttgtacctgggatgtcaaaggttttgatagtttttatctgcttcttctttatgtataagaccaagcatttgtttcttctctagatgtaatcattcttatattattataagcttggactgacaaggtcaattaatttggttgcaggaagagagggaaaaaactgctagaaatgaaacatttgccattaggatatcaaatgttgcaaacatggttctctttgctgctaaagtatatgcatcagtcaagagtggttcattggccatcatagcatccacattggattcgctgcttgatcttctctctggtttcatattatggtttacagctttctccatgcagacaccaaacccatatcaatatcctattggaaagaaacgtatgcagccgttggttagtgctgctgcttttgttctctaagttttttacattttctatgcctttaatcagggcatttttgcacttgtcacttgctattgggctaatgttgattactgcatataataacaatgttcatggatttaaaagttgtctaacaaggtaattatactatgcgttcttgtcatatttgattttaaagggaccttaaactctggcgctgctatttttattttgtggtcatggtaagccttaatattcattttgtttgttgatgcagaggcaacttagccttcttcttgagatcaatctctaatcatcacatgacgtagtccaaaaaacaaaggaataattttcacctaaagtatggaaccacgagaaatgcaaacttaatgcatctaatagcatgtttggccaagcctttttttgggccaaaagtgtttttttttcaaaaattaaggtgttttttttcaaaaagtgtttggccaagcttttagaaggaaaaaattgtgcttttgaggagacgcagaagtagtttttgagaagcaaaaaaaagtagcttatctccaaaagcacttttctgagaagcacttttgagaaaaatacacatagatgcagtttttaaaagcttggccaaacgctaattactgctcaaaagtgcttttcaaattaattagccaaacacaaactgcttatcaccaaaaacacttttttgaaaagtacttttgagaaaagtacttctcaaaataagctgattttagaagcttggccaaacaggctataagacaaattaaatgaattaaaacaacataatatttgatagtaaccaactataaaaggttgaaataaaagaaacgacgtgcaaactttcaataatgacctctagcagacagcttacatgactgcaataaaacctacagagatgcaaatcttcagcatctctttctccaatagttgtcttctaagtgtagcctcagtggcgaaccacactgagaatgtttgtgagacagaaagagagagagagcagtggctgctgttactgacagtatagaatgagagagggtggggttacaggaagattattaagcgtctattagtaatttggcaaaaatttaggtgttctgtttttactgtggagggatgaatatggtctctgtttatgatctgtcatggatattggagcttctagcctcccatatggaccattttctcccacatcaggttaggttgatagccattgtgctcgctttaagtagcgatcctcaaattcaattagttaatcgtgttttggtgatatgcatatagacatctagattatcactcctgatgttacctataaaaagaactattatctcctgatgtttctactagtccaatgtctgaacataactaaggaggtaacatagacttgagttacacttggattcttgcatagtctttcttgccgttcatgtattcctgttatctcatttggattatcaaaattgacaacaatcacttactcttttattgttccatgaataattagtttgggcatgaatttggtgtagtactcataacagttgcatttagttagtaagcttaggatgcacatcttaaggaggaggagtgttttctagcttcttggtttgaagataatttgcctaatatctgtaaataaataactccgagaagttttactttggtgctaagtacttaaattgccatcgtggagatactagttcatttaatttgtgttatctattcagatttttgaccttctggtttaaatcagttgataattccttaggatacagggatgatcccactgtaaaaatctagtctgcaaacaagttttgccctgcatgctggctgatcctatgaagttgaatgattttacatgtttgatattttcatgtagctagagcaaagtgcaggtctatggctatcttcaaagtgcatgttgtgtaattcccaatgggttcaaagtgaactgtgttttaactttcagttttacttgtatttctacatatctggtgataacaacttaccggcatgaatagagatattgtatgattgttttcttttcttccttgggagctggtccaatttaactttgaaaaatgatacacagggaatccttgtttttgcttctgtcatggcgactttgggactgcagataattctggagtctatgcgtacactaatatctgatgtaagttgtggcttctatgattgcaaatttctgctctatttatgctgtattgtctggttgaaaattacatggattgttataattattccttgatcctgcacaacgacaaatgttaacattgaccttctcacaggagtctgatttcaaccttaccaaggagcaggagagatgggttgttgggattatggtctttgtgactttggtgaaactagttttaatgttgtattgccggtcttttaccaatgagattgtgaaagcatatgcccaggatcatttctttgatgttatcacaaacataattggtctcattgcagcattgcttgctaactacatcaccgactggatagatcccgttggagctatgattgtaagttctatctctagattctattccaccaacaacctcctcccttaaaagaaatgtgcaaagaaaaaggaaaagttttaatggggctgtcaatcctctcactttaaacaaggttagttgaacaaagttagtggctttaaactattttccctctgctgcagctcgcactgtataccattcgaacttggtcaatgactgtattggagaatgtgaactctctcgtcggcaagtcagctgcaccagaatatctacagaagctgacttacctttgctggaatcatcacaaggccgtaaggcatatagataccgtgagggcttatacatttggttctcactactttgttgaagttgatatcgtcctgcctgcggacatgcctttgcaagaggcacatgatattggcgagtcgttgcaggagaagcttgaactattgcctgagattgagcgggccttcgttcatcttgactacgaatacagccacaaacctgaacatgcacaggcataccaatagtcaaaaggatattgtgacatcttatctaaccaatgtacctaatacctctgcataagtgaactctgatatgctgttcgagatcggttgatctggtgattgctccttaaaagaaaatatggaaaagaaaaggctgctatgatctggatgttccctagaacaagtaatatgaattattattatttttttaatttactttgcctattcatatatataacatgattcctcagtttgcttgctcctggtatattgctaacttatattagaggaatttgggtttc

SEQ ID NO: 23 - DNA, 1200 bp, Nicotiana tabacum
atgttagaagtagtacctcttcacggcggcgatcaaggcgtcggcgccgaagaggagcttttattgctggagacaaacaatgccgaccgatcatggagattaaacttcgacgagttgcggttatcgtctgaaaccaaagagaagcctccacgtggcctccatgattgccttggggttttaagtcaagaagacaacattgctgagtactaccagcaacaggtagaaatgctcgagggcttcaatgaaatggacaccttgactgatcgtggttttgtacctgggatgtcaaaggaagagagggaaaaaactgctagaaatgaaacatttgccattaggatatcaaatgttgcaaacatggttctctttgctgctaaagtatatgcatcagtcaagagtggttcattggccatcatagcatccacattggattcgctgcttgatcttctctctggtttcatattatggtttacagctttctccatgcagacaccaaacccatatcaatatcctattggaaagaaacgtatgcagccgttgggaatccttgtttttgcttctgtcatggcgactttgggactgcagataattctggagtctatgcgtacactaatatctgatgagtctgatttcaaccttaccaaggagcaggagagatgggttgttgggattatggtctttgtgactttggtgaaactagttttaatgttgtattgccggtcttttaccaatgagattgtgaaagcatatgcccaggatcatttctttgatgttatcacaaacataattggtctcattgcagcattgcttgctaactacatcaccgactggatagatcccgttggagctatgattctcgcactgtataccattcgaacttggtcaatgactgtattggagaatgtgaactctctcgtcggcaagtcagctgcaccagaatatctacagaagctgacttacctttgctggaatcatcacaaggccgtaaggcatatagataccgtgagggcttatacatttggttctcactactttgttgaagttgatatcgtcctgcctgcggacatgcctttgcaagaggcacatgatattggcgagtcgttgcaggagaagcttgaactattgcctgagattgagcgggccttcgttcatcttgactacgaatacagccacaaacctgaacatgcacaggcataccaatag

SEQ ID NO: 24 - protein, 399 aa, Nicotiana tabacum
MLEVVPLHGGDQGVGAEEELLLLETNNADRSWRLNFDELRLSSETKEKPPRGLHDCLGVLSQEDNIAEYYQQQVEMLEGFNEMDTLTDRGFVPGMSKEEREKTARNETFAIRISNVANMVLFAAKVYASVKSGSLAIIASTLDSLLDLLSGFILWFTAFSMQTPNPYQYPIGKKRMQPLGILVFASVMATLGLQIILESMRTLISDESDFNLTKEQERWVVGIMVFVTLVKLVLMLYCRSFTNEIVKAYAQDHFFDVITNIIGLIAALLANYITDWIDPVGAMILALYTIRTWSMTVLENVNSLVGKSAAPEYLQKLTYLCWNHHKAVRHIDTVRAYTFGSHYFVEVDIVLPADMPLQEAHDIGESLQEKLELLPEIERAFVHLDYEYSHKPEHAQAYQ

SEQ ID NO: 25 - DNA, 3680 bp, Nicotiana tabacum
aggcaagaccaaacaagtcacatttctcatgcatgccactatttttgagagcaaaaacataatctgaaaatttggatatctacgcattttcacatgtttcaaactccttcactttgtcagcacatcaacagccaatttttctctctttgaaaataaaggaaagggaaagaaaggaaaagggaagttgggaaacatatgccaaatcccctgtcctttctttccctaaataattcccatttctggctgtttcgatttcttgatctgaggatcggaggaattgaatttttaaaattctgttatattccatccattgccacttcttttcttgattgatttttggataagaaaataaagggatttttcaaataaaaatggatgtggaagaggcattgctgaggaatgaagttccaaatgtcataccaaagcgtcgaaactcagttaattctatgagatgtgatttcttctctaaactacctagaaaggttaagacagggcttgatcctgaagaaccttttcttttggacttgtctaaaaccactggtttaattgaaggtaaagcctcttttaagcatttctaagtgcatcatctttttgctcatctcttgttctaatttctatgttgattttgttgcttgattcttagctcatcttctaatgtagttatttatgatcttatgaataggggagaaagaatattatgaaagacagattgcaactttaaagtcctttgaggaagtagactcacttgattcagctgatgtcattgatgaagaacaagacctactagatcaagcacagcatgaaagagcaatgaacatttccaattttgcaaatgtcttattacttgcctttaaggtataacttctttttcattgtttctattgtgcaaacttttaatgcctcaaaccttctcctgaatacaccccaggatcccttttatttctttgttatgagtattatctttttacaattaacccttgtggcccgaccttttctcagaccccacgcatagcatatgcaggagcttagtgcacccgactacccttttatcttttatataatggtagtgtctgagctaacttgaacgcacctcaactattcaacatcccactaacacaagtatcaggttacatctgctcactaaggtttaggcaaatgggaagaaatcacctatcatttcttatctctgttgagatttgaatattgatctctcatgattttcacccacttttggcttctaggctacatccccaagatcctgtttattatctcaaagaaaaggaagacagccctcaggttcagggcagggtagtttgaagtttgcaatagctagtttagctacttaatttttttattgctcaaattataccacatgtaagtttgacattaatgacatattgaatgatcattgtgagacagtaggtagttgtctccaataatgttccttgtagagaaaagaaatgttgtatatttcatctacgagtagttaaatttgcttaaatcaaactgaaccctcgttaatttggactgtttgcagatctatgctactgtaaaaagtggttctttagccattgcagcgtcgacgttggattcactacttgatctaatggctggtggtattctttggttcacacacctgtcaatgaagagcataaacatttacaagtaccctataggaaagttaagagttcaaccagtggggattatcatctttgctgctgttatggctactcttggtatgtcctggttcacctgtcatatctttctcttaattttggcagtctagaattcatgaataacccttgatactgaagaagaggataaataacttctatcataagaataagttcgaccaaaaagttctccattgaagcattgtgaattgcaaaatgatggcgaatacctctaaccacttcttagcagtttatattttgtggatttaggtggtttagtgtggtgtaaagattaagtatacaaaaaattgcaaagagaagtgtttaaagagaattagcaattctagatgattgtttgtatcggtcatgatttctctccttgtgaaaaaagaaatggaaaagaacaatctaaagaagttacaatggaagtctgcatttttgtctcattctgatctgcatttagacagcgcatgtatggtgatcgtgtcctatcacactaattgagtatctgcgattgcataggctttcaagtcttagtgcaggctgtggaacaactgataaaagatacaccctcagacaagatgactggggagcaactggcttggctatatgcaatcatgctgacagccactggagtgaagctcgtcttatggatttattgcagaagttcaggaaacaagatagttagagcatatgcaaaggtcctttttccccatatactctcctgaaaaatctcatttaatgcagtgttatcctttctttcatccattgagcaacatttgacaaattgtggaaccatgcatgatatccaggatcattacttcgatgtggtaacaaatgttgtcggtttggttgctgctgttctcggtgatcgattctattggtggatcgatcctgttggtgctattgtccttgctgtatatacaattacaaattggtcaggaactgtgctggaaaatgcaggttcttactttttcctttgtcagctaacatgcattcacaaatgatgctaatttgattttggtttcgaaagtaatcaacttacgcgaacaaaaaataatacacccaaactctaatgctgcagtttgcaattcttggatatacttcttggatcttttggctcttatagagtagaattttccccttttgtggggaatggtcagtgaatgattttgatgtttatttgctatttacctagctaacacttgaatgtttctctctcctgcagtttctctagttggacaatcagcccctcctgaatttctacagaaactgacatatcttgttctaaggcatgatcctcagataaaaagagttgataccgttcgagcctatacttttggagttctttactttgttgaggtgcgatgtccaccactctgaagtgcttttctcctgcacaattttcaatttttaatagttcataaaattggttgaagagagcaagaaaacaactacgtctcaattcaagcaagttggagccaattatatgaatactcactatccatgtcacttcaattaagctcgtccccgctcaacattataaattattagcttctctagtagtataattttggaaaatttagacaacttccttcataatctgataattggcaattgtctgttttgtaacaggttgacatagagctcccagaagatttgccactgaaagaagcccatgccattggagagtcacttcagattaagattgaagaacttccagaagttgaacgtgcttttgtccatcttgattatgagtgtgatcacaaaccagaacactccattttgagtagaattcccaacagcccaccttaatattctagtctctcaactccgtgttatttcttagtacttttacaatgtaaaattaagagcccattttgctatgtggaagtatcatgaagagtgaggcctgacgttgtgatatgtatacagaaaagaaggaaactaatggttggagaattccatttttcccttatgaagcacctaattagcttcacatttcct

SEQ ID NO: 26 - DNA, 1197 bp, Nicotiana tabacum
atggatgtggaagaggcattgctgaggaatgaagttccaaatgtcataccaaagcgtcgaaactcagttaattctatgagatgtgatttcttctctaaactacctagaaaggttaagacagggcttgatcctgaagaaccttttcttttggacttgtctaaaaccactggtttaattgaaggggagaaagaatattatgaaagacagattgcaactttaaagtcctttgaggaagtagactcacttgattcagctgatgtcattgatgaagaacaagacctactagatcaagcacagcatgaaagagcaatgaacatttccaattttgcaaatgtcttattacttgcctttaagatctatgctactgtaaaaagtggttctttagccattgcagcgtcgacgttggattcactacttgatctaatggctggtggtattctttggttcacacacctgtcaatgaagagcataaacatttacaagtaccctataggaaagttaagagttcaaccagtggggattatcatctttgctgctgttatggctactcttggctttcaagtcttagtgcaggctgtggaacaactgataaaagatacaccctcagacaagatgactggggagcaactggcttggctatatgcaatcatgctgacagccactggagtgaagctcgtcttatggatttattgcagaagttcaggaaacaagatagttagagcatatgcaaaggatcattacttcgatgtggtaacaaatgttgtcggtttggttgctgctgttctcggtgatcgattctattggtggatcgatcctgttggtgctattgtccttgctgtatatacaattacaaattggtcaggaactgtgctggaaaatgcagtttctctagttggacaatcagcccctcctgaatttctacagaaactgacatatcttgttctaaggcatgatcctcagataaaaagagttgataccgttcgagcctatacttttggagttctttactttgttgaggttgacatagagctcccagaagatttgccactgaaagaagcccatgccattggagagtcacttcagattaagattgaagaacttccagaagttgaacgtgcttttgtccatcttgattatgagtgtgatcacaaaccagaacactccattttgagtagaattcccaacagcccaccttaa

SEQ ID NO: 27 - protein, 398 aa, Nicotiana tabacum
MDVEEALLRNEVPNVIPKRRNSVNSMRCDFFSKLPRKVKTGLDPEEPFLLDLSKTTGLIEGEKEYYERQIATLKSFEEVDSLDSADVIDEEQDLLDQAQHERAMNISNFANVLLLAFKIYATVKSGSLAIAASTLDSLLDLMAGGILWFTHLSMKSINIYKYPIGKLRVQPVGIIIFAAVMATLGFQVLVQAVEQLIKDTPSDKMTGEQLAWLYAIMLTATGVKLVLWIYCRSSGNKIVRAYAKDHYFDVVTNVVGLVAAVLGDRFYWWIDPVGAIVLAVYTITNWSGTVLENAVSLVGQSAPPEFLQKLTYLVLRHDPQIKRVDTVRAYTFGVLYFVEVDIELPEDLPLKEAHAIGESLQIKIEELPEVERAFVHLDYECDHKPEHSILSRIPNSPP

SEQ ID NO: 28 - DNA, 4195 bp, Nicotiana tabacum
  misc_feature (1013)..(1027): n is a, c, g, or t
tagcaaaaagacaaagttagcaacttaaaacagaaagtttgagacccaacgcaaagacagttttttttaaagaaacaaaattatctaatggtttggtagtacgtactacgttttaatcttctttatatttttaattagtacaacatctgactttgtcttttttctaattaaaataaaagttagatcatactcgaagttatatatatctaatcaatgcaaatagtgtgaagcttaattacatgatttggagtttgcattactgaaaatatatactcctacaactcttgataatggagggagaattagaggctaacaatattaatggaactaaaacgccattgttggaggggtggaagcttagcggaagtggacggcggagcagccggcgtttcagccggcataactcttttacgtcgctccgccgtgatttcttgtctaggcttccagataaggtgatcaactcttttgttattgattctgaagcttcatacatcattaataacctctccatatcctctgacttaaccaaaggttcttctctctctctcaggttgtttggttccggactaaatatgtggttaactgattatgatatatataaagattattatatgttgtataaaactatagtgcttgtaattaatggattatgtaaagttaagaattagttttatcttgctattgttaatatgcatgttcttatatattcccatgaacatgttcttggcttgagaaaaagtgaaactttttcttttctatgctaaatttggtgtatagactaggttctgtttgatattaattactcctattaaaggattcaaacagaagctgttatacaatcgtttgatcatgttaatccaatcacactgcatattaaactccttaacatcttttaaagattagaaaaggatgacctgggatcgaatccccctcaatgccttttgggttgagtctgtcgcacatggcttgcctagtgcggattacctctcctgtgtggcttgcaggctattacnnnnnnnnnnnnnnngcggctgcggggttttcccctcttaaaccaaaaaaaaaaaaaaaaaaagaaaaaaggaatatcaatttttttcttttttctttttccttttttttttttttttattttatttgcaaataaagcaaaattttgctggaaactacactagggaaattcaaatatctaccgctagaaaaggatatctttaacaccctcagtcagtggcgaagccacatggttataaggatggtcaattgaccacccttcgtcgaaaaattacactgtgtatataggtaaaatattacgttttagcggtatacaacacatattgaacaccctttgtcgggaattttttttacttcattcaaatttgaacacctttggaaaaaaatttaggttcgccactgccctcggtgctccgttgactaagttttatgatgataggagaaaaggaatactatgaaaaacagtttgagactttgaagtcatttgaggaagttgattctgcagttgcttctgattgcattgatgaagaggatctcgaagaacaagctcaacatgagagagcaatgagaatctccaattatgcaaacattatactgcttgctctcaaggtgaccagaaattacttaattgaactcgtcattaacatgagaatgagaaatcatctattaatgtgtatgcatttctttgtcctgcaacatttttatatatgcagtaaaagtgaaattctggtttatgtttgaatgacctggaaaaatgataaagatggtggtttatgcctttttgtcacaatagcagtattgacacatatcgcgccttgcagatctatgccacagtaaagagtggttctttagctattgctgcatctacactggattcattgcttgacctcatggctggtggcatactatggtttactcatctttcaatgaaaaatattaatgtctataaatatcctattggaaaattgagagtgcagcctgttggaatcatcgtctttgctgctattatggctacacttggtatgttatctgctttgactttgcatttgaaattccattatcgggttagtgaatacatagcgactttagcttacagaagacatggcccttgacaggaggatatggaggtcgaagattagggtagaagggtaataggtcgtagtgtgtttttctaatatgttccaggtttattagcgcgagctgactagtacattgtcttcgattcttagagtgctagtattagggttgttttcagtactatcttccgcttcggttttctagtactttgtcgtaatactgcttgttgctattgctttcttccatttgtttgttttctcggttcatacattgatagtatcattttcctggccttgttgttattaccttattcctattcttcctctcgagccgggagtctttcggaaatagcctctctatccctcagggtaggggtaaggtctgcgtatacattactctcctcataccccacttgtgggattccattgggttgttgttgttgggttagtgaatacatgtcagtttggacaggtgagagtgaggcattggaaataaaaaaaaaaaaaaacaggatgacggctttcaaaagacgagtaagagacggggagatggaggctctcgaaaccaaatgagattagagagaacaggggaattagcaccattcatatgagagctaacctctttgtatatgaaattcttcaatttgcataatcatgtgcatttctttgtaggctttcaggtgctgatccaggctgtagaacaactagttgaaaataaagctcctgaaaagatgactttgaatcagctcgcatggttatattccatcatgttaactgccacagtagtaaaacttgccctttggctttactgcagaagctcaggaaacaacattgttcgtgcgtatgcaaaggtgtgtgtagtgtccttaccttctggtttccacatcttctcctgataatctcttttcctaatttgttgatgtatttgtcaggatcactattttgatgtggttactaacgtagtcgggttaatagcagctgtacttggtgataagttctactggtggattgatcccgttggtgctcttatccttgctatttatacaatctcaaattggtcagccactgtgatagagaatgcaggtatatacttacatgttcctgttgaatttatagttcgtcaataattcatggaagttaacagcgacgttcaacaaacacagaactagtaacgcagactagaatctaaccttgtaagaaaaattatccctttaggatgtctgcaagaattatgcttgttggacacctcaagtctgagcacataatatatgttgtccaagccaacttgcacgcagctcgactattccaccggttacctgctacctctcaccagtaaacgtatcgagtaactctgctcatcaaggtttaggcagatggaaagaaattaactagtgtctttttgccaccgctggggtttgaactggagacctcatggttctcctctcacttcattgaccactagaccacaccctgggatgcaaaactccgatattttcttggtgttatttatatcaatacatcaaataaaacttgaatgaggttcttgatgcagtgtcactggtaggacaatcagctcctcctgaagttatgcagaagttaacatatgttgttataagacatcctcaagtgaaacgtattgatacagttcgagcatacacctttggtgtcttgtactttgttgaggtcagtctccaatagcatgaaatcattttcctaaacatctttggtctgaactaactgaattattaaggcatagccttttccagatctctgctgatttcaaaatgttgcttcctttcttttaacataggttgatattgaactcccggaagatttgccattgaaagaagcacatattatcggagagactctacaaataaagctcgagaaactccctgaagtggaacgcgcatttgttcatcttgattttgaatgtgaacacaaaccagaacactccgtccccagcaagctgcccaacaatgaatcttaagtgtagaacacacaaactaggagaaatttcaatataaagaataggtctttgattgggagctcagctgctcctgaacctctataaatactcttggtcatgtttgaggaatttgcatgat

SEQ ID NO: 29 - DNA, 1251 bp, Nicotiana tabacum
atggagggagaattagaggctaacaatattaatggaactaaaacgccattgttggaggggtggaagcttagcggaagtggacggcggagcagccggcgtttcagccggcataactcttttacgtcgctccgccgtgatttcttgtctaggcttccagataaggtgatcaactcttttgttattgattctgaagcttcatacatcattaataacctctccatatcctctgacttaaccaaaggagaaaaggaatactatgaaaaacagtttgagactttgaagtcatttgaggaagttgattctgcagttgcttctgattgcattgatgaagaggatctcgaagaacaagctcaacatgagagagcaatgagaatctccaattatgcaaacattatactgcttgctctcaagatctatgccacagtaaagagtggttctttagctattgctgcatctacactggattcattgcttgacctcatggctggtggcatactatggtttactcatctttcaatgaaaaatattaatgtctataaatatcctattggaaaattgagagtgcagcctgttggaatcatcgtctttgctgctattatggctacacttggctttcaggtgctgatccaggctgtagaacaactagttgaaaataaagctcctgaaaagatgactttgaatcagctcgcatggttatattccatcatgttaactgccacagtagtaaaacttgccctttggctttactgcagaagctcaggaaacaacattgttcgtgcgtatgcaaaggatcactattttgatgtggttactaacgtagtcgggttaatagcagctgtacttggtgataagttctactggtggattgatcccgttggtgctcttatccttgctatttatacaatctcaaattggtcagccactgtgatagagaatgcagtgtcactggtaggacaatcagctcctcctgaagttatgcagaagttaacatatgttgttataagacatcctcaagtgaaacgtattgatacagttcgagcatacacctttggtgtcttgtactttgttgaggttgatattgaactcccggaagatttgccattgaaagaagcacatattatcggagagactctacaaataaagctcgagaaactccctgaagtggaacgcgcatttgttcatcttgattttgaatgtgaacacaaaccagaacactccgtccccagcaagctgcccaacaatgaatcttaa

SEQ ID NO: 30 - protein, 416 aa, Nicotiana tabacum
MEGELEANNINGTKTPLLEGWKLSGSGRRSSRRFSRHNSFTSLRRDFLSRLPDKVINSFVIDSEASYIINNLSISSDLTKGEKEYYEKQFETLKSFEEVDSAVASDCIDEEDLEEQAQHERAMRISNYANIILLALKIYATVKSGSLAIAASTLDSLLDLMAGGILWFTHLSMKNINVYKYPIGKLRVQPVGIIVFAAIMATLGFQVLIQAVEQLVENKAPEKMTLNQLAWLYSIMLTATVVKLALWLYCRSSGNNIVRAYAKDHYFDVVTNVVGLIAAVLGDKFYWWIDPVGALILAIYTISNWSATVIENAVSLVGQSAPPEVMQKLTYVVIRHPQVKRIDTVRAYTFGVLYFVEVDIELPEDLPLKEAHIIGETLQIKLEKLPEVERAFVHLDFECEHKPEHSVPSKLPNNES

SEQ ID NO: 31 - protein, 299 aa, Artificial Sequence
  polypeptide sequence of a mutated cation efflux protein
MEISRSNVSGGGGSGGALDDSFSSFRTELLSPAAQAVVDQSSSSASWRLNISEFRLPERSRSSSDHHSFSVRRLLPTPRKQGKIAEYYKKQERLLEGFNEMDTINESGCLPGSLTEDEMKQLARSERMAIHLSNMANVVLFIAKIYASIESRSLAVIASTLDSLLDLLSGFILWFTSHAMKNPNQYHYPIGKKRMQPLGIIVFASVMATLGLQILFESAKELITKSRPEMDHEKEKWTIGIMVSVTMVKFLLMVYCRRFKNEIVRAYAQDHFFDVITNSVGLVTAVLAVRFYWWIDPTG

SEQ ID NO: 32 - DNA, 903 bp, Artificial Sequence
  cDNA sequence of a mutated cation efflux protein
atggagataagtcgcagcaatgttagtggtggtggcggcagcggcggcgctctggacgacagttttagcagttttaggacggaactgctgtctccggctgctcaggcggtggtggatcagtcgtcttcgtcggcgtcatggagacttaacattagcgaattccgtcttcccgaacgaagccgctcctcctccgatcatcactcctttagtgtccgtcgtctacttcccactcccaggaaacaaggtaaaattgctgaatactacaaaaaacaagaaaggctgcttgaagggttcaatgagatggacaccattaatgaatctggttgtttacctggaagtctaactgaggatgaaatgaagcagcttgcaagaagtgaaaggatggctattcatttatcaaacatggctaatgtggttcttttcattgcaaaaatctacgcttctattgagagcagatctttggctgtaatcgcgtcaacgttggactccctcttagacctcttatcagggtttatactgtggttcacttctcatgccatgaaaaatccaaaccagtatcactatcctattggaaaaaagaggatgcagccattgggtattattgtttttgcatctgtaatggcgacactaggattacaaatattgttcgagtcagctaaagaactcataactaagtctcgccctgagatggaccatgagaaggaaaaatggacgattggtattatggtctctgtcactatggtcaagtttctgcttatggtctactgtcgaaggttcaaaaacgaaatcgtaagagcctatgctcaagatcatttctttgatgtcatcaccaactcagttggattagtgactgctgtcttagcagtccgattctactggtggattgatcctacgggagcttaa

SEQ ID NO: 33 - protein, 300 aa, Artificial Sequence
  polypeptide sequence of a mutated cation efflux protein
MEMKQLARSERMAIHLSNMANVVLFIAKIYASIESRSLAVIASTLDSLLDLLSGFILWFTSHAMKNPNQYHYPIGKKRMQPLGIIVFASVMATLGLQILFESAKELITKSRPEMDHEKEKWTIGIMVSVTMVKFLLMVYCRRFKNEIVRAYAQDHFFDVITNSVGLVTAVLAVRFYWWIDPTGAIIIAMYTISTWAKTVAENVWSLIGRTAPPDFLTKLTYLIWNHHEEIKHIDTVRAYTFGAHYFVEVDIVLPEDMLLNKAHNIGETLQEKLEQLPEVERAFVHIDFEFTHRPEHKTMV

SEQ ID NO: 34 - DNA, 903 bp, Artificial Sequence
  cDNA sequence of a mutated cation efflux protein
atggaaatgaagcagcttgcaagaagtgaaaggatggctattcatttatcaaacatggctaatgtggttcttttcattgcaaaaatctacgcttctattgagagcagatctttggctgtaatcgcgtcaacgttggactccctcttagacctcttatcagggtttatactgtggttcacttctcatgccatgaaaaatccaaaccagtatcactatcctattggaaaaaagaggatgcagccattgggtattattgtttttgcatctgtaatggcgacactaggattacaaatattgttcgagtcagctaaagaactcataactaagtctcgccctgagatggaccatgagaaggaaaaatggacgattggtattatggtctctgtcactatggtcaagtttctgcttatggtctactgtcgaaggttcaaaaacgaaatcgtaagagcctatgctcaagatcatttctttgatgtcatcaccaactcagttggattagtgactgctgtcttagcagtccgattctactggtggattgatcctacgggagctataattatagctatgtacacaattagcacgtgggcgaagacagtggcagaaaatgtctggtcactcattggaagaacagctccaccagattttcttacgaaattaacctatcttatatggaatcatcacgaagagatcaagcacattgatactgttcgagcatatacttttggtgctcattattttgtagaggttgatatagtgttgccagaggacatgctgttgaacaaggcacataatattggtgagacactgcaagaaaaattggagcaactccctgaagttgagcgagcttttgttcatatagacttcgagttcactcacaggccagaacacaaaactatggtataa

SEQ ID NO: 35 - skipped

SEQ ID NO: 36 - DNA, 16 bp, Artificial Sequence
  primer M13.fw
gtaaaacgacggccag

SEQ ID NO: 37 - DNA, 17 bp, Artificial Sequence
  primer M13.rv
gtcatagctgtttcctg

SEQ ID NO: 38 - DNA, 15123 bp, Artificial Sequence
  Gateway Destination Binary (GDB) expression vector sequence
agcttgcatgcctgcaggtcgagcttttaggattccatagtgataagatatgttcttatctaaacaaaaaagcaagcgtcggcaaaccatacagctgtccacaaaaaggaaaggctgtaataacaagcggacccagcttctcagtggaagatactttatcagacactgaataatggatggaccctaccacgattaaagaggagcgtctgtctaaagtaaagtagatgcgtctttaataattcatctactttagacgtcatgcatgacgtttaacatgcattgtatccagatcctccctggctatataaagggagttaaatttcattgttaaggcatcgaaaaaaaaatttcaagtctatctctcaagaaaaacttagaaaattactttgtcttaaggatccgggcccagctgtcacaagtttgtacaaaaaagctgaacgagaaacgtaaaatgatataaatatcaatatattaaattagattttgcataaaaaacagactacataatactgtaaaacacaacatatccagtcactatggcgccgcattaggcaccccaggctttacactttatgcttccggctcgtataatgtgtggattttgagttacgatccgtcgagattttcaggagctaaggaagctaaaatggagaaaaaaatcactggatataccaccgttgatatatcccaatggcatcgtaaagaacattttgaggcatttcagtcagttgctcaatgtacctataaccagaccgttcaactggatattacggcctttttaaagaccgtaaagaaaaataagcacaagttttatccggcctttattcacattcttgcccgcctgatgaatgctcatccggaatttcgtatggcaatgaaagacggtgagctggtgatatgggatagtgttcacccttgttacaccgttttccatgagcaaactgaaacgttttcatcgctctggagtgaataccacgacgatttccggcagtttctacacatatattcgcaagatgtggcgtgttacggtgaaaacctggcctatttccctaaagggtttattgagaatatgtttttcgtctcagccaatccctgggtgagtttcaccagttttgatttaaacgtggccaatatggacaacttcttcgcccccgttttcacgatgggcaaatattatacgcaaggcgacaaggtgctgatgccgctggcgattcaggttcatcatgccgtttgtgatggcttccatgtcggcagaatgcttaatgaattacaacagtactgcgatgagtggcagggcggggcgtaaacgcgacgatccggcttactaaaagccagataacagtatgcgtatttgcgcgctgatttttgcggtataagaatatatactgatatgtatacccgaagtatgtcaaaaagaggtatgctatgaagcagcgtattacagtgacagttgacagcgacagctatcagttgctcaaggcatatatgatgtcaatatctccggtctggtaagcacaaccatgcagaatgaagcccgtcgtctgcgtgccgaacgctggaaagcggaaaatcaggaagggatggctgaggtcgcccggtttattgaaatgaacggctcttttgctgacgagaacaggggctggtgaaatgcagtttaaggtttacacctataaaagagagagccgttatcgtctgtttgtggatgtacagagtgatattattgacacgcctgggcgacggatggtgatccccctggccagtgcacgtctgctgtcagataaagtctcccgtgaactttacccggtggtgcatatcggggatgaaagctggcgcatgatgaccaccgatatggccagtgtgccggtctccgttatcggggaagaagtggctgatctcagccaccgcgaaaatgacatcaaaaacgccattaacctgatgttctggggaatataaatgtcaggctcccttatacacagccagtctgcacctcgaccatagtgactggatatgttgtgttttacagtattatgtagtctgttttttatgcaaaatctaatttaatatattgatatttatatcattttacgtttctcgttcagctttcttgtacaaagtggtgcagctgagatctaggcctaagtaagtaagatcgttcaaacatttggcaataaagtttctttagattgaatcctgttgccggtcttgcgatgattatcatataatttctgttgaattacgttaagcatgtagtaattaacatgtaatggatgacgttatttatgagatgggtttttatgattagagtcccgcaattatacatttaatacgcgatagaaaacaaaatatagcgcgcaaactaggataaattatcgcgcgcggtgtcatctatgttactagatcgaaggccttgttctcgagcaattcactggccgtcgttttacaacgtcgtgactgggaaaaccctggcgttacccaacttaatcgccttgcagcacatccccctttcgccagcaggcgtaatagcgaagaggcccgcaccgattgcccttcccaacagttgcgcagcctgaatggcgcccgctcctttcgctttcttcccttcctttctcgccacgttcgccggctttccccgtcaagctctaaatcgggggctccctttagggttccgatttagtgctttacggcacctcgaccccaaaaaacttgatttgggtgatggttcacaaactatcagtgtttgacaggatatattggcgggtaaacctaagagaaaagagcgtttattagaataatcggatatttaaaagggcgtgaaaaggtttatccgttcgtccatttgtatgtgcatgccaaccacaggcttaagaaaacttgatttgggtgatggttcacaaactatcagtgtttgacaggatatattggcgggtaaacctaagagaaaagagcgtttattagaataatcggatatttaaaagggcgtgaaaaggtttatccgttcgtccatttgtatgtgcatgccaaccacaggcttaaggttctagactggcgccggccagcgagacgagcaagattggccgccgcccgaaacgatccgacagcgcgcccagcacaggtgcgcaggcaaattgcaccaacgcatacagcgccagcagaatgccatagtgggcggtgacctcgttcgagtgaaccagatcgcgcaggaggcccggcagcaccggcataatcaggccgatgccgacagcgtcgagcgcgacagtgctcagaattacgatcaggggtatgttgggtttcacgtctggcctccggaccagcctccgctggtccgattgaacgcgcggattctttatcactgataagttggtggacatattatgtttatcagtgataaagtgtcaagcatgacaaagttgcagccgaatacagtgatccgtgccgccctggacctgttgaacgaggtcggcgtagacggtctgacgacacgcaaactggcggaacggttgggggttcagcagccggcgctttactggcacttcaggaacaagcgggcgctgctcgacgcactggccgaagccatgctggcggagaatcatacgcattcggtgccgagagccgacgacgactggcgctcatttctgatcgggaatgcccgcagcttcaggcaggcgctgctcgcctaccgcgatggcgcgcgcatccatgccggcacgcgaccgggcgcaccgcagatggaaacggccgacgcgcagcttcgcttcctctgcgaggcgggtttttcggccggggacgccgtcaatgcgctgatgacaatcagctacttcactgttggggccgtgcttgaggagcaggccggcgacagcgatgccggcgagcgcggcggcaccgttgaacaggctccgctctcgccgctgttgcgggccgcgatagacgccttcgacgaagccggtccggacgcagcgttcgagcagggactcgcggtgattgtcgatggattggcgaaaaggaggctcgttgtcaggaacgttgaaggaccgagaaagggtgacgattgatgaggaccgctgccggagcgcaacccactcactacagcagagccatgtagacaacatcccctccccctttccaccgcgtcagacgcccgtagcagcccgctacgggctttttcatgccctgccctagcgtccaagcctcacggccgcgctcggcctctctggcggccttctggcgctcgtcgaccgctcactgactcgctgcgctcggtcgttcggctgcggcgagcggtatcagctcactcaaaggcggtaatacggttatccacagaatcaggggataacgcaggaaagaacatgtgagcaaaaggccagcaaaaggccaggaaccgtaaaaaggccgcgttgctggcgtttttccataggctccgcccccctgacgagcatcacaaaaatcgacgctcaagtcagaggtggcgaaacccgacaggactataaagataccaggcgtttccccctggaagctccctcgtgcgctctcctgttccgaccctgccgcttaccggatacctgtccgcctttctcccttcgggaagcgtggcgcttttccgctgcataaccctgcttcggggtcattatagcgattttttcggtatatccatcctttttcgcacgatatacaggattttgccaaagggttcgtgtagactttccttggtgtatccaacggcgtcagccgggcaggataggtgaagtaggcccacccgcgagcgggtgttccttcttcactgtcccttattcgcacctggcggtgctcaacgggaatcctgctctgcgaggctggccggctaccgccggcgtaacagatgagggcaagcggatggctgatgaaaccaagccaaccaggaagggcagcccacctatcaaggtgtactgccttccagacgaacgaagagcgattgaggaaaaggcggcggcggccggcatgagcctgtcggcctacctgctggccgtcggccagggctacaaaatcacgggcgtcgtggactatgagcacgtccgcgagctggcccgcatcaatggcgacctgggccgcctgggcggcctgctgaaactctggctcaccgacgacccgcgcacggcgcggttcggtgatgccacgatcctcgccctgctggcgaagatcgaagagaagcaggacgagcttggcaaggtcatgatgggcgtggtccgcccgagggcagagccatgacttttttagccgctaaaacggccggggggtgcgcgtgattgccaagcacgtccccatgcgctccatcaagaagagcgacttcgcggagctggtgaagtacatcaccgacgagcaaggcaagaccgagcgcctttggtacctcaccgggctggttgccctcgccgctgggctggcggccgtctatggccctgcaaacgcgccagaaacgccgtcgaagccgtgtgcgagacaccgccgccgccggcgttgtggatacctcgcggaaaacttggccctcactgacagatgaggggcggacgttgacacttgaggggccgactcacccggcgcggcgttgacagatgaggggcaggctcgatttcggccggcgacgtggagctggccagcctcgcaaatcggcgaaaacgcctgattttacgcgagtttcccacagatgatgtggacaagcctggggataagtgccctgcggtattgacacttgaggggcgcgactactgacagatgaggggcgcgatccttgacacttgaggggcagagtgctgacagatgaggggcgcacctattgacatttgaggggctgtccacaggcagaaaatccagcatttgcaagggtttccgcccgtttttcggccaccgctaacctgtcttttaacctgcttttaaaccaatatttataaaccttgtttttaaccagggctgcgccctgtgcgcgtgaccgcgcacgccgaaggggggtgcccccccttctcgaaccctcccggcccgctaacgcgggcctcccatccccccaggggctgcgcccctcggccgcgaacggcctcaccccaaaaatggcagcgctggcagtccttgccattgccgggatcggggcagtaacgggatgggcgatcagcccgagcgcgacgcccggaagcattgacgtgccgcaggtgctggcatcgacattcagcgaccaggtgccgggcagtgagggcggcggcctgggtggcggcctgcccttcacttcggccgtcggggcattcacggacttcatggcggggccggcaatttttaccttgggcattcttggcatagtggtcgcgggtgccgtgctcgtgttcgggggtgacgcgtgaaaattttcgataaacccagcgaaccatttgaggtgataggtaagattataccgaggtatgaaaacgagaattggacctttacagaattactctatgaagcgccatatttaaaaagctaccaagacgaagaggatgaagaggatgaggaggcagattgccttgaatatattgacaatactgataagataatatatcttttatatagaagatatggccgtatgtaaggatttcagggggcaaggcataggcagcgcgcttatcaatatatctatagaatgggcaaagcataaaaacttgcatggactaatgcttgaaacccaggacaataaccttatagcttgtaaattctatcataattgggtaatgactccaacttattgatagtgttttatgttcagataatgcccgatgactttgtcatgcagctccaccgattttgagaacgacagcgacttccgtcccagccgtgccaggtgctgcctcagattcaggttatgccgctcaattcgctgcgtatatcgcttgctgattacgtgcagctttcccttcaggcgggattcatacagcggccagccatccgtcatccatatcaccacgtcaaagggtgacagcaggctcataagacgccccagcgtcgccatagtgcgttcaccgaatacgtgcgcaacaaccgtcttccggagactgtcatacgcctaaaacagccagcgctggcgcgatttagccccgacatagccccactgttcgtccatttccgcgcagacgatgacgacactgcccggctgtatgcgcgaggttacctgctgccagtggcgataagtcgtgtcttaccgggttggactcaagacgatagttaccggataaggcgcagcggtcgggctgaacggggggttcgtgcacacagcccagcttggagcgaacgacctacaccgaactgagatacctacagcgtgagctatgagaaagcgccacgcttcccgaagggagaaaggcggacaggtatccggtaagcggcagggtcggaacaggagagcgcacgagggagcttccagggggaaacgcctggtatctttatagtcctgtcgggtttcgccacctctgacttgagcgtcgatttttgtgatgctcgtcaggggggcggagcctatggaaaaacgccagcaacgcggcctttttacggttcctggccttttgctggccttttgctcacatgttctttcctgcgttatcccctgattctgtggataaccgtattaccgcctttgagtgagctgataccgctcgccgcagccgaacgaccgagcgcagcgagtcagtgagcgaggaagcggaagagcgcctgatgcggtattttctccttacgcatctgtgcggtatttcacaccgcatagttaccgactgcggcctgagttttttaagtgacgtaaaatcgtgttgaggccaacgcccataatgcgggctgttgcccggcatccaacgccattcatggccatatcaatgattttctggtgcgtaccgggttgagaagcggtgtaagtgaacagcagttgccatgttttacggcagtgagagcagagatagcgctgatgtccggcggtgcttttgccgttacgcaccaccccgtcagtagctgaacaggagggacacctgatagacacagaagccactggagcacctcaaaaacaccatcatacactaaatcagtaagttggcagcatcacccgttaacataattgtggtttcaaaatcggctccgtcgatactatgttatacgccaactttgaaaacaactttgaaaaagctgttttctggtatttaaggttttagaatgcaaggaacagtgaattggagttcgtcttgttataattagcttcttggggtatctttaaatactgtagaaaagaggaaggaaataataaatggctaaaatgagaatatcaccggaattgaaaaaactgatcgaaaaataccgctgcgtaaaagatacggaaggaatgtctcctgctaaggtatataagctggtgggagaaaatgaaaacctatatttaaaaatgacggacagccggtataaagggaccacctatgatgtggaacgggaaaaggacatgatgctatggctggaaggaaagctgcctgttccaaaggtcctgcactttgaacggcatgatggctggagcaatctgctcatgagtgaggccgatggcgtcctttgctcggaagagtatgaagatgaacaaagccctgaaaagattatcgagctgtatgcggagtgcatcaggctctttcactccatcgacatatcggattgtccctatacgaatagcttagacagccgcttagccgaattggattacttactgaataacgatctggccgatgtggattgcgaaaactgggaagaagacactccatttaaagatccgcgcgagctgtatgattttttaaagacggaaaagcccgaagaggaacttgtcttttcccacggcgacctgggagacagcaacatctttgtgaaagatggcaaagtaagtggctttattgatcttgggagaagcggcagggcggacaagtggtatgacattgccttctgcgtccggtcgatcagggaggttatcggggaagaacagtatgtcgagctattttttgacttactggggatcaagcctgattgggagaaaataaaatattatattttactggatgaattgttttagtacctagagaaaattttcctaggtgtggcgcaacgatgccggcgacaagcaggagcgcaccgacttcttccgcatcaagtgttttggctctcaggccgaggcccacggcaagtatttgggcaaggggtcgctggtattcgtgcagggcaagattcggaataccaagtacgagaaggacggccagacggtctacgggaccgacttcattgccgataaggtggattatctggacaccaaggcaccaggcgggtcaaatcaggaataagggcacattgccccggcgtgagtcggggcaatcccgcaaggagggtgaatgaatcggacgtttgaccggaaggcatacaggcaagaactgatcgacgcggggttttccgccgaggatgccgaaaccatcgcaagccgcaccgtcatgcgtgcgccccgcgaaaccttccagtccgtcggctcgatggtccagcaagctacggccaagatcgagcgcgacagcgtgcaactggctccccctgccctgcccgcgccatcggccgccgtggagcgttcgcgtcgtctcgaacaggaggcggcaggtttggcgaagtcgatgaccatcgacacgcgaggaactatgacgaccaagaagcgaaaaaccgccggcgaggacctggcaaaacaggtcagcgaggccaagcaggccgcgttgctgaaacacacgaagcagcagatcaaggaaatgcagctttccttgttcgatattgcgccgtggccggacacgatgcgagcgatgccaaacgacacggcccgctctgccctgttcaccacgcgcaacaagaaaatcccgcgcgaggcgctgcaaaacaaggtcattttccacgtcaacaaggacgtgaagatcacctacaccggcgtcgagctgcgggccgacgatgacgaactggtgtggcagcaggtgttggagtacgcgaagcgcacccctatcggcgagccgatcaccttcacgttctacgagctttgccaggacctgggctggtcgatcaatggccggtattacacgaaggccgaggaatgcctgtcgcgcctacaggcgacggcgatgggcttcacgtccgaccgcgttgggcacctggaatcggtgtcgctgctgcaccgcttccgcgtcctggaccgtggcaagaaaacgtcccgttgccaggtcctgatcgacgaggaaatcgtcgtgctgtttgctggcgaccactacacgaaattcatctgggagaagtaccgcaagctgtcgccgacggcccgacggatgttcgactatttcagctcgcaccgggagccgtacccgctcaagctggaaaccttccgcctcatgtgcggatcggattccacccgcgtgaagaagtggcgcgagcaggtcggcgaagcctgcgaagagttgcgaggcagcggcctggtggaacacgcctgggtcaatgatgacctggtgcattgcaaacgctagggccttgtggggtcagttccggctgggggttcagcagccagcgtgatcactttactggcatttcaggaacaagcgggcactgctcgacgcacttgcttcgctcagtatcgctcgggacgcacggcgcgctctacgaactgccgataaacagaggattaaaattgacaattgtgattaaggctcagattcgacggcttggagcggccgacgtgcaggatttccgcgagatccgattgtcggccctgaagaaagctccagagatgttcgggtccgtttacgagcacgaggagaaaaagcccatggaggcgttcgctgaacggttgcgagatgccgtggcattcggcgcctacatcgacggcgagatcattgggctgtcggtcttcaaacaggaggacggccccaaggacgctcacaaggcgcatctgtccggcgttttcgtggagcccgaacagcgaggccgaggggtcgccggtatgctgctgcgggcgttgccggcgggtttattgctcgtgatgatcgtccgacagattccaacgggaatctggtggatgcgcatcttcatcctcggcgcacttaatatttcgctattctggagcttgttgtttatttcggtctaccgcctgccgggcggggtcgcggcgacggtaggcgctgtgcagccgctgatggtcgtgttcatctctgccgctctgctaggtagcccgatacgattgatggcggtcctgggggctatttgcggaactgcgggcgtggcgctgttggtgttgacaccaaacgcagcgctagatcctgtcggcgtcgcagcgggcctggcgggggcggtttccatggcgttcggaaccgtgctgacccgcaagtggcaacctcccgtgcctctgctcacctttaccgcctggcaactggcggccggaggacttctgctcgttccagtagctttagtgtttgatccgccaatcccgatgcctacaggaaccaatgttctcggcctggcgtggctcggcctgatcggagcgggtttaacctacttcctttggttccgggggatctcgcgactcgaacctacagttgtttccttactgggctttctcagccccaggtctggggtcgatcagccggggatgcatcaggccgacagtcggaacttcgggtccccgacctgtaccattcggtgagcaatggataggggagttgaaatcgtcaacgttcacttctaaagaaatagcgccactcagcttcctcagcggctttatccagcgatttcctattatgtcggcatagttctcaagatcgacagcctgtcacggttaagcgagaaatgaataagaaggctgataattcggatctctgcgagggagatgatatttgatgacaggcagcaacgctctgtcatcgttacaatcaacatgctaccctccgcgagatcatccgtgtttcaaacccggcagcttagttgccgttcttccgaatagcatcggtaacatgagcaaagtctgccgccttacaacggctctcccgctgactagtcgtcccggagacgtcctgatgggctgcctgtatcgagtggtgattttgtgccgagctgccggtcggggagctgttggctggctggtggcaggatatattgtggtgtaaacaaattgacgcttagacaacttaataacacattgcggacgtttttaatgtactggacgtcctgatgggctgcctgtatcgagtggtgattttgtgccgagctgccggtcggggagctgttggctggctggtggcaggatatattgtggtgtaaacaaattgacgcttagacaacttaataacacattgcggacgtttttaatgtactggggtggtttttcttttcaccagtgagacgggcaacacgtgattgcccttcaccgcctggccctgagagagttgcagcaagcggtccacgctggtttgccccagcaggcgaaaatcctgtttgatggtggttccgaaatcggcaaaatcccttataaatcaaaagaatagcccgagatagggttgagtgttgttccagtttggaacaagagtccactattaaagaacgtggactccaacgtcaaagggcgaaaaaccgtctatcagggcgatggcccacaaactgaaggcggccgcaaacgatatcaatctcatcatgagcggagaattaagggagtcacgttatgacccccgccgatgacgcgggacaagccgttttacgtttggaactgacagaaccgcaacgttgaaggagccactcagccgccggtttctggagtttaatgagctaagcacatacgtcagaaaccattattgcgcgttcaaaagtcgcctaaggtcactatcagctagcaaatatttcttgtcaaaaatgctccactgacgttccataaattcccctcggtatccaattagagtctcatattcactctcaatccaaataatctgcaccggatctggatcgtttcgcatgattgaacaagatggattgcacgcaggttctccggccgcttgggtggagaggctattcggctatgactgggcacaacagacaatcggctgctctgatgccgccgtgttccggctgtcagcgcaggggcgcccggttctttttgtcaagaccgacctgtccggtgccctgaatgaactccaggacgaggcagcgcggctatcgtggctggccacgacgggcgttccttgcgctgctgtgctcgacgttgtcactgaagcgggaagggactggctgctattgggcgaagtgccggggcaggatctcctgtcatctcaccttgctcctgccgagaaagtatccatcatggctgatgcaatgcggcggctgcatacgcttgatccggctacctgcccattcgaccaccaagcgaaacatcgcatcgagcgagcacgtactcggatggaagccggtcttgtcgatcaggatgatctggacgaagagcatcaggggctcgcgccagccgaactgttcgccaggctcaaggcgcgcatgcccgacggcgatgatctcgtcgtgacccatggcgatgcctgcttgccgaatatcatggtggaaaatggccgcttttctggattcatcgactgtggccggctgggtgtggcggaccgctatcaggacatagcgttggctacccgtgatattgctgaagagcttggcggcgaatgggctgaccgcttcctcgtgctttacggtatcgccgctcccgattcgcagcgcatcgccttctatcgccttcttgacgagttcttctgagcgggactctggggttcgaaatgaccgaccaagcgacgcccaacctgccatcacgagatttcgattccaccgccgccttctatgaaaggttgggcttcggaatcgttttccgggacgccggctggatgatcctccagcgcggggatctcatgctggagttcttcgcccacgggatctctgcggaacaggcggtcgaaggtgccgatattattacgacagcaacggccgacaagcacaacgccacgatcctgagcgacaatatgatcggacccggcgtccacatcaacggcgtcggcggcgactgcccaggcaagaccgagatgcaccgcgatatattgctgcgttcggatattttcgtggagttcccgccacagacccggatgatccccgaccgttcaaacatttggcaataaagtttctaaagattgaatcctgttgccggtcttgcgatgattatcatataatttctgttgaattacgttaagcatgtaataattaacatgtaatgcatgacgttatttatgagatgggtttttatgattagagtcccgcaattatacatttaatacgcgatagaaaacaaaatatagcgcgcaaactaggataaattatcgcgcgcggtgtcatctatgttactagatcgggcctcctgatatcaatgctgcagcggcggctctggtggtggttctggtggcggctctgagggtggtggctctgagggtggcggttctgagggtggcggctctgagggaggcggttccggtggtggctctggttccggtgattttgattatgaaaagatggcaaacgctaataagggggctatgaccgaaaatgccgatgaaaacgcgctacagtctgacgctaaaggcaaacttgattctgtcgctactgattacggtgctgctatgatggtttcattggtgacgtttccggccttgctaatggtaatggtgctactggtgattttgctggctctaattcccaaatggctcaagtcggtgacggtgataattcacctttaatgaatatttccgtcaatatttaccttccctccctcaatcggttgaatgtcgcccttttgtctttggcccaatacgcaaaccgcctctccccgcgcgttggccgattcattatgcactggcacgacaggtttcccgactggaaagcgggcagtgagcgcaacgcaattatgtgagttagctcactcattaggcaccccaggctttacactttatgcttccggctcgtatgttgtgtggaattgtgagcggataacaatttcacacaggaaacagctatgaccatgattacgccaagctggcgcca

SEQ ID NO: 39 - DNA, 1200 bp, Artificial Sequence
  cation efflux antisense (AS) sequence
tcaaaaagctcgctcaacttcagggagttgctccaatttttcttgcagtgtctcaccaatattatgtgccttgttcaacagcatgtcctctggcaacactatatcaacctctacaaaataatgagcaccaaaagtatatgctcgaacagtatcaatgtgcttgatctcttcgtgatgattccatataagataggttaatttcgtaagaaaatctggtggagctgttcttccaatgagtgaccagacattttctgccactgtcttcgcccacgtgctaattgtgtacatagctataattatagctcccgtaggatcaatccaccagtagaatcggactgctaagacagcagtcactaatccaactgagttggtgatgacatcaaagaaatgatcttgagcataggctcttacgatttcgtttttgaaccttcgacagtagaccataagcagaaacttgaccatagtgacagagaccataataccaatcgtccatttttccttctcatggtccatctcagggcgagacttagttatgagttctttagctgactcgaacaatatttgtaatcctagtgtcgccattacagatgcaaaaacaataatacccaatggctgcatcctcttttttccaataggatagtgatactggtttggatttttcatggcatgagaagtgaaccacagtataaaccctgataagaggtctaagagggagtccaacgttgacgcgattacagccaaagatctgctctcaatagaagcgtagatttttgcaatgaaaagaaccacattagccatgtttgataaatgaatagccatcctttcacttcttgcaagctgcttcatttcatcctcagttagacttccaggtaaacaaccagattcattaatggtgtccatctcattgaacccttcaagcagcctttcttgttttttgtagtattcagcaattttaccttgtttcctgggagtgggaagtagacgacggacactaaaggagtgatgatcggaggaggagcggcttcgttcgggaagacggaattcgctaatgttaagtctccatgacgccgacgaagacgactgatccaccaccgcctgagcagccggagacagcagttccgtcctaaaactgctaaaactgtcgtccagagcgccgccgctgccgccaccaccactaacattgctgcgacttatctccat

SEQ ID NO: 40 - DNA, 41 bp, Artificial Sequence
  primer AS.fw
tgtacaaaaaagcaggctcatcaaaaagctcgctcaacttc

SEQ ID NO: 41 - DNA, 39 bp, Artificial Sequence
  primer AS.rv
tgtacaagaaagctgggtatggagataagtcgcagcaat

SEQ ID NO: 42 - DNA, 29 bp, Artificial Sequence
  primer attB1
ggggacaagtttgtacaaaaaagcaggct

SEQ ID NO: 43 - DNA, 29 bp, Artificial Sequence
  primer attB2
ggggaccactttgtacaagaaagctgggt

SEQ ID NO: 44 - DNA, 1653 bp, Artificial Sequence
  luciferase control sequence
atggaagacgccaaaaacataaagaaaggcccggcgccattctatccgctggaagatggaaccgctggagagcaactgcataaggctatgaagagatacgccctggttcctggaacaattgcttttacagatgcacatatcgaggtggacattacgtacgctgagtacttcgaaatgtccgttcggttggcagaagctatgaaacgatatgggctgaatacaaatcacagaatcgtcgtatgcagtgaaaactctcttcaattctttatgccggtgttgggcgcgttatttatcggagttgcagttgcgcccgcgaacgacatttataatgaacgtgaattgctcaacagtatgggcatttcgcagcctaccgtggtgttcgtttccaaaaaggggttgcaaaaaattttgaacgtgcaaaaaaagctcccaatcatccaaaaaattattatcatggattctaaaacggattaccagggatttcagtcgatgtacacgttcgtcacatctcatctacctcccggttttaatgaatacgattttgtgccagagtccttcgatagggacaagacaattgcactgatcatgaactcctctggatctactggtctgcctaaaggtgtcgctctgcctcatagaactgcctgcgtgagattctcgcatgccagagatcctatttttggcaatcaaatcattccggatactgcgattttaagtgttgttccattccatcacggttttggaatgtttactacactcggatatttgatatgtggatttcgagtcgtcttaatgtatagatttgaagaagagctgtttctgaggagccttcaggattacaagattcaaagtgcgctgctggtgccaaccctattctccttcttcgccaaaagcactctgattgacaaatacgatttatctaatttacacgaaattgcttctggtggcgctcccctctctaaggaagtcggggaagcggttgccaagaggttccatctgccaggtatcaggcaaggatatgggctcactgagactacatcagctattctgattacacccgagggggatgataaaccgggcgcggtcggtaaagttgttccattttttgaagcgaaggttgtggatctggataccgggaaaacgctgggcgttaatcaaagaggcgaactgtgtgtgagaggtcctatgattatgtccggttatgtaaacaatccggaagcgaccaacgccttgattgacaaggatggatggctacattctggagacatagcttactgggacgaagacgaacacttcttcatcgttgaccgcctgaagtctctgattaagtacaaaggctatcaggtggctcccgctgaattggaatccatcttgctccaacaccccaacatcttcgacgcaggtgtcgcaggtcttcccgacgatgacgccggtgaacttcccgccgccgttgttgttttggagcacggaaagacgatgacggaaaaagagatcgtggattacgtcgccagtcaagtaacaaccgcgaaaaagttgcgcggaggagttgtgtttgtggacgaagtaccgaaaggtcttaccggaaaactcgacgcaagaaaaatcagagagatcctcataaaggccaagaagggcggaaagatcgccgtgtaa

SEQ ID NO: 45 - DNA, 41 bp, Artificial Sequence
  primer delta 117C fw
tgtacaaaaaagcaggctcaatggagataagtcgcagcaat

SEQ ID NO: 46 - DNA, 40 bp, Artificial Sequence
  primer delta 117C rv
tgtacaagaaagctgggttttaagctcccgtaggatcaat

SEQ ID NO: 47 - DNA, 41 bp, Artificial Sequence
  primer delta 117N fw
tgtacaaaaaagcaggctcaatggaaatgaagcagcttgca

SEQ ID NO: 48 - DNA, 42 bp, Artificial Sequence
  primer delta 117N rv
tgtacaagaaagctgggttttataccatagttttgtgttctg

SEQ ID NO: 49 - DNA, 20173 bp, Tobacco rattle virus
tactccaaaaatgtcaaagatacagtctcagaagaccaaagggctattgagacttttcaacaaagggtaatttcgggaaacctcctcggattccattgcccagctatctgtcacttcatcgaaaggacagtagaaaaggaaggtggctcctacaaatgccatcattgcgataaaggaaaggctatcattcaagatgcctctgccgacagtggtcccaaagatggacccccacccacgaggagcatcgtggaaaaagaagacgtcccaaccacgtcttcaaagcaagtggattgatgtgacatctccactgacgtaagggatgacgcacaatcccactatccttcgcaagacccttcttctatataaggaagttcatttcatttggagaggacagcccaagctttctagaggatccataaaacatttcaatcctttgaacgcggtagaacgtgctaattggattttggtgagaacgcggtagaacgtacttatcacctacagttttattttgtttttctttttggtttaatctatccagcttagtaccgagtgggggaaagtgactggtgtgcctaaaaccttttctttgatactttgtaaaaatacatacagatacaatggcgaacggtaacttcaagttgtctcaattgctcaatgtggacgagatgtctgctgagcagaggagtcatttctttgacttgatgctgactaaacctgattgtgagatcgggcaaatgatgcaaagagttgttgttgataaagtcgatgacatgattagagaaagaaagactaaagatccagtgattgttcatgaagttctttctcagaaggaacagaacaagttgatggaaatttatcctgaattcaatatcgtgtttaaagacgacaaaaacatggttcatgggtttgcggctgctgagcgaaaactacaagctttattgcttttagatagagttcctgctctgcaagaggtggatgacatcggtggtcaatggtcgttttgggtaactagaggtgagaaaaggattcattcctgttgtccaaatctagatattcgggatgatcagagagaaatttctcgacagatatttcttactgctattggtgatcaagctagaagtggtaagagacagatgtcggagaatgagctgtggatgtatgaccaatttcgtgaaaatattgctgcgcctaacgcggttaggtgcaataatacatatcagggttgtacatgtaggggtttttctgatggtaagaagaaaggcgcgcagtatgcgatagctcttcacagcctgtatgacttcaagttgaaagacttgatggctactatggttgagaagaaaactaaagtggttcatgctgctatgctttttgctcctgaaagtatgttagtggacgaaggtccattaccttctgttgacggttactacatgaagaagaacgggaagatctatttcggttttgagaaagatccttccttttcttacattcatgactgggaagagtacaagaagtatctactggggaagccagtgagttaccaagggaatgtgttctacttcgaaccgtggcaggtgagaggagacacaatgcttttttcgatctacaggatagctggagttccgaggaggtctctatcatcgcaagagtactaccgaagaatatatatcagtagatgggaaagcatggttgttgtcccaattttcgatctggtcgaatcaacgcgagagttggtcaagaaagacctgtttgtaagaaacaattcatggacaagtgtttggattacatagctaggttatctgaccagcagctgaccataagcaatgttaaatcatacttgagttcaaataattgggtcttattcataaacggggcggccgtgaagaacaagcaaagtgtagattctcgagatttacagttgttggctcaaactttgctagtgaaggaacaagtggcgagacctgtcatgagggagttgcgtgaagcaattctgactgagacgaaacctatcacgtcattgactgatgtgctgggtttaatatcaagaaaactgtggaagcagtttgctaacaagatcgcagtcggcggattcgttggcatggttggtactctaattggattctatccaaagaaggtactaacctgggcgaaggacacaccaaatggtccagaactatgttacgagaactcgcacaaaaccaaggtgatagtatttctgagtgttgtgtatgccattggaggaatcacgcttatgcgtcgagacatccgagatggactggtgaaaaaactatgtgatatgtttgatatcaaacggggggcccatgtcttagacgttgagaatccgtgccgctattatgaaatcaacgatttctttagcagtctgtattcggcatctgagtccggtgagaccgttttaccagatttatccgaggtaaaagccaagtctgataagctattgcagcagaagaaagaaatcgctgacgagtttctaagtgcaaaattctctaactattctggcagttcggtgagaacttctccaccatcggtggtcggttcatctcgaagcggactgggtctgttgttggaagacagtaacgtgctgacccaagctagagttggagtttcaagaaaggtagacgatgaggagatcatggagcagtttctgagtggtcttattgacactgaagcagaaattgacgaggttgtttcagccttttcagctgaatgtgaaagaggggaaacaagcggtacaaaggtgttgtgtaaacctttaacgccaccaggatttgagaacgtgttgccagctgtcaaacctttggtcagcaaaggaaaaacggtcaaacgtgtcgattacttccaagtgatgggaggtgagagattaccaaaaaggccggttgtcagtggagacgattctgtggacgctagaagagagtttctgtactacttagatgcggagagagtcgctcaaaatgatgaaattatgtctctgtatcgtgactattcgagaggagttattcgaactggaggtcagaattacccgcacggactgggagtgtgggatgtggagatgaagaactggtgcatacgtccagtggtcactgaacatgcttatgtgttccaaccagacaaacgtatggatgattggtcgggatacttagaagtggctgtttgggaacgaggtatgttggtcaacgacttcgcggtcgaaaggatgagtgattatgtcatagtttgcgatcagacgtatctttgcaataacaggtaataatcctctctcttgatatttttaaattatagaattaattagtttactttattctttactatatgatttaaatagtttaatcttgtttttgagtaaactattcgattttgatatttgtattcgtcctacaaagttggaaatactgatgatattttcttttgaacgtgatacctaccaatactaatcttacggaatcttttaatagagcactaatcaacatggaactaaagaccaattcttaagtgtctctgttgtacagttcattttagtagtgcgtttaagtattattatctcccttcatgcggggcaattatgtagattaaaatcgaaattatataaaatttacataagtctaagtctagggtctccagctaattgttatttttttaacgatgttgactaaagcaataacgacgttgacttgtgttaaacaggttgatcttggacaatttaagtgccctggatctaggaccagttaactgttcttttgaattagttgacggtgtacctggttgtggtaagtcgacaatgattgtcaactcagctaatccttgtgtcgatgtggttctctctactgggagagcagcaaccgacgacttgatcgagagattcgcgagcaaaggttttccatgcaaattgaaaaggagagtgaagacggttgattcttttttgatgcattgtgtcgatggttctttaaccggagacgtgttgcatttcgacgaagctctcatggcccatgctggtatggtgtacttttgcgctcagatagctggtgctaaacgatgtatctgtcaaggagatcagaatcaaatttctttcaagcctagggtatctcaagttgatttgaggttttctagtctggtcggaaagtttgacattgttacagaaaaaagagaaacttacagaagtccagcagatgtggctgccgtattgaacaagtactatactggagatgtcagaacacataacgcgactgctaattcgatgacggtgaggaagattgtgtctaaagaacaggtttctttgaagcctggtgctcagtacataactttccttcagtctgagaagaaggagttggtaaatttgttggcattgaggaaagtggcagctaaagtgagtacagtacacgagtcgcaaggagagacattcaaagatgtagtcctagtcaggacgaaacctacggatgactcaatcgctagaggtcgggagtacttaatcgtggcattgtcgcgtcacacacaatcacttgtgtatgaaactgtgaaagaggacgatgtaagcaaagagatcagggaaagtgccgcgcttacgaaggcggctttggcaagattttttgttactgagaccgtcttatgacggtttcggtctaggtttgatgtctttagacatcatgaagggccttgcgccgttccagattcaggtacgattacggacttggagatgtggtacgacgctttgtttccgggaaattcgttaagagactcaagcctagacgggtatttggtggcaacgactgattgcaatttgcgattagacaatgttacgatcaaaagtggaaactggaaagacaagtttgctgaaaaagaaacgtttctgaaaccggttattcgtactgctatgcctgacaaaaggaagactactcagttggagagtttgttagcattgcagaaaaggaaccaagcggcacccgatctacaagaaaatgtgcacgcgacagttctaatcgaagagacgatgaagaagctgaaatctgttgtctacgatgtgggaaaaattcgggctgatcctattgtcaatagagctcaaatggagagatggtggagaaatcaaagcacagcggtacaggctaaggtagtagcagatgtgagagagttacatgaaatagactattcgtcttacatgtatatgatcaaatctgacgtgaaacctaagactgatttaacaccgcaatttgaatactcagctctacagactgttgtgtatcacgagaagttgatcaactcgttgttcggtccaattttcaaagaaattaatgaacgcaagttggatgctatgcaaccacattttgtgttcaacacgagaatgacatcgagtgatttaaacgatcgagtgaagttcttaaatacggaagcggcttacgactttgttgagatagacatgtctaaattcgacaagtcggcaaatcgcttccatttacaactgcagctggagatttacaggttatttgggctggatgagtgggcggccttcctttgggaggtgtcgcacactcaaactactgtgagagatattcaaaatggtatgatggcgcatatttggtaccaacaaaagagtggagatgctgatacttataatgcaaattcagatagaacactgtgtgcactcttgtctgaattaccattggagaaagcagtcatggttacatatggaggagatgactcactgattgcgtttcctagaggaacgcagtttgttgatccgtgtccaaagttggctactaagtggaatttcgagtgcaagatttttaagtacgatgtcccaatgttttgtgggaagttcttgcttaagacgtcatcgtgttacgagttcgtgccagatccggtaaaagttctgacgaagttggggaaaaagagtataaaggatgtgcaacatttagccgagatctacatctcgctgaatgattccaatagagctcttgggaactacatggtggtatccaaactgtccgagtctgtttcagaccggtatttgtacaaaggtgattctgttcatgcgctttgtgcgctatggaagcatattaagagttttacagctctgtgtacattattccgagacgaaaacgataaggaattgaacccggctaaggttgattggaagaaggcacagagagctgtgtcaaacttttacgactggtaatatggaagacaagtcattggtcaccttgaagaagaagactttcgaagtctcaaaattctcaaatctaggggccattgaattgtttgtggacggtaggaggaagagaccgaagtattttcacagaagaagagaaactgtcctaaatcatgttggtgggaagaagagtgaacacaagttagacgtttttgaccaaagggattacaaaatgattaaatcttacgcgtttctaaaggtagtaggtgtacaactagttgtaacatcacatctacctgcagatacgcctgggttcattcaaatcgatctgttggattcgagacttactgagaaaagaaagagaggaaagactattcagagattcaaagctcgagcttgcgataactgttcagttgcgcagtacaaggttgaatacagtatttccacacaggagaacgtacttgatgtctggaaggtgggttgtatttctgagggcgttccggtctgtgacggtacataccctttcagtatcgaagtgtcgctaatatgggttgctactgattcgactaggcgcctcaatgtggaagaactgaacagttcggattacattgaaggcgattttaccgatcaagaggttttcggtgagttcatgtctttgaaacaagtggagatgaagacgattgaggcgaagtacgatggtccttacagaccagctactactagacctaagtcattattgtcaagtgaagatgttaagagagcgtctaataagaaaaactcgtcttaatgcataaagaaatttattgtcaatatgacgtgtgtactcaagggttgtgtgaatgaagtcactgttcttggtcacgagacgtgtagtatcggtcatgctaacaaattgcgaaagcaagttgctgacatggttggtgtcacacgtaggtgtgcggaaaataattgtggatggtttgtctgtgttgttatcaatgattttacttttgatgtgtataattgttgtggccgtagtcaccttgaaaagtgtcgtaaacgtgttgaaacaagaaatcgagaaatttggaaacaaattcgacgaaatcaagctgaaaacatgtctgcgacagctaaaaagtctcataattcgaagacctctaagaagaaattcaaagaggacagagaatttgggacaccaaaaagatttttaagagatgatgttcctttcgggattgatcgtttgtttgctttttgattttattttatattgttatctgtttctgtgtatagactgtttgagattggcgcttggccgactcattgtcttaccataggggaacggactttgtttgtgttgttattttatttgtattttattaaaattctcaatgatctgaaaaggcctcgaggctaagagattattggggggtgagtaagtacttttaaagtgatgatggttacaaaggcaaaaggggtaaaacccctcgcctacgtaagcgttattacgcccggatcccccggggagctcgaattcgctgaaatcaccagtctctctctacaaatctatctctctctattttttccataaataatgtgtgagtagtttcccgataagggaaattagggttcttatagggtttcgctcatgtgttgagcatataagaaacccttagtatgtatttgtatttgtaaaatacttctattatcaataaaatttctaattcctaaaaccaaaatccagtactaaaatccagatctcctaaagtccctatagatctttgtcgtgaatataaaccagacacgagacgactaaacctggagcccagacgccgttcgaagctagaagtaccgcttaggcaggaggccgttagggaaaagatgctaaggcagggttggttacgttgactcccccgtaggtttggtttaaatatgatgaagtggacggaaggaaggaggaagacaaggaaggataaggttgcaggccctgtgcaaggtaagaagatggaaatttgatagaggtacgctactatacttatactatacgctaagggaatgcttgtatttataccctataccccctaataaccccttatcaatttaagaaataatccgcataagcccccgcttaaaaattggtatcagagccatgaataggtctatgaccaaaactcaagaggataaaacctcaccaaaatacgaaagagttcttaactctaaagataaaagatctttcaagatcaaaactagttccctcacaccggagcatgcgatatcctcgacctgcaggcatgcaagcttggcgtaatcatggtcatagctgtttcctgtgtgaaattgttatccgctcacaattccacacaacatacgagccggaagcataaagtgtaaagcctggggtgcctaatgagtgagctaactcacattaattgcgttgcgctcactgcccgctttccagtcgggaaacctgtcgtgccagctgcattaatgaatcggccaacgcgcggggagaggcggtttgcgtattgggccaaagacaaaagggcgacattcaaccgattgagggagggaaggtaaatattgacggaaattattcattaaaggtgaattatcaccgtcaccgacttgagccatttgggaattagagccagcaaaatcaccagtagcaccattaccattagcaaggccggaaacgtcaccaatgaaaccatcgatagcagcaccgtaatcagtagcgacagaatcaagtttgcctttagcgtcagactgtagcgcgttttcatcggcattttcggtcatagcccccttattagcgtttgccatcttttcataatcaaaatcaccggaaccagagccaccaccggaaccgcctccctcagagccgccaccctcagaaccgccaccctcagagccaccaccctcagagccgccaccagaaccaccaccagagccgccgccagcattgacaggaggcccgatctagtaacatagatgacaccgcgcgcgataatttatcctagtttgcgcgctatattttgttttctatcgcgtattaaatgtataattgcgggactctaatcataaaaacccatctcataaataacgtcatgcattacatgttaattattacatgcttaacgtaattcaacagaaattatatgataatcatcgcaagaccggcaacaggattcaatcttaagaaactttattgccaaatgtttgaacgatcggggatcatccgggtctgtggcgggaactccacgaaaatatccgaacgcagcaagatatcgcggtgcatctcggtcttgcctgggcagtcgccgccgacgccgttgatgtggacgccgggcccgatcatattgtcgctcaggatcgtggcgttgtgcttgtcggccgttgctgtcgtaatgatatcggcaccttcgaccgcctgttccgcagagatcccgtgggcgaagaactccagcatgagatccccgcgctggaggatcatccagccggcgtcccggaaaacgattccgaagcccaacctttcatagaaggcggcggtggaatcgaaatctcgtgatggcaggttgggcgtcgcttggtcggtcatttcgaaccccagagtcccgctcagaagaactcgtcaagaaggcgatagaaggcgatgcgctgcgaatcgggagcggcgataccgtaaagcacgaggaagcggtcagcccattcgccgccaagctcttcagcaatatcacgggtagccaacgctatgtcctgatagcggtccgccacacccagccggccacagtcgatgaatccagaaaagcggccattttccaccatgatattcggcaagcaggcatcgccatgggtcacgacgagatcatcgccgtcgggcatgcgcgccttgagcctggcgaacagttcggctggcgcgagcccctgatgctcttcgtccagatcatcctgatcgacaagaccggcttccatccgagtacgtgctcgctcgatgcgatgtttcgcttggtggtcgaatgggcaggtagccggatcaagcgtatgcagccgccgcattgcatcagccatgatggatactttctcggcaggagcaaggtgagatgacaggagatcctgccccggcacttcgcccaatagcagccagtcccttcccgcttcagtgacaacgtcgagcacagctgcgcaaggaacgcccgtcgtggccagccacgatagccgcgctgcctcgtcctgcagttcattcagggcaccggacaggtcggtcttgacaaaaagaaccgggcgcccctgcgctgacagccggaacacggcggcatcagagcagccgattgtctgttgtgcccagtcatagccgaatagcctctccacccaagcggccggagaacctgcgtgcaatccatcttgttcaatcatgcgaaacgatccagatccggtgcagattatttggattgagagtgaatatgagactctaattggataccgaggggaatttatggaacgtcagtggagcatttttgacaagaaatatttgctagctgatagtgaccttaggcgacttttgaacgcgcaataatggtttctgacgtatgtgcttagctcattaaactccagaaacccgcggctgagtggctccttcaacgttgcggttctgtcagttccaaacgtaaaacggcttgtcccgcgtcatcggcgggggtcataacgtgactcccttaattctccgctcatgatcagattgtcgtttcccgccttcagtttaaactatcagtgtttgacaggatatattggcgggtaaacctaagagaaaagagcgtttattagaataatcggatatttaaaagggcgtgaaaaggtttatccgttcgtccatttgtatgtgcatgccaaccacagggttccccagatctggcgccggccagcgagacgagcaagattggccgccgcccgaaacgatccgacagcgcgcccagcacaggtgcgcaggcaaattgcaccaacgcatacagcgccagcagaatgccatagtgggcggtgacgtcgttcgagtgaaccagatcgcgcaggaggcccggcagcaccggcataatcaggccgatgccgacagcgtcgagcgcgacagtgctcagaattacgatcaggggtatgttgggtttcacgtctggcctccggaccagcctccgctggtccgattgaacgcgcggattctttatcactgataagttggtggacatattatgtttatcagtgataaagtgtcaagcatgacaaagttgcagccgaatacagtgatccgtgccgccctggacctgttgaacgaggtcggcgtagacggtctgacgacacgcaaactggcggaacggttgggggttcagcagccggcgctttactggcacttcaggaacaagcgggcgctgctcgacgcactggccgaagccatgctggcggagaatcatacgcattcggtgccgagagccgacgacgactggcgctcatttctgatcgggaatgcccgcagcttcaggcaggcgctgctcgcctaccgcgatggcgcgcgcatccatgccggcacgcgaccgggcgcaccgcagatggaaacggccgacgcgcagcttcgcttcctctgcgaggcgggtttttcggccggggacgccgtcaatgcgctgatgacaatcagctacttcactgttggggccgtgcttgaggagcaggccggcgacagcgatgccggcgagcgcggcggcaccgttgaacaggctccgctctcgccgctgttgcgggccgcgatagacgccttcgacgaagccggtccggacgcagcgttcgagcagggactcgcggtgattgtcgatggattggcgaaaaggaggctcgttgtcaggaacgttgaaggaccgagaaagggtgacgattgatcaggaccgctgccggagcgcaacccactcactacagcagagccatgtagacaacatcccctccccctttccaccgcgtcagacgcccgtagcagcccgctacgggctttttcatgccctgccctagcgtccaagcctcacggccgcgctcggcctctctggcggccttctggcgctcttccgcttcctcgctcactgactcgctgcgctcggtcgttcggctgcggcgagcggtatcagctcactcaaaggcggtaatacggttatccacagaatcaggggataacgcaggaaagaacatgtgagcaaaaggccagcaaaaggccaggaaccgtaaaaaggccgcgttgctggcgtttttccataggctccgcccccctgacgagcatcacaaaaatcgacgctcaagtcagaggtggcgaaacccgacaggactataaagataccaggcgtttccccctggaagctccctcgtgcgctctcctgttccgaccctgccgcttaccggatacctgtccgcctttctcccttcgggaagcgtggcgcttttccgctgcataaccctgcttcggggtcattatagcgattttttcggtatatccatcctttttcgcacgatatacaggattttgccaaagggttcgtgtagactttccttggtgtatccaacggcgtcagccgggcaggataggtgaagtaggcccacccgcgagcgggtgttccttcttcactgtcccttattcgcacctggcggtgctcaacgggaatcctgctctgcgaggctggccggctaccgccggcgtaacagatgagggcaagcggatggctgatgaaaccaagccaaccaggaagggcagcccacctatcaaggtgtactgccttccagacgaacgaagagcgattgaggaaaaggcggcggcggccggcatgagcctgtcggcctacctgctggccgtcggccagggctacaaaatcacgggcgtcgtggactatgagcacgtccgcgagctggcccgcatcaatggcgacctgggccgcctgggcggcctgctgaaactctggctcaccgacgacccgcgcacggcgcggttcggtgatgccacgatcctcgccctgctggcgaagatcgaagagaagcaggacgagcttggcaaggtcatgatgggcgtggtccgcccgagggcagagccatgacttttttagccgctaaaacggccggggggtgcgcgtgattgccaagcacgtccccatgcgctccatcaagaagagcgacttcgcggagctggtgaagtacatcaccgacgagcaaggcaagaccgagcgcctttgcgacgctcaccgggctggttgccctcgccgctgggctggcggccgtctatggccctgcaaacgcgccagaaacgccgtcgaagccgtgtgcgagacaccgcggccgccggcgttgtggatacctcgcggaaaacttggccctcactgacagatgaggggcggacgttgacacttgaggggccgactcacccggcgcggcgttgacagatgaggggcaggctcgatttcggccggcgacgtggagctggccagcctcgcaaatcggcgaaaacgcctgattttacgcgagtttcccacagatgatgtggacaagcctggggataagtgccctgcggtattgacacttgaggggcgcgactactgacagatgaggggcgcgatccttgacacttgaggggcagagtgctgacagatgaggggcgcacctattgacatttgaggggctgtccacaggcagaaaatccagcatttgcaagggtttccgcccgtttttcggccaccgctaacctgtcttttaacctgcttttaaaccaatatttataaaccttgtttttaaccagggctgcgccctgtgcgcgtgaccgcgcacgccgaaggggggtgcccccccttctcgaaccctcccggcccgctaacgcgggcctcccatccccccaggggctgcgcccctcggccgcgaacggcctcaccccaaaaatggcagcgctggcagtccttgccattgccgggatcggggcagtaacgggatgggcgatcagcccgagcgcgacgcccggaagcattgacgtgccgcaggtgctggcatcgacattcagcgaccaggtgccgggcagtgagggcggcggcctgggtggcggcctgcccttcacttcggccgtcggggcattcacggacttcatggcggggccggcaatttttaccttgggcattcttggcatagtggtcgcgggtgccgtgctcgtgttcgggggtgcgataaacccagcgaaccatttgaggtgataggtaagattataccgaggtatgaaaacgagaattggacctttacagaattactctatgaagcgccatatttaaaaagctaccaagacgaagaggatgaagaggatgaggaggcagattgccttgaatatattgacaatactgataagataatatatcttttatatagaagatatcgccgtatgtaaggatttcagggggcaaggcataggcagcgcgcttatcaatatatctatagaatgggcaaagcataaaaacttgcatggactaatgcttgaaacccaggacaataaccttatagcttgtaaattctatcataattgggtaatgactccaacttattgatagtgttttatgttcagataatgcccgatgactttgtcatgcagctccaccgattttgagaacgacagcgacttccgtcccagccgtgccaggtgctgcctcagattcaggttatgccgctcaattcgctgcgtatatcgcttgctgattacgtgcagctttcccttcaggcgggattcatacagcggccagccatccgtcatccatatcaccacgtcaaagggtgacagcaggctcataagacgccccagcgtcgccatagtgcgttcaccgaatacgtgcgcaacaaccgtcttccggagactgtcatacgcgtaaaacagccagcgctggcgcgatttagccccgacatagccccactgttcgtccatttccgcgcagacgatgacgtcactgcccggctgtatgcgcgaggttaccgactgcggcctgagttttttaagtgacgtaaaatcgtgttgaggccaacgcccataatgcgggctgttgcccggcatccaacgccattcatggccatatcaatgattttctggtgcgtaccgggttgagaagcggtgtaagtgaactgcagttgccatgttttacggcagtgagagcagagatagcgctgatgtccggcggtgcttttgccgttacgcaccaccccgtcagtagctgaacaggagggacagctgatagacacagaagccactggagcacctcaaaaacaccatcatacactaaatcagtaagttggcagcatcacccataattgtggtttcaaaatcggctccgtcgatactatgttatacgccaactttgaaaacaactttgaaaaagctgttttctggtatttaaggttttagaatgcaaggaacagtgaattggagttcgtcttgttataattagcttcttggggtatctttaaatactgtagaaaagaggaaggaaataataaatggctaaaatgagaatatcaccggaattgaaaaaactgatcgaaaaataccgctgcgtaaaagatacggaaggaatgtctcctgctaaggtatataagctggtgggagaaaatgaaaacctatatttaaaaatgacggacagccggtataaagggaccacctatgatgtggaacgggaaaaggacatgatgctatggctggaaggaaagctgcctgttccaaaggtcctgcactttgaacggcatgatggctggagcaatctgctcatgagtgaggccgatggcgtcctttgctcggaagagtatgaagatgaacaaagccctgaaaagattatcgagctgtatgcggagtgcatcaggctctttcactccatcgacatatcggattgtccctatacgaatagcttagacagccgcttagccgaattggattacttactgaataacgatctggccgatgtggattgcgaaaactgggaagaagacactccatttaaagatccgcgcgagctgtatgattttttaaagacggaaaagcccgaagaggaacttgtcttttcccacggcgacctgggagacagcaacatctttgtgaaagatggcaaagtaagtggctttattgatcttgggagaagcggcagggcggacaagtggtatgacattgccttctgcgtccggtcgatcagggaggatatcggggaagaacagtatgtcgagctattttttgacttactggggatcaagcctgattgggagaaaataaaatattatattttactggatgaattgttttagtacctagatgtggcgcaacgatgccggcgacaagcaggagcgcaccgacttcttccgcatcaagtgttttggctctcaggccgaggcccacggcaagtatttgggcaaggggtcgctggtattcgtgcagggcaagattcggaataccaagtacgagaaggacggccagacggtctacgggaccgacttcattgccgataaggtggattatctggacaccaaggcaccaggcgggtcaaatcaggaataagggcacattgccccggcgtgagtcggggcaatcccgcaaggagggtgaatgaatcggacgtttgaccggaaggcatacaggcaagaactgatcgacgcggggttttccgccgaggatgccgaaaccatcgcaagccgcaccgtcatgcgtgcgccccgcgaaaccttccagtccgtcggctcgatggtccagcaagctacggccaagatcgagcgcgacagcgtgcaactggctccccctgccctgcccgcgccatcggccgccgtggagcgttcgcgtcgtctcgaacaggaggcggcaggtttggcgaagtcgatgaccatcgacacgcgaggaactatgacgaccaagaagcgaaaaaccgccggcgaggacctggcaaaacaggtcagcgaggccaagcaggccgcgttgctgaaacacacgaagcagcagatcaaggaaatgcagctttccttgttcgatattgcgccgtggccggacacgatgcgagcgatgccaaacgacacggcccgctctgccctgttcaccacgcgcaacaagaaaatcccgcgcgaggcgctgcaaaacaaggtcattttccacgtcaacaaggacgtgaagatcacctacaccggcgtcgagctgcgggccgacgatgacgaactggtgtggcagcaggtgttggagtacgcgaagcgcacccctatcggcgagccgatcaccttcacgttctacgagctttgccaggacctgggctggtcgatcaatggccggtattacacgaaggccgaggaatgcctgtcgcgcctacaggcgacggcgatgggcttcacgtccgaccgcgttgggcacctggaatcggtgtcgctgctgcaccgcttccgcgtcctggaccgtggcaagaaaacgtcccgttgccaggtcctgatcgacgaggaaatcgtcgtgctgtttgctggcgaccactacacgaaattcatatgggagaagtaccgcaagctgtcgccgacggcccgacggatgttcgactatttcagctcgcaccgggagccgtacccgctcaagctggaaaccttccgcctcatgtgcggatcggattccacccgcgtgaagaagtggcgcgagcaggtcggcgaagcctgcgaagagttgcgaggcagcggcctggtggaacacgcctgggtcaatgatgacctggtgcattgcaaacgctagggccttgtggggtcagttccggctgggggttcagcagccagcgctttactggcatttcaggaacaagcgggcactgctcgacgcacttgcttcgctcagtatcgctcgggacgcacggcgcgctctacgaactgccgataaacagaggattaaaattgacaattgtgattaaggctcagattcgacggcttggagcggccgacgtgcaggatttccgcgagatccgattgtcggccctgaagaaagctccagagatgttcgggtccgtttacgagcacgaggagaaaaagcccatggaggcgttcgctgaacggttgcgagatgccgtggcattcggcgcctacatcgacggcgagatcattgggctgtcggtcttcaaacaggaggacggccccaaggacgctcacaaggcgcatctgtccggcgttttcgtggagcccgaacagcgaggccgaggggtcgccggtatgctgctgcgggcgttgccggcgggtttattgctcgtgatgatcgtccgacagattccaacgggaatctggtggatgcgcatcttcatcctcggcgcacttaatatttcgctattctggagcttgttgtttatttcggtctaccgcctgccgggcggggtcgcggcgacggtaggcgctgtgcagccgctgatggtcgtgttcatctctgccgctctgctaggtagcccgatacgattgatggcggtcctgggggctatttgcggaactgcgggcgtggcgctgttggtgttgacaccaaacgcagcgctagatcctgtcggcgtcgcagcgggcctggcgggggcggtttccatggcgttcggaaccgtgctgacccgcaagtggcaacctcccgtgcctctgctcacctttaccgcctggcaactggcggccggaggacttctgctcgttccagtagctttagtgtttgatccgccaatcccgatgcctacaggaaccaatgttctcggcctggcgtggctcggcctgatcggagcgggtttaacctacttcctttggttccgggggatctcgcgactcgaacctacagttgtttccttactgggctttctcagccccagatctggggtcgatcagccggggatgcatcaggccgacagtcggaacttcgggtccccgacctgtaccattcggtgagcaatggataggggagttgatatcgtcaacgttcacttctaaagaaatagcgccactcagcttcctcagcggctttatccagcgatttcctattatgtcggcatagttctcaagatcgacagcctgtcacggttaagcgagaaatgaataagaaggctgataattcggatctctgcgagggagatgatatttgatcacaggcagcaacgctctgtcatcgttacaatcaacatgctaccctccgcgagatcatccgtgtttcaaacccggcagcttagttgccgttcttccgaatagcatcggtaacatgagcaaagtctgccgccttacaacggctctcccgctgacgccgtcccggactgatgggctgcctgtatcgagtggtgattttgtgccgagctgccggtcggggagctgttggctggctggtggcaggatatattgtggtgtaaacaaattgacgcttagacaacttaataacacattgcggacgtttttaatgtactggggtggtttttcttttcaccagtgagacgggcaacagctgattgcccttcaccgcctggccctgagagagttgcagcaagcggtccacgctggtttgccccagcaggcgaaaatcctgtttgatggtggttccgaaatcggcaaaatcccttataaatcaaaagaatagcccgagatagggttgagtgttgttccagtttggaacaagagtccactattaaagaacgtggactccaacgtcaaagggcgaaaaaccgtctatcagggcgatggcccactacgtgaaccatcacccaaatcaagttttttggggtcgaggtgccgtaaagcactaaatcggaaccctaaagggagcccccgatttagagcttgacggggaaagccggcgaacgtggcgagaaaggaagggaagaaagcgaaaggagcgggcgccattcaggctgcgcaactgttgggaagggcgatcggtgcgggcctcttcgctattacgccagctggcgaaagggggatgtgctgcaaggcgattaagttgggtaacgccagggttttcccagtcacgacgttgtaaaacgacggccagtgaattcgagctcggtacccccc

SEQ ID NO: 50 - DNA, 9663 bp, Tobacco rattle virus
ataaaacattgcacctatggtgttgccctggctggggtatgtcagtgatcgcagtagaatgtactaattgacaagttggagaatacggtagaacgtccttatccaacacagcctttatccctctccctgacgaggtttttgtcagtgtaatatttctttttgaactatccagcttagtaccgtacgggaaagtgactggtgtgcttatctttgaaatgttactttgggtttcggttctttaggttagtaagaaagcacttgtcttctcatacaaaggaaaacctgagacgtatcgcttacgaaagtagcaatgaaagaaaggtggtggttttaatcgctaccgcaaaaacgatggggtcgttttaattaacttctcctacgcaagcgtctaaacggacgttggggttttgctagtttctttagagaaaactagctaagtctttaatgttatcattagagatggcataaatataatacttgtgtctgctgataagatcattttaatttggacgattagacttgttgaactacaggttactgaatcacttgcgctaatcaacatgggagatatgtacgatgaatcatttgacaagtcgggcggtcctgctgacttgatggacgattcttgggtggaatcagtttcgtggaaagatctgttgaagaagttacacagcataaaatttgcactacagtctggtagagatgagatcactgggttactagcggcactgaatagacagtgtccttattcaccatatgagcagtttccagataagaaggtgtatttccttttagactcacgggctaacagtgctcttggtgtgattcagaacgcttcagcgttcaagagacgagctgatgagaagaatgcagtggcgggtgttacaaatattcctgcgaatccaaacacaacggttacgacgaaccaagggagtactactactaccaaggcgaacactggctcgactttggaagaagacttgtacacttattacaaattcgatgatgcctctacagctttccacaaatctctaacttcgttagagaacatggagttgaagagttattaccgaaggaactttgagaaagtattcgggattaagtttggtggagcagctgctagttcatctgcaccgcctccagcgagtggaggtccgatacgtcctaatccctagggatttaaggacgtgaactctgttgagatctctgtgaaattcagagggtgggtgataccatattcactgatgccattagcgacatctaaatagggctaattgtgactaatttgagggaatttcctttaccattgacgtcagtgtcgttggtagcatttgagtttcgcaatgcacgaattacttaggaagtggcttgacgacactaatgtgttattgttagataatggtttggtggtcaaggtacgtagtagagtcccacatattcgcacgtatgaagtaattggaaagttgtcagtttttgataattcactgggagatgatacgctgtttgagggaaaagtagagaacgtatttgtttttatgttcaggcggttcttgtgtgtcaacaaagatggacattgttactcaaggaagcacgatgagctttattattacggacgagtggacttagattctgtgagtaaggttaccgaattctctagaaggcctccatggggatccggtaccgagctcacgcgtctcgaggcccgggcatgtcccgaagacattaaactacggttctttaagtagatccgtgtctgaagttttaggttcaatttaaacctacgagattgacattctcgactgatcttgattgatcggtaagtcttttgtaatttaattttctttttgattttattttaaattgttatctgtttctgtgtatagactgtttgagatcggcgtttggccgactcattgtcttaccataggggaacggactttgtttgtgttgttattttatttgtattttattaaaattctcaacgatctgaaaaagcctcgcggctaagagattgttggggggtgagtaagtacttttaaagtgatgatggttacaaaggcaaaaggggtaaaacccctcgcctacgtaagcgttattacgcccgtctgtacttatatcagtacactgacgagtccctaaaggacgaaacgggagaacgctagccaccaccaccaccaccacgtgtgaattacaggtgaccagctcgaatttccccgatcgttcaaacatttggcaataaagtttcttaagattgaatcctgttgccggtcttgcgatgattatcatataatttctgttgaattacgttaagcatgtaataattaacatgtaatgcatgacgttatttatgagatgggtttttatgattagagtcccgcaattatacatttaatacgcgatagaaaacaaaatatagcgcgcaaactaggataaattatcgcgcgcggtgtcatctatgttactagatcgggaattaaactatcagtgtttgacaggatatattggcgggtaaacctaagagaaaagagcgtttattagaataacggatatttaaaagggcgtgaaaaggtttatccgttcgtccatttgtatgtgcatgccaaccacagggttcccctcgggatcaaagtactttgatccaacccctccgctgctatagtgcagtcggcttctgacgttcagtgcagccgtcttctgaaaacgacatgtcgcacaagtcctaagttacgcgacaggctgccgccctgcccttttcctggcgttttcttgtcgcgtgttttagtcgcataaagtagaatacttgcgactagaaccggagacattacgccatgaacaagagcgccgccgctggcctgctgggctatgcccgcgtcagcaccgacgaccaggacttgaccaaccaacgggccgaactgcacgcggccggctgcaccaagctgttttccgagaagatcaccggcaccaggcgcgaccgcccggagctggccaggatgcttgaccacctacgccctggcgacgttgtgacagtgaccaggctagaccgcctggcccgcagcacccgcgacctactggacattgccgagcgcatccaggaggccggcgcgggcctgcgtagcctggcagagccgtgggccgacaccaccacgccggccggccgcatggtgttgaccgtgttcgccggcattgccgagttcgagcgttccctaatcatcgaccgcacccggagcgggcgcgaggccgccaaggcccgaggcgtgaagtttggcccccgccctaccctcaccccggcacagatcgcgcacgcccgcgagctgatcgaccaggaaggccgcaccgtgaaagaggcggctgcactgcttggcgtgcatcgctcgaccctgtaccgcgcacttgagcgcagcgaggaagtgacgcccaccgaggccaggcggcgcggtgccttccgtgaggacgcattgaccgaggccgacgccctggcggccgccgagaatgaacgccaagaggaacaagcatgaaaccgcaccaggacggccaggacgaaccgtttttcattaccgaagagatcgaggcggagatgatcgcggccgggtacgtgttcgagccgcccgcgcacgtctcaaccgtgcggctgcatgaaatcctggccggtttgtctgatgccaagctggcggcctggccggccagcttggccgctgaagaaaccgagcgccgccgtctaaaaaggtgatgtgtatttgagtaaaacagcttgcgtcatgcggtcgctgcgtatatgatgcgatgagtaaataaacaaatacgcaaggggaacgcatgaaggttatcgctgtacttaaccagaaaggcgggtcaggcaagacgaccatcgcaacccatctagcccgcgccctgcaactcgccggggccgatgttctgttagtcgattccgatccccagggcagtgcccgcgattgggcggccgtgcgggaagatcaaccgctaaccgttgtcggcatcgaccgcccgacgattgaccgcgacgtgaaggccatcggccggcgcgacttcgtagtgatcgacggagcgccccaggcggcggacttggctgtgtccgcgatcaaggcagccgacttcgtgctgattccggtgcagccaagcccttacgacatatgggccaccgccgacctggtggagctggttaagcagcgcattgaggtcacggatggaaggctacaagcggcctttgtcgtgtcgcgggcgatcaaaggcacgcgcatcggcggtgaggttgccgaggcgctggccgggtacgagctgcccattcttgagtcccgtatcacgcagcgcgtgagctacccaggcactgccgccgccggcacaaccgttcttgaatcagaacccgagggcgacgctgcccgcgaggtccaggcgctggccgctgaaattaaatcaaaactcatttgagttaatgaggtaaagagaaaatgagcaaaagcacaaacacgctaagtgccggccgtccgagcgcacgcagcagcaaggctgcaacgttggccagcctggcagacacgccagccatgaagcgggtcaactttcagttgccggcggaggatcacaccaagctgaagatgtacgcggtacgccaaggcaagaccattaccgagctgctatctgaatacatcgcgcagctaccagagtaaatgagcaaatgaataaatgagtagatgaattttagcggctaaaggaggcggcatggaaaatcaagaacaaccaggcaccgacgccgtggaatgccccatgtgtggaggaacgggcggttggccaggcgtaagcggctgggttgtctgccggccctgcaatggcactggaacccccaagcccgaggaatcggcgtgacggtcgcaaaccatccggcccggtacaaatcggcgcggcgctgggtgatgacctggtggagaagttgaaggccgcgcaggccgcccagcggcaacgcatcgaggcagaagcacgccccggtgaatcgtggcaagcggccgctgatcgaatccgcaaagaatcccggcaaccgccggcagccggtgcgccgtcgattaggaagccgcccaagggcgacgagcaaccagattttttcgttccgatgctctatgacgtgggcacccgcgatagtcgcagcatcatggacgtggccgttttccgtctgtcgaagcgtgaccgacgagctggcgaggtgatccgctacgagcttccagacgggcacgtagaggtttccgcagggccggccggcatggccagtgtgtgggattacgacctggtactgatggcggtttcccatctaaccgaatccatgaaccgataccgggaagggaagggagacaagcccggccgcgtgttccgtccacacgttgcggacgtactcaagttctgccggcgagccgatggcggaaagcagaaagacgacctggtagaaacctgcattcggttaaacaccacgcacgttgccatgcagcgtacgaagaaggccaagaacggccgcctggtgacggtatccgagggtgaagccttgattagccgctacaagatcgtaaagagcgaaaccgggcggccggagtacatcgagatcgagctagctgattggatgtaccgcgagatcacagaaggcaagaacccggacgtgctgacggttcaccccgattactttttgatcgatcccggcatcggccgttttctctaccgcctggcacgccgcgccgcaggcaaggcagaagccagatggttgttcaagacgatctacgaacgcagtggcagcgccggagagttcaagaagttctgtttcaccgtgcgcaagctgatcgggtcaaatgacctgccggagtacgatttgaaggaggaggcggggcaggctggcccgatcctagtcatgcgctaccgcaacctgatcgagggcgaagcatccgccggttcctaatgtacggagcagatgctagggcaaattgccctagcaggggaaaaaggtcgaaaaggtctctttcctgtggatagcacgtacattgggaacccaaagccgtacattgggaaccggaacccgtacattgggaacccaaagccgtacattgggaaccggtcacacatgtaagtgactgatataaaagagaaaaaaggcgatttttccgcctaaaactctttaaaacttattaaaactcttaaaacccgcctggcctgtgcataactgtctggccagcgcacagccgaagagctgcaaaaagcgcctacccttcggtcgctgcgctccctacgccccgccgcttcgcgtcggcctatcgcggccgctggccgctcaaaaatggctggcctacggccaggcaatctaccagggcgcggacaagccgcgccgtcgccactcgaccgccggcgcccacatcaaggcaccctgcctcgcgcgtttcggtgatgacggtgaaaacctctgacacatgcagctcccggagacggtcacagcttgtctgtaagcggatgccgggagcagacaagcccgtcagggcgcgtcagcgggtgttggcgggtgtcggggcgcagccatgacccagtcacgtagcgatagcggagtgtatactggcttaactatgcggcatcagagcagattgtactgagagtgcaccatatgcggtgtgaaataccgcacagatgcgtaaggagaaaataccgcatcaggcgctcttccgcttcctcgctcactgactcgctgcgctcggtcgttcggctgcggcgagcggtatcagctcactcaaaggcggtaatacggttatccacagaatcaggggataacgcaggaaagaacatgtgagcaaaaggccagcaaaaggccaggaaccgtaaaaaggccgcgttgctggcgtttttccataggctccgcccccctgacgagcatcacaaaaatcgacgctcaagtcagaggtggcgaaacccgacaggactataaagataccaggcgtttccccctggaagctccctcgtgcgctctcctgttccgaccctgccgcttaccggatacctgtccgcctttctcccttcgggaagcgtggcgctttctcatagctcacgctgtaggtatctcagttcggtgtaggtcgttcgctccaagctgggctgtgtgcacgaaccccccgttcagcccgaccgctgcgccttatccggtaactatcgtcttgagtccaacccggtaagacacgacttatcgccactggcagcagccactggtaacaggattagcagagcgaggtatgtaggcggtgctacagagttcttgaagtggtggcctaactacggctacactagaaggacagtatttggtatctgcgctctgctgaagccagttaccttcggaaaaagagttggtagctcttgatccggcaaacaaaccaccgctggtagcggtggtttttttgtttgcaagcagcagattacgcgcagaaaaaaaggatctcaagaagatcctttgatcttttctacggggtctgacgctcagtggaacgaaaactcacgttaagggattttggtcatgcattctaggtactaaaacaattcatccagtaaaatataatattttattttctcccaatcaggcttgatccccagtaagtcaaaaaatagctcgacatactgttcttccccgatatcctccctgatcgaccggacgcagaaggcaatgtcataccacttgtccgccctgccgcttctcccaagatcaataaagccacttactttgccatctttcacaaagatgttgctgtctcccaggtcgccgtgggaaaagacaagttcctcttcgggcttttccgtctttaaaaaatcatacagctcgcgcggatctttaaatggagtgtcttcttcccagttttcgcaatccacatcggccagatcgttattcagtaagtaatccaattcggctaagcggctgtctaagctattcgtatagggacaatccgatatgtcgatggagtgaaagagcctgatgcactccgcatacagctcgataatcttttcagggctttgttcatcttcatactcttccgagcaaaggacgccatcggcctcactcatgagcagattgctccagccatcatgccgttcaaagtgcaggacctttggaacaggcagctttccttccagccatagcatcatgtccttttcccgttccacatcataggtggtccctttataccggctgtccgtcatttttaaatataggttttcattttctcccaccagcttatataccttagcaggagacattccttccgtatcttttacgcagcggtatttttcgatcagttttttcaattccggtgatattctcattttagccatttattatttccttcctcttttctacagtatttaaagataccccaagaagctaattataacaagacgaactccaattcactgttccttgcattctaaaaccttaaataccagaaaacagctttttcaaagttgttttcaaagttggcgtataacatagtatcgacggagccgattttgaaaccgcggtgatcacaggcagcaacgctctgtcatcgttacaatcaacatgctaccctccgcgagatcatccgtgtttcaaacccggcagcttagttgccgttcttccgaatagcatcggtaacatgagcaaagtctgccgccttacaacggctctcccgctgacgccgtcccggactgatgggctgcctgtatcgagtggtgattttgtgccgagctgccggtcggggagctgttggctggctggtggcaggatatattgtggtgtaaacaaattgacgcttagacaacttaataacacattgcggacgtttttaatgtactgaattaacgccgaattaattcctaggccaccatgttgggcccggcgcgccaagcttgcatgcctgcaggtcaacatggtggagcacgacactctcgtctactccaagaatatcaaagatacagtctcagaagaccagagggctattgagacttttcaacaaagggtaatatcgggaaacctcctcggattccattgcccagctatctgtcacttcatcgaaaggacagtagaaaaggaagatggcttctacaaatgccatcattgcgataaaggaaaggctatcgttcaagatgcctctaccgacagtggtcccaaagatggacccccacccacgaggaacatcgtggaaaaagaagacgttccaaccacgtcttcaaagcaagtggattgatgtgatggtcaacatggtggagcacgacactctcgtctactccaagaatatcaaagatacagtctcagaagaccagagggctattgagacttttcaacaaagggtaatatcgggaaacctcctcggattccattgcccagctatctgtcacttcatcgaaaggacagtagaaaaggaagatggcttctacaaatgccatcattgcgataaaggaaaggctatcgttcaagatgcctctaccgacagtggtcccaaagatggacccccacccacgaggaacatcgtggaaaaagaagacgttccaaccacgtcttcaaagcaagtggattgatgtgatatctccactgacgtaagggatgacgcacaatcccactatccttcgcaagacccttcctctatataaggaagttcatttcatttggagagg

SEQ ID NO: 51 - DNA, 300 bp, Artificial Sequence
  virus-induced gene silencing (VIGS) target sequence
attatagctatgtacacaattagcacgtgggcgaagacagtggcagaaaatgtctggtcactcattggaagaacagctccaccagattttcttacgaaattaacctatcttatatggaatcatcacgaagagatcaagcacattgatactgttcgagcatatacttttggtgctcattattttgtagaggttgatatagtgttgccagaggacatgctgttgaacaaggcacataatattggtgagacactgcaagaaaaattggagcaactccctgaagttgagcgagcttttgttcat

SEQ ID NO: 52 - DNA, 300 bp, Artificial Sequence
  VIGS control sequence
cgtcgtccaacattatcatggcctcgtgaaatcccgttagtaaaaggtggtaaacctgacgttgtacaaattgttaggaattataatgcttatctacgtgcaagtgatgatttaccaaaaatgtttattgaatcggacccaggattcttttccaatgctattgttgaaggtgccaagaagtttcctaatactgaatttgtcaaagtaaaaggtcttcatttttcgcaagaagatgcacctgatgaaatgggaaaatatatcaaatcgttcgttgagcgagttctcaaaaatgaacaataa

SEQ ID NO: 53 - DNA, 39 bp, Artificial Sequence
  yeast Fw primer
agggaatattaagcttatggagataagtcgcagcaatgt

SEQ ID NO: 54 - DNA, 38 bp, Artificial Sequence
  yeast Rv primer
gttactagtggatccttataccatagttttgtgttctg

SEQ ID NO: 55 - DNA, 14971 bp, Artificial Sequence
  modified pTES3 vector pYES3/UT.1
agcttgcatgcctgcaggtcgagcttttaggattccatagtgataagatatgttcttatctaaacaaaaaagcaagcgtcggcaaaccatacagctgtccacaaaaaggaaaggctgtaataacaagcggacccagcttctcagtggaagatactttatcagacactgaataatggatggaccctaccacgattaaagaggagcgtctgtctaaagtaaagtagatgcgtctttaataattcatctactttagacgtcatgcatgacgtttaacatgcattgtatccagatcctccctggctatataaagggagttaaatttcattgttaaggcatcgaaaaaaaaatttcaagtctatctctcaagaaaaacttagaaaattactttgtcttaaggatccgggcccagctgtcacaagtttgtacaaaaaagcaggctactaaaagctcgctcaacttcagggagttgctccaatttttcttgcagtgtctcaccaatattatgtgccttgttcaacagcatgtcctctggcaacactatatcaacctctacaaaataatgagcaccaaaagtatatgctcgaacagtatcaatgtgcttgatctcttcgtgatgattccatataagataggttaatttcgtaagaaaatctggtggagctgttcttccaatgagtgaccagacattttctgccactgtcttcgcccacgtgctaattgtgtacatagctatgatttcgtttttgaaccttcgacagtagaccataagcagaaacttgaccatagtgacagagaccataataccaatcgtccatttttccttctcatggtccatctcagggcgagactgatcgtaagcatagaaccaccgaaacaacaaacgtagattaagatgtcaagggtaatgcaattgttagtgaaattgcagtaagttacaagtctatatcctacaattgaagtagcactatgcgagttaatcttcacttagctatgcaacatcagtagaaatatcaaaaccagtccctttttattaggtagtatacagtagcctaatttatcttatgtaaacatctttggcctaactggtttggctacaacttcatttcagtagtaactcaacccgtttttcgtcttcttgtttcctataaattgcatgtttttttttgtcttgatgtaaaagattttagaaactcaaaactctactaaccataggaacctgctgctctgaaaattctcaggatagttgaagtgaagcaattcacataccttagttatgagttctttagctgactcgaacaatatttgtaatcctagtgtcgccattacagatgcaaaaacaataatacccaatggctgcatcctcttttttccaataggatagtgatactggtttggatttttcatggcatgagaagtgaaccacagtataaaccctgataagaggtctaagagggagtccaacgttgacgcgattacagccaaagatctgctctcaatagaagcgtagatttttgcaatgaaaagaaccacattagccatgtttgataaatgaatagccatcctttcacttcttgcaagctgcttcatttcatcctcagttagacttccaggtaaacaaccagattcattaatggtgtccatctcattgaacccttcaagcagcctttcttgttttttgtagtattcagcaattttaccttgtttcctgggagtgggaagtagacgacggacactaaaggagtgatgatcggaggaggagcggcttcgttcgggaagacggaattcgctaatgttaagtctccatgacgccgacgaagacgactgatccaccaccgcctgagcagccggagacagcagttccgtcctaaaactgctaaaactgtcgtccagagcgccgccgctgccgccaccaccactaacattgctgcgacttatctccatacccagctttcttgtacaaagtggtgcagctgagatctaggcctaagtaagtaagatcgttcaaacatttggcaataaagtttctttagattgaatcctgttgccggtcttgcgatgattatcatataatttctgttgaattacgttaagcatgtagtaattaacatgtaatggatgacgttatttatgagatgggtttttatgattagagtcccgcaattatacatttaatacgcgatagaaaacaaaatatagcgcgcaaactaggataaattatcgcgcgcggtgtcatctatgttactagatcgaaggccttgttctcgagcaattcactggccgtcgttttacaacgtcgtgactgggaaaaccctggcgttacccaacttaatcgccttgcagcacatccccctttcgccagcaggcgtaatagcgaagaggcccgcaccgattgcccttcccaacagttgcgcagcctgaatggcgcccgctcctttcgctttcttcccttcctttctcgccacgttcgccggctttccccgtcaagctctaaatcgggggctccctttagggttccgatttagtgctttacggcacctcgaccccaaaaaacttgatttgggtgatggttcacaaactatcagtgtttgacaggatatattggcgggtaaacctaagagaaaagagcgtttattagaataatcggatatttaaaagggcgtgaaaaggtttatccgttcgtccatttgtatgtgcatgccaaccacaggcttaagaaaacttgatttgggtgatggttcacaaactatcagtgtttgacaggatatattggcgggtaaacctaagagaaaagagcgtttattagaataatcggatatttaaaagggcgtgaaaaggtttatccgttcgtccatttgtatgtgcatgccaaccacaggcttaaggttctagactggcgccggccagcgagacgagcaagattggccgccgcccgaaacgatccgacagcgcgcccagcacaggtgcgcaggcaaattgcaccaacgcatacagcgccagcagaatgccatagtgggcggtgacctcgttcgagtgaaccagatcgcgcaggaggcccggcagcaccggcataatcaggccgatgccgacagcgtcgagcgcgacagtgctcagaattacgatcaggggtatgttgggtttcacgtctggcctccggaccagcctccgctggtccgattgaacgcgcggattctttatcactgataagttggtggacatattatgtttatcagtgataaagtgtcaagcatgacaaagttgcagccgaatacagtgatccgtgccgccctggacctgttgaacgaggtcggcgtagacggtctgacgacacgcaaactggcggaacggttgggggttcagcagccggcgctttactggcacttcaggaacaagcgggcgctgctcgacgcactggccgaagccatgctggcggagaatcatacgcattcggtgccgagagccgacgacgactggcgctcatttctgatcgggaatgcccgcagcttcaggcaggcgctgctcgcctaccgcgatggcgcgcgcatccatgccggcacgcgaccgggcgcaccgcagatggaaacggccgacgcgcagcttcgcttcctctgcgaggcgggtttttcggccggggacgccgtcaatgcgctgatgacaatcagctacttcactgttggggccgtgcttgaggagcaggccggcgacagcgatgccggcgagcgcggcggcaccgttgaacaggctccgctctcgccgctgttgcgggccgcgatagacgccttcgacgaagccggtccggacgcagcgttcgagcagggactcgcggtgattgtcgatggattggcgaaaaggaggctcgttgtcaggaacgttgaaggaccgagaaagggtgacgattgatgaggaccgctgccggagcgcaacccactcactacagcagagccatgtagacaacatcccctccccctttccaccgcgtcagacgcccgtagcagcccgctacgggctttttcatgccctgccctagcgtccaagcctcacggccgcgctcggcctctctggcggccttctggcgctcgtcgaccgctcactgactcgctgcgctcggtcgttcggctgcggcgagcggtatcagctcactcaaaggcggtaatacggttatccacagaatcaggggataacgcaggaaagaacatgtgagcaaaaggccagcaaaaggccaggaaccgtaaaaaggccgcgttgctggcgtttttccataggctccgcccccctgacgagcatcacaaaaatcgacgctcaagtcagaggtggcgaaacccgacaggactataaagataccaggcgtttccccctggaagctccctcgtgcgctctcctgttccgaccctgccgcttaccggatacctgtccgcctttctcccttcgggaagcgtggcgcttttccgctgcataaccctgcttcggggtcattatagcgattttttcggtatatccatcctttttcgcacgatatacaggattttgccaaagggttcgtgtagactttccttggtgtatccaacggcgtcagccgggcaggataggtgaagtaggcccacccgcgagcgggtgttccttcttcactgtcccttattcgcacctggcggtgctcaacgggaatcctgctctgcgaggctggccggctaccgccggcgtaacagatgagggcaagcggatggctgatgaaaccaagccaaccaggaagggcagcccacctatcaaggtgtactgccttccagacgaacgaagagcgattgaggaaaaggcggcggcggccggcatgagcctgtcggcctacctgctggccgtcggccagggctacaaaatcacgggcgtcgtggactatgagcacgtccgcgagctggcccgcatcaatggcgacctgggccgcctgggcggcctgctgaaactctggctcaccgacgacccgcgcacggcgcggttcggtgatgccacgatcctcgccctgctggcgaagatcgaagagaagcaggacgagcttggcaaggtcatgatgggcgtggtccgcccgagggcagagccatgacttttttagccgctaaaacggccggggggtgcgcgtgattgccaagcacgtccccatgcgctccatcaagaagagcgacttcgcggagctggtgaagtacatcaccgacgagcaaggcaagaccgagcgcctttggtacctcaccgggctggttgccctcgccgctgggctggcggccgtctatggccctgcaaacgcgccagaaacgccgtcgaagccgtgtgcgagacaccgccgccgccggcgttgtggatacctcgcggaaaacttggccctcactgacagatgaggggcggacgttgacacttgaggggccgactcacccggcgcggcgttgacagatgaggggcaggctcgatttcggccggcgacgtggagctggccagcctcgcaaatcggcgaaaacgcctgattttacgcgagtttcccacagatgatgtggacaagcctggggataagtgccctgcggtattgacacttgaggggcgcgactactgacagatgaggggcgcgatccttgacacttgaggggcagagtgctgacagatgaggggcgcacctattgacatttgaggggctgtccacaggcagaaaatccagcatttgcaagggtttccgcccgtttttcggccaccgctaacctgtcttttaacctgcttttaaaccaatatttataaaccttgtttttaaccagggctgcgccctgtgcgcgtgaccgcgcacgccgaaggggggtgcccccccttctcgaaccctcccggcccgctaacgcgggcctcccatccccccaggggctgcgcccctcggccgcgaacggcctcaccccaaaaatggcagcgctggcagtccttgccattgccgggatcggggcagtaacgggatgggcgatcagcccgagcgcgacgcccggaagcattgacgtgccgcaggtgctggcatcgacattcagcgaccaggtgccgggcagtgagggcggcggcctgggtggcggcctgcccttcacttcggccgtcggggcattcacggacttcatggcggggccggcaatttttaccttgggcattcttggcatagtggtcgcgggtgccgtgctcgtgttcgggggtgacgcgtgaaaattttcgataaacccagcgaaccatttgaggtgataggtaagattataccgaggtatgaaaacgagaattggacctttacagaattactctatgaagcgccatatttaaaaagctaccaagacgaagaggatgaagaggatgaggaggcagattgccttgaatatattgacaatactgataagataatatatcttttatatagaagatatggccgtatgtaaggatttcagggggcaaggcataggcagcgcgcttatcaatatatctatagaatgggcaaagcataaaaacttgcatggactaatgcttgaaacccaggacaataaccttatagcttgtaaattctatcataattgggtaatgactccaacttattgatagtgttttatgttcagataatgcccgatgactttgtcatgcagctccaccgattttgagaacgacagcgacttccgtcccagccgtgccaggtgctgcctcagattcaggttatgccgctcaattcgctgcgtatatcgcttgctgattacgtgcagctttcccttcaggcgggattcatacagcggccagccatccgtcatccatatcaccacgtcaaagggtgacagcaggctcataagacgccccagcgtcgccatagtgcgttcaccgaatacgtgcgcaacaaccgtcttccggagactgtcatacgcctaaaacagccagcgctggcgcgatttagccccgacatagccccactgttcgtccatttccgcgcagacgatgacgacactgcccggctgtatgcgcgaggttacctgctgccagtggcgataagtcgtgtcttaccgggttggactcaagacgatagttaccggataaggcgcagcggtcgggctgaacggggggttcgtgcacacagcccagcttggagcgaacgacctacaccgaactgagatacctacagcgtgagctatgagaaagcgccacgcttcccgaagggagaaaggcggacaggtatccggtaagcggcagggtcggaacaggagagcgcacgagggagcttccagggggaaacgcctggtatctttatagtcctgtcgggtttcgccacctctgacttgagcgtcgatttttgtgatgctcgtcaggggggcggagcctatggaaaaacgccagcaacgcggcctttttacggttcctggccttttgctggccttttgctcacatgttctttcctgcgttatcccctgattctgtggataaccgtattaccgcctttgagtgagctgataccgctcgccgcagccgaacgaccgagcgcagcgagtcagtgagcgaggaagcggaagagcgcctgatgcggtattttctccttacgcatctgtgcggtatttcacaccgcatagttaccgactgcggcctgagttttttaagtgacgtaaaatcgtgttgaggccaacgcccataatgcgggctgttgcccggcatccaacgccattcatggccatatcaatgattttctggtgcgtaccgggttgagaagcggtgtaagtgaacagcagttgccatgttttacggcagtgagagcagagatagcgctgatgtccggcggtgcttttgccgttacgcaccaccccgtcagtagctgaacaggagggacacctgatagacacagaagccactggagcacctcaaaaacaccatcatacactaaatcagtaagttggcagcatcacccgttaacataattgtggtttcaaaatcggctccgtcgatactatgttatacgccaactttgaaaacaactttgaaaaagctgttttctggtatttaaggttttagaatgcaaggaacagtgaattggagttcgtcttgttataattagcttcttggggtatctttaaatactgtagaaaagaggaaggaaataataaatggctaaaatgagaatatcaccggaattgaaaaaactgatcgaaaaataccgctgcgtaaaagatacggaaggaatgtctcctgctaaggtatataagctggtgggagaaaatgaaaacctatatttaaaaatgacggacagccggtataaagggaccacctatgatgtggaacgggaaaaggacatgatgctatggctggaaggaaagctgcctgttccaaaggtcctgcactttgaacggcatgatggctggagcaatctgctcatgagtgaggccgatggcgtcctttgctcggaagagtatgaagatgaacaaagccctgaaaagattatcgagctgtatgcggagtgcatcaggctctttcactccatcgacatatcggattgtccctatacgaatagcttagacagccgcttagccgaattggattacttactgaataacgatctggccgatgtggattgcgaaaactgggaagaagacactccatttaaagatccgcgcgagctgtatgattttttaaagacggaaaagcccgaagaggaacttgtcttttcccacggcgacctgggagacagcaacatctttgtgaaagatggcaaagtaagtggctttattgatcttgggagaagcggcagggcggacaagtggtatgacattgccttctgcgtccggtcgatcagggaggttatcggggaagaacagtatgtcgagctattttttgacttactggggatcaagcctgattgggagaaaataaaatattatattttactggatgaattgttttagtacctagagaaaattttcctaggtgtggcgcaacgatgccggcgacaagcaggagcgcaccgacttcttccgcatcaagtgttttggctctcaggccgaggcccacggcaagtatttgggcaaggggtcgctggtattcgtgcagggcaagattcggaataccaagtacgagaaggacggccagacggtctacgggaccgacttcattgccgataaggtggattatctggacaccaaggcaccaggcgggtcaaatcaggaataagggcacattgccccggcgtgagtcggggcaatcccgcaaggagggtgaatgaatcggacgtttgaccggaaggcatacaggcaagaactgatcgacgcggggttttccgccgaggatgccgaaaccatcgcaagccgcaccgtcatgcgtgcgccccgcgaaaccttccagtccgtcggctcgatggtccagcaagctacggccaagatcgagcgcgacagcgtgcaactggctccccctgccctgcccgcgccatcggccgccgtggagcgttcgcgtcgtctcgaacaggaggcggcaggtttggcgaagtcgatgaccatcgacacgcgaggaactatgacgaccaagaagcgaaaaaccgccggcgaggacctggcaaaacaggtcagcgaggccaagcaggccgcgttgctgaaacacacgaagcagcagatcaaggaaatgcagctttccttgttcgatattgcgccgtggccggacacgatgcgagcgatgccaaacgacacggcccgctctgccctgttcaccacgcgcaacaagaaaatcccgcgcgaggcgctgcaaaacaaggtcattttccacgtcaacaaggacgtgaagatcacctacaccggcgtcgagctgcgggccgacgatgacgaactggtgtggcagcaggtgttggagtacgcgaagcgcacccctatcggcgagccgatcaccttcacgttctacgagctttgccaggacctgggctggtcgatcaatggccggtattacacgaaggccgaggaatgcctgtcgcgcctacaggcgacggcgatgggcttcacgtccgaccgcgttgggcacctggaatcggtgtcgctgctgcaccgcttccgcgtcctggaccgtggcaagaaaacgtcccgttgccaggtcctgatcgacgaggaaatcgtcgtgctgtttgctggcgaccactacacgaaattcatctgggagaagtaccgcaagctgtcgccgacggcccgacggatgttcgactatttcagctcgcaccgggagccgtacccgctcaagctggaaaccttccgcctcatgtgcggatcggattccacccgcgtgaagaagtggcgcgagcaggtcggcgaagcctgcgaagagttgcgaggcagcggcctggtggaacacgcctgggtcaatgatgacctggtgcattgcaaacgctagggccttgtggggtcagttccggctgggggttcagcagccagcgtgatcactttactggcatttcaggaacaagcgggcactgctcgacgcacttgcttcgctcagtatcgctcgggacgcacggcgcgctctacgaactgccgataaacagaggattaaaattgacaattgtgattaaggctcagattcgacggcttggagcggccgacgtgcaggatttccgcgagatccgattgtcggccctgaagaaagctccagagatgttcgggtccgtttacgagcacgaggagaaaaagcccatggaggcgttcgctgaacggttgcgagatgccgtggcattcggcgcctacatcgacggcgagatcattgggctgtcggtcttcaaacaggaggacggccccaaggacgctcacaaggcgcatctgtccggcgttttcgtggagcccgaacagcgaggccgaggggtcgccggtatgctgctgcgggcgttgccggcgggtttattgctcgtgatgatcgtccgacagattccaacgggaatctggtggatgcgcatcttcatcctcggcgcacttaatatttcgctattctggagcttgttgtttatttcggtctaccgcctgccgggcggggtcgcggcgacggtaggcgctgtgcagccgctgatggtcgtgttcatctctgccgctctgctaggtagcccgatacgattgatggcggtcctgggggctatttgcggaactgcgggcgtggcgctgttggtgttgacaccaaacgcagcgctagatcctgtcggcgtcgcagcgggcctggcgggggcggtttccatggcgttcggaaccgtgctgacccgcaagtggcaacctcccgtgcctctgctcacctttaccgcctggcaactggcggccggaggacttctgctcgttccagtagctttagtgtttgatccgccaatcccgatgcctacaggaaccaatgttctcggcctggcgtggctcggcctgatcggagcgggtttaacctacttcctttggttccgggggatctcgcgactcgaacctacagttgtttccttactgggctttctcagccccaggtctggggtcgatcagccggggatgcatcaggccgacagtcggaacttcgggtccccgacctgtaccattcggtgagcaatggataggggagttgaaatcgtcaacgttcacttctaaagaaatagcgccactcagcttcctcagcggctttatccagcgatttcctattatgtcggcatagttctcaagatcgacagcctgtcacggttaagcgagaaatgaataagaaggctgataattcggatctctgcgagggagatgatatttgatgacaggcagcaacgctctgtcatcgttacaatcaacatgctaccctccgcgagatcatccgtgtttcaaacccggcagcttagttgccgttcttccgaatagcatcggtaacatgagcaaagtctgccgccttacaacggctctcccgctgactagtcgtcccggagacgtcctgatgggctgcctgtatcgagtggtgattttgtgccgagctgccggtcggggagctgttggctggctggtggcaggatatattgtggtgtaaacaaattgacgcttagacaacttaataacacattgcggacgtttttaatgtactggacgtcctgatgggctgcctgtatcgagtggtgattttgtgccgagctgccggtcggggagctgttggctggctggtggcaggatatattgtggtgtaaacaaattgacgcttagacaacttaataacacattgcggacgtttttaatgtactggggtggtttttcttttcaccagtgagacgggcaacacgtgattgcccttcaccgcctggccctgagagagttgcagcaagcggtccacgctggtttgccccagcaggcgaaaatcctgtttgatggtggttccgaaatcggcaaaatcccttataaatcaaaagaatagcccgagatagggttgagtgttgttccagtttggaacaagagtccactattaaagaacgtggactccaacgtcaaagggcgaaaaaccgtctatcagggcgatggcccacaaactgaaggcggccgcaaacgatatcaatctcatcatgagcggagaattaagggagtcacgttatgacccccgccgatgacgcgggacaagccgttttacgtttggaactgacagaaccgcaacgttgaaggagccactcagccgccggtttctggagtttaatgagctaagcacatacgtcagaaaccattattgcgcgttcaaaagtcgcctaaggtcactatcagctagcaaatatttcttgtcaaaaatgctccactgacgttccataaattcccctcggtatccaattagagtctcatattcactctcaatccaaataatctgcaccggatctggatcgtttcgcatgattgaacaagatggattgcacgcaggttctccggccgcttgggtggagaggctattcggctatgactgggcacaacagacaatcggctgctctgatgccgccgtgttccggctgtcagcgcaggggcgcccggttctttttgtcaagaccgacctgtccggtgccctgaatgaactccaggacgaggcagcgcggctatcgtggctggccacgacgggcgttccttgcgctgctgtgctcgacgttgtcactgaagcgggaagggactggctgctattgggcgaagtgccggggcaggatctcctgtcatctcaccttgctcctgccgagaaagtatccatcatggctgatgcaatgcggcggctgcatacgcttgatccggctacctgcccattcgaccaccaagcgaaacatcgcatcgagcgagcacgtactcggatggaagccggtcttgtcgatcaggatgatctggacgaagagcatcaggggctcgcgccagccgaactgttcgccaggctcaaggcgcgcatgcccgacggcgatgatctcgtcgtgacccatggcgatgcctgcttgccgaatatcatggtggaaaatggccgcttttctggattcatcgactgtggccggctgggtgtggcggaccgctatcaggacatagcgttggctacccgtgatattgctgaagagcttggcggcgaatgggctgaccgcttcctcgtgctttacggtatcgccgctcccgattcgcagcgcatcgccttctatcgccttcttgacgagttcttctgagcgggactctggggttcgaaatgaccgaccaagcgacgcccaacctgccatcacgagatttcgattccaccgccgccttctatgaaaggttgggcttcggaatcgttttccgggacgccggctggatgatcctccagcgcggggatctcatgctggagttcttcgcccacgggatctctgcggaacaggcggtcgaaggtgccgatattattacgacagcaacggccgacaagcacaacgccacgatcctgagcgacaatatgatcggacccggcgtccacatcaacggcgtcggcggcgactgcccaggcaagaccgagatgcaccgcgatatattgctgcgttcggatattttcgtggagttcccgccacagacccggatgatccccgaccgttcaaacatttggcaataaagtttctaaagattgaatcctgttgccggtcttgcgatgattatcatataatttctgttgaattacgttaagcatgtaataattaacatgtaatgcatgacgttatttatgagatgggtttttatgattagagtcccgcaattatacatttaatacgcgatagaaaacaaaatatagcgcgcaaactaggataaattatcgcgcgcggtgtcatctatgttactagatcgggcctcctgatatcaatgctgcagcggcggctctggtggtggttctggtggcggctctgagggtggtggctctgagggtggcggttctgagggtggcggctctgagggaggcggttccggtggtggctctggttccggtgattttgattatgaaaagatggcaaacgctaataagggggctatgaccgaaaatgccgatgaaaacgcgctacagtctgacgctaaaggcaaacttgattctgtcgctactgattacggtgctgctatgatggtttcattggtgacgtttccggccttgctaatggtaatggtgctactggtgattttgctggctctaattcccaaatggctcaagtcggtgacggtgataattcacctttaatgaatatttccgtcaatatttaccttccctccctcaatcggttgaatgtcgcccttttgtctttggcccaatacgcaaaccgcctctccccgcgcgttggccgattcattatgcactggcacgacaggtttcccgactggaaagcgggcagtgagcgcaacgcaattatgtgagttagctcactcattaggcaccccaggctttacactttatgcttccggctcgtatgttgtgtggaattgtgagcggataacaatttcacacaggaaacagctatgaccatgattacgccaagctggcgcca

SEQ ID NO: 56 - DNA, 37 bp, Artificial Sequence
  delta117C Fw primer
agggaatattaagcttatggagataagtcgcagcaat

SEQ ID NO: 57 - DNA, 36 bp, Artificial Sequence
  delta117C Rv primer
gttactagtggatccttaagctcccgtaggatcaat

SEQ ID NO: 58 - DNA, 5775 bp, Artificial Sequence
  pTES3 vector pYES3/UT.2
acggattagaagccgccgagcgggtgacagccctccgaaggaagactctcctccgtgcgtcctcgtcttcaccggtcgcgttcctgaaacgcagatgtgcctcgcgccgcactgctccgaacaataaagattctacaatactagcttttatggttatgaagaggaaaaattggcagtaacctggccccacaaaccttcaaatgaacgaatcaaattaacaaccataggatgataatgcgattagttttttagccttatttctggggtaattaatcagcgaagcgatgatttttgatctattaacagatatataaatgcaaaaactgcataaccactttaactaatactttcaacattttcggtttgtattacttcttattcaaatgtaataaaagtatcaacaaaaaattgttaatatacctctatactttaacgtcaaggagaaaaaaccccggatcggactactagcagctgtaatacgactcactatagggaatattaagcttggtaccgagctcggatccactagtaacggccgccagtgtgctggaattctgcagatatccagcacagtggcggccgctcgaaaacccgctgatcctagagggccgcatcatgtaattagttatgtcacgcttacattcacgccctccccccacatccgctctaaccgaaaaggaaggagttagacaacctgaagtctaggtccctatttatttttttatagttatgttagtattaagaacgttatttatatttcaaatttttcttttttttctgtacagacgcgtgtacgcatgtaacattatactgaaaaccttgcttgagaaggttttgggacgctcgaaggctttaatttgcaagctgcggccctgcattaatgaatcggccaacgcgcggggagaggcggtttgcgtattgggcgctcttccgcttcctcgctcactgactcgctgcgctcggtcgttcggctgcggcgagcggtatcagctcactcaaaggcggtaatacggttatccacagaatcaggggataacgcaggaaagaacatgtgagcaaaaggccagcaaaagcccaggaaccgtaaaaaggccgcgttgctggcgtttttccataggctccgcccccctgacgagcatcacaaaaatcgacgctcaagtcagaggtggcgaaacccgacaggactataaagataccaggcgtttccccctggaagctccctcgtgcgctctcctgttccgaccctgccgcttaccggatacctgtccgcctttctcccttcgggaagcgtggcgctttctcatagctcacgctgtaggtatctcagttcggtgtaggtcgttcgctccaagctgggctgtgtgcacgaaccccccgttcagcccgaccgctgcgccttatccggtaactatcgtcttgagtccaacccggtaagacacgacttatcgccactggcagcagccactggtaacaggattagcagagcgaggtatgtaggcggtgctacagagttcttgaagtggtggcctaactacggctacactagaaggacagtatttggtatctgcgctctgctgaagccagttaccttcggaaaaagagttggtagctcttgatccggcaaacaaaccaccgctggtagcggtggtttttttgtttgcaagcagcagattacgcgcagaaaaaaaggatctcaagaagatcctttgatcttttctacggggtctgacgctcagtggaacgaaaactcacgttaagggattttggtcatgagattatcaaaaaggatcttcacctagatccttttaaattaaaaatgaagttttaaatcaatctaaagtatatatgagtaaacttggtctgacagttaccaatgcttaatcagtgaggcacctatctcagcgatctgtctatttcgttcatccatagttgcctgactccccgtcgtgtagataactacgatacgggagcgcttaccatctggccccagtgctgcaatgataccgcgagacccacgctcaccggctccagatttatcagcaataaaccagccagccggaagggccgagcgcagaagtggtcctgcaactttatccgcctccatccagtctattaattgttgccgggaagctagagtaagtagttcgccagttaatagtttgcgcaacgttgttgccattgctacaggcatcgtggtgtcacgctcgtcgtttggtatggcttcattcagctccggttcccaacgatcaaggcgagttacatgatcccccatgttgtgcaaaaaagcggttagctccttcggtcctccgatcgttgtcagaagtaagttggccgcagtgttatcactcatggttatggcagcactgcataattctcttactgtcatgccatccgtaagatgcttttctgtgactggtgagtactcaaccaagtcattctgagaatagtgtatgcggcgaccgagttgctcttgcccggcgtcaacacgggataataccgcgccacatagcagaactttaaaagtgctcatcattggaaaacgttcttcggggcgaaaactctcaaggatcttaccgctgttgagatccagttcgatgtaacccactcgtgcacccaactgatcttcagcatcttttactttcaccagcgtttctgggtgagcaaaaacaggaaggcaaaatgccgcaaaaaagggaataagggcgacacggaaatgttgaatactcatactcttcctttttcaatattattgaagcatttatcagggttattgtctcatgagcggatacatatttgaatgtatttagaaaaataaacaaataggggttccgcgcacatttccccgaaaagtgccacctgacgtctaagaaaccattattatcatgacattaacctataaaaataggcgtatcacgaggccctttcgtcttcaagaaattcggtcgaaaaaagaaaaggagagggccaagagggagggcattggtgactattgagcacgtgagtatacgtgattaagcacacaaaggcagcttggagtatgtctgttattaatttcacaggtagttctggtccattggtgaaagtttgcggcttgcagagcacagaggccgcagaatgtgctctagattccgatgctgacttgctgggtattatatgtgtgcccaatagaaagagaacaattgacccggttattgcaaggaaaatttcaagtcttgtaaaagcatataaaaatagttcaggcactccgaaatacttggttggcgtgtttcgtaatcaacctaaggaggatgttttggctctggtcaatgattacggcattgatatcgtccaactgcacggagatgagtcgtggcaagaataccaagagttcctcggtttgccagttattaaaagactcgtatttccaaaagactgcaacatactactcagtgcagcttcacagaaacctcattcgtttattcccttgtttgattcagaagcaggtgggacaggtgaacttttggattggaactcgatttctgactgggttggaaggcaagagagccccgagagcttacattttatgttagctggtggactgacgccagaaaatgttggtgatgcgcttagattaaatggcgttattggtgttgatgtaagcggaggtgtggagacaaatggtgtaaaagactctaacaaaatagcaaatttcgtcaaaaatgctaagaaataggttattactgagtagtatttatttaagtattgtttgtgcacttgccctagcttatcgatgataagctgtcaaagatgagaattaattccacggactatagactatactagatactccgtctactgtacgatacacttccgctcaggtccttgtcctttaacgaggccttaccactcttttgttactctattgatccagctcagcaaaggcagtgtgatctaagattctatcttcgcgatgtagtaaaactagctagaccgagaaagagactagaaatgcaaaaggcacttctacaatggctgccatcattattatccgatgtgacgctgcagcttctcaatgatattcgaatacgctttgaggagatacagcctaatatccgacaaactgttttacagatttacgatcgtacttgttacccatcattgaattttgaacatccgaacctgggagttttccctgaaacagatagtatatttgaacctgtataataatatatagtctagcgctttacggaagacaatgtatgtatttcggttcctggagaaactattgcatctattgcataggtaatcttgcacgtcgcatccccggttcattttctgcgtttccatcttgcacttcaatagcatatctttgttaacgaagcatctgtgcttcattttgtagaacaaaaatgcaacgcgagagcgctaatttttcaaacaaagaatctgagctgcatttttacagaacagaaatgcaacgcgaaagcgctattttaccaacgaagaatctgtgcttcatttttgtaaaacaaaaatgcaacgcgacgagagcgctaatttttcaaacaaagaatctgagctgcatttttacagaacagaaatgcaacgcgagagcgctattttaccaacaaagaatctatacttcttttttgttctacaaaaatgcatcccgagagcgctatttttctaacaaagcatcttagattactttttttctcctttgtgcgctctataatgcagtctcttgataactttttgcactgtaggtccgttaaggttagaagaaggctactttggtgtctattttctcttccataaaaaaagcctgactccacttcccgcgtttactgattactagcgaagctgcgggtgcattttttcaagataaaggcatccccgattatattctataccgatgtggattgcgcatactttgtgaacagaaagtgatagcgttgatgattcttcattggtcagaaaattatgaacggtttcttctattttgtctctatatactacgtataggaaatgtttacattttcgtattgttttcgattcactctatgaatagttcttactacaatttttttgtctaaagagtaatactagagataaacataaaaaatgtagaggtcgagtttagatgcaagttcaaggagcgaaaggtggatgggtaggttatatagggatatagcacagagatatatagcaaagagatacttttgagcaatgtttgtggaagcggtattcgcaatgggaagctccaccccggttgataatcagaaaagccccaaaaacaggaagattgtataagcaaatatttaaattgtaaacgttaatattttgttaaaattcgcgttaaatttttgttaaatcagctcattttttaacgaatagcccgaaatcggcaaaatcccttataaatcaaaagaatagaccgagatagggttgagtgttgttccagtttccaacaagagtccactattaaagaacgtggactccaacgtcaaagggcgaaaaagggtctatcagggcgatggcccactacgtgaaccatcaccctaatcaagttttttggggtcgaggtgccgtaaagcagtaaatcggaagggtaaacggatgcccccatttagagcttgacggggaaagccggcgaacgtggcgagaaaggaagggaagaaagcgaaaggagcgggggctagggcggtgggaagtgtaggggtcacgctgggcgtaaccaccacacccgccgcgcttaatggggcgctacagggcgcgtggggatgatccactagt

SEQ ID NO: 59 - DNA, 37 bp, Artificial Sequence
  delta117N Fw primer
agggaatattaagcttatggaaatgaagcagcttgca

SEQ ID NO: 60 - DNA, 38 bp, Artificial Sequence; identical to SEQ ID NO: 54
  delta117N Rv primer